European Patent Application EP 4 471 152 A2, published December 4, 2024. Title: SPNS2 NEUTRALIZING ANTIBODY. Applicant: Teijin Pharma Limited. Application EP 24204947.6, filed October 7, 2024. The sequence listing filed with the application follows.

SEQUENCE LISTING (348 sequences)

SEQ ID NO: 1 - protein, 549 aa, Homo sapiens
MMCLECASAAAGGAEEEEADAERRRRRRGAQRGAGGSGCCGARGAGGAGVSAAGDEVQTLSGSVRRAPTGPPGTPGTPGCAATAKGPGAQQPKPASLGRGRGAAAAILSLGNVLNYLDRYTVAGVLLDIQQHFGVKDRGAGLLQSVFICSFMVAAPIFGYLGDRFNRKVILSCGIFFWSAVTFSSSFIPQQYFWLLVLSRGLVGIGEASYSTIAPTIIGDLFTKNTRTLMLSVFYFAIPLGSGLGYITGSSVKQAAGDWHWALRVSPVLGMITGTLILILVPATKRGHADQLGDQLKARTSWLRDMKALIRNRSYVFSSLATSAVSFATGALGMWIPLYLHRAQVVQKTAETCNSPPCGAKDSLIFGAITCFTGFLGVVTGAGATRWCRLKTQRADPLVCAVGMLGSAIFICLIFVAAKSSIVGAYICIFVGETLLFSNWAITADILMYVVIPTRRATAVALQSFTSHLLGDAGSPYLIGFISDLIRQSTKDSPLWEFLSLGYALMLCPFVVVLGGMFFLATALFFVSDRARAEQQVNQLAMPPASVKV

SEQ ID NO: 2 - DNA, 1650 bp, Homo sapiens
  source 1..1650: mol_type = genomic DNA
atgatgtgcctggaatgcgcctcggcggcggcgggcggcgcggaggaggaggaggcggacgcggagcggcggcgccggcgccggggggcgcagcgaggggctggcggtagcggttgctgcggggcgcggggcgcgggcggcgctggagtctcggccgcgggcgatgaggtgcagacgctgtcgggcagcgtaaggcgggccccgaccggaccccccggcacccccggcacccccggctgcgcagctactgcaaagggccccggcgctcagcagcccaaaccggccagcttgggccgcgggcggggggcagccgccgccatcctcagcttgggcaacgtgctcaactacctggacaggtacaccgtggcaggcgtccttctggacatccagcagcactttggggtcaaggaccgaggcgccggcctgctgcagtcagtgttcatctgtagcttcatggtggctgcccccatcttcggctacctgggcgaccgcttcaacaggaaggtgattctcagctgcggcattttcttctggtcggccgtcaccttctccagctccttcattccccagcagtacttctggctgctggtcctgtcccgggggctggtgggcatcggggaggccagctactccaccatcgcccccactatcattggcgacctcttcaccaagaacacgcgtacgctcatgctgtccgtcttctacttcgccatcccactgggcagtggcctgggctacattactggctccagcgtgaagcaggcagccggagactggcactgggcattgcgggtgtcccctgtcctgggcatgatcacaggaacactcatcctcattctggtcccagccactaaaaggggtcatgccgaccagctcggggaccagctcaaggcccggacctcatggctccgagatatgaaggccctgattcgaaaccgcagctacgtcttctcctccctggccacgtcggctgtctccttcgccacgggggccctgggcatgtggatcccgctctacctgcaccgcgcccaagttgtgcagaagacagcagagacgtgcaacagcccgccctgtggggccaaggacagcctcatctttggggccatcacctgctttacgggatttctgggcgtggtcacgggggcaggagccacgcgctggtgccgcctgaagacccagcgggccgacccactggtgtgtgccgtgggcatgctgggctctgccatcttcatctgcctgatcttcgtggctgccaagagcagcatcgtaggagcctatatctgtatcttcgtcggggagacgctgctgttttctaactgggccatcactgcagacatcctcatgtacgtggtcatccccacgcggcgcgccactgccgtggccttgcagagcttcacctcccacctgctgggggacgccgggagcccctacctcattggctttatctcagacctgatccgccagagcactaaggactccccgctctgggagttcctgagcctgggctacgcgctcatgctctgccctttcgtcgtggtcctgggcggcatgttcttcctcgccactgcgctcttcttcgtcagcgaccgcgccagggctgagcagcaggtgaaccagctggcgatgccgcccgcatctgtgaaagtctga

SEQ ID NO: 3 - protein, 13 aa, Homo sapiens
LDIQQHFGVKDRG

SEQ ID NO: 4 - protein, 14 aa, Homo sapiens
PQQYFWLLVLSRGL

SEQ ID NO: 5 - protein, 9 aa, Homo sapiens
VKQAAGDWH

SEQ ID NO: 6 - protein, 26 aa, Homo sapiens
PLYLHRAQVVQKTAETCNSPPCGAKD

SEQ ID NO: 7 - protein, 4 aa, Homo sapiens
AKSS

SEQ ID NO: 8 - protein, 19 aa, Homo sapiens
RQSTKDSPLWEFLSLGYAL

SEQ ID NO: 9 - DNA, 26 bp, synthetic construct
  misc_feature 1..26: note = Homo sapiens
  source 1..26: mol_type = other DNA
aagcttatgatgtgcctggaatgcgc

SEQ ID NO: 10 - DNA, 28 bp, synthetic construct
  misc_feature 1..28: note = Homo sapiens
  source 1..28: mol_type = other DNA
gcggccgctcagactttcacagatgcgg

SEQ ID NO: 11 - DNA, 26 bp, synthetic construct
  misc_feature 1..26: note = Homo sapiens
  source 1..26: mol_type = other DNA
gaattcatgtccgctcaagttctggg

SEQ ID NO: 12 - DNA, 29 bp, synthetic construct
  misc_feature 1..29: note = Homo Sapiens
  source 1..29: mol_type = other DNA
gcggccgctcataagggctcttctggcgg

SEQ ID NO: 13 - protein, 470 aa, Homo sapiens
MSAQVLGFLRSWTPLPLAAPRGPAAAGNDAGAPTATAPGGEGEPHSRPCDARLGSTDKELKAGAAATGSAPTAPGTPWQREPRVEVMDPAGGPRGVLPRPCRVLVLLNPRGGKGKALQLFRSHVQPLLAEAEISFTLMLTERRNHARELVRSEELGRWDALVVMSGDGLMHEVVNGLMERPDWETAIQKPLCSLPAGSGNALAASLNHYAGYEQVTNEDLLTNCTLLLCRRLLSPMNLLSLHTASGLRLFSVLSLAWGFIADVDLESEKYRRLGEMRFTLGTFLRLAALRTYRGRLAYLPVGRVGSKTPASPVVVQQGPVDAHLVPLEEPVPSHWTVVPDEDFVLVLALLHSHLGSEMFAAPMGRCAAGVMHLFYVRAGVSRAMLLRLFLAMEKGRHMEYECPYLVYVPVVAFRLEPKDGKGVFAVDGELMVSEAVQGQVHPNYFWMVSGCVEPPPSWKPQQMPPPEEPL

SEQ ID NO: 14 - DNA, 1413 bp, Homo sapiens
  source 1..1413: mol_type = genomic DNA
atgtccgctcaagttctgggatttttacgcagctggactcccctccccctggcagccccgaggggtccagccgccgcagggaatgacgccggtgctcctacagccacggctccgggcggggaaggcgagccccacagccggccctgcgacgcccgcctgggcagcaccgataaggagctgaaggcaggagccgccgccacgggcagcgcccccacagcgccagggaccccctggcagcgggagccgcgggtcgaggttatggatccagcgggcggcccccggggcgtgctcccgcggccctgccgcgtgctggtgctgctgaacccgcgcggcggcaagggcaaggccttgcagctcttccggagtcacgtgcagccccttttggctgaggctgaaatctccttcacgctgatgctcactgagcggcggaaccacgcgcgggagctggtgcggtcggaggagctgggccgctgggacgctctggtggtcatgtctggagacgggctgatgcacgaggtggtgaacgggctcatggagcggcctgactgggagaccgccatccagaagcccctgtgtagcctcccagcaggctctggcaacgcgctggcagcttccttgaaccattatgctggctatgagcaggtcaccaatgaagacctcctgaccaactgcacgctattgctgtgccgccggctgctgtcacccatgaacctgctgtctctgcacacggcttcggggctgcgcctcttctctgtgctcagcctggcctggggcttcattgctgatgtggacctagagagtgagaagtatcggcgtctgggggagatgcgcttcactctgggcaccttcctgcgtctggcagccctgcgcacctaccgcggccgactggcctacctccctgtaggaagagtgggttccaagacacctgcctcccccgttgtggtccagcagggcccggtagatgcacaccttgtgccactggaggagccagtgccctctcactggacagtggtgcccgacgaggactttgtgctagtcctggcactgctgcactcgcacctgggcagtgagatgtttgctgcacccatgggccgctgtgcagctggcgtcatgcatctgttctacgtgcgggcgggagtgtctcgtgccatgctgctgcgcctcttcctggccatggagaagggcaggcatatggagtatgaatgcccctacttggtatatgtgcccgtggtcgccttccgcttggagcccaaggatgggaaaggtgtgtttgcagtggatggggaattgatggttagcgaggccgtgcagggccaggtgcacccaaactacttctggatggtcagcggttgcgtggagcccccgcccagctggaagccccagcagatgccaccgccagaagagcccttatga

SEQ ID NO: 15 - DNA, 37 bp, synthetic construct
  misc_feature 1..37: note = Homo sapiens
  source 1..37: mol_type = other DNA
ggggaattcccaccatggcaactgccctcccgccgcg

SEQ ID NO: 16 - DNA, 35 bp, synthetic construct
  misc_feature 1..35: note = Homo Sapiens
  source 1..35: mol_type = other DNA
aaagcggccgctcagttgcagaagatcccattctg

SEQ ID NO: 17 - protein, 378 aa, Homo sapiens
MATALPPRLQPVRGNETLREHYQYVGKLAGRLKEASEGSTLTTVLFLVICSFIVLENLMVLIAIWKNNKFHNRMYFFIGNLALCDLLAGIAYKVNILMSGKKTFSLSPTVWFLREGSMFVALGASTCSLLAIAIERHLTMIKMRPYDANKRHRVFLLIGMCWLIAFTLGALPILGWNCLHNLPDCSTILPLYSKKYIAFCISIFTAILVTIVILYARIYFLVKSSSRKVANHNNSERSMALLRTVVIVVSVFIACWSPLFILFLIDVACRVQACPILFKAQWFIVLAVLNSAMNPVIYTLASKEMRRAFFRLVCNCLVRGRGARASPIQPALDPSRSKSSSSNNSSHSPKVKEDLPHTAPSSCIMDKNAALQNGIFCN

SEQ ID NO: 18 - DNA, 1137 bp, Homo sapiens
  source 1..1137: mol_type = genomic DNA
atggcaactgccctcccgccgcgtctccagccggtgcgggggaacgagaccctgcgggagcattaccagtacgtggggaagttggcgggcaggctgaaggaggcctccgagggcagcacgctcaccaccgtgctcttcttggtcatctgcagcttcatcgtcttggagaacctgatggttttgattgccatctggaaaaacaataaatttcacaaccgcatgtactttttcattggcaacctggctctctgcgacctgctggccggcatcgcttacaaggtcaacattctgatgtctggcaagaagacgttcagcctgtctcccacggtctggttcctcagggagggcagtatgttcgtggcccttggggcgtccacctgcagcttactggccatcgccatcgagcggcacttgacaatgatcaaaatgaggccttacgacgccaacaagaggcaccgcgtcttcctcctgatcgggatgtgctggctcattgccttcacgctgggcgccctgcccattctgggctggaactgcctgcacaatctccctgactgctctaccatcctgcccctctactccaagaagtacattgccttctgcatcagcatcttcacggccatcctggtgaccatcgtgatcctctacgcacgcatctacttcctggtgaagtccagcagccgtaaggtggccaaccacaacaactcggagcggtccatggcactgctgcggaccgtggtgattgtggtgagcgtgttcatcgcctgctggtccccactcttcatcctcttcctcattgatgtggcctgcagggtgcaggcgtgccccatcctcttcaaggctcagtggttcatcgtgttggctgtgctcaactccgccatgaacccggtcatctacacgctggccagcaaggagatgcggcgggccttcttccgtctggtctgcaactgcctggtcaggggacggggggcccgcgcctcacccatccagcctgcgctcgacccaagcagaagtaaatcaagcagcagcaacaatagcagccactctccgaaggtcaaggaagacctgccccacacagccccctcatcctgcatcatggacaagaacgcagcacttcagaatgggatcttctgcaactga

SEQ ID NO: 19 - protein, 549 aa, Mus musculus
MMCLECASAAAGGAEEEEADAERRRRRRGAQPGAGGSACCGARGVGGAGVVSADEEVQTLSGSVRRVPSGLPSIPSTPGCAAAAKGPSAPQPKPASLGRGRGAAAAILSLGNVLNYLDRYTVAGVLLDIQQHFGVKDRGAGLLQSVFICSFMVAAPIFGYLGDRFNRKVILSCGIFFWSAVTFSSSFIPQQYFWLLVLSRGLVGIGEASYSTIAPTIIGDLFTKNTRTLMLSVFYFAIPLGSGLGYITGSSVKQAAGDWHWALRVSPVLGMITGTLILILVPATKRGHADQLGGQLKARTSWLRDMKALIRNRSYVFSSLATSAVSFATGALGMWIPLYLHRAQVVQKTAETCNSPPCGAKDSLIFGAITCFTGFLGVVTGAGATRWCRLRTQRADPLVCAVGMLGSAIFICLIFVAAKTSIVGAYICIFVGETLLFSNWAITADILMYVVIPTRRATAVALQSFTSHLLGDAGSPYLIGFISDLIRQSTKDSPLWEFLSLGYALMLCPFVVVLGGMFFLATALFFLSDRAKAEQQVNQLVMPPASVKV

SEQ ID NO: 20 - DNA, 1650 bp, Mus musculus
  source 1..1650: mol_type = genomic DNA
atgatgtgcctggaatgcgcctcggcggcggcgggcggcgcggaggaggaggaggcggacgccgagcggcggcgccggcgccggggggcgcagccaggggctggaggtagcgcttgctgcggggcgcggggtgttgggggcgctggagtcgtgtccgccgacgaagaggtgcagacgttgtccggcagcgtgaggcgggtcccgtccggactccccagcatccccagcacccctggctgcgcagcagctgccaagggccccagcgcgccgcagcccaaaccggccagcttaggccgagggcggggggcagctgctgccatcctgagtttaggcaacgtgctcaactacctggacaggtacactgtggcaggtgttcttctggacatccagcagcactttggggtcaaggaccggggcgccggcttgctgcagtcagtgttcatctgcagcttcatggtggctgcccccatctttggctacctgggcgaccgcttcaatagaaaggtgatcctcagctgtggcatcttcttctggtctgctgtcaccttctcgagttctttcatccctcagcagtacttctggctactagtcctgtcccgagggctagtaggtattggtgaagccagctactccaccatagcacccaccatcattggcgacttgtttaccaagaacacacgcacattgatgctatctgtcttctattttgccatccccctgggcagtggcctgggctatatcacaggttccagcgtgaagcaggcagctggagactggcattgggccctgcgggtttcccccgtcctgggcatgatcacaggaacactcatcctcatcttggtcccagccactaagagaggccatgctgatcaacttggggggcagctcaaagcacggacctcctggcttcgagacatgaaggccctgatccgaaaccgcagttacgtcttctcctccctggccacatccgctgtgtccttcgccacaggggccctgggcatgtggattcccctctatcttcaccgtgctcaagttgtacaaaagacagcagagacttgcaacagcccgccctgtggagccaaagacagcctcatctttggagccattacctgctttactggcttcctgggcgtagtcacgggcgcgggagccactcgttggtgccgcctgcggactcaacgtgctgacccattggtgtgtgctgtgggcatgctgggatccgccatcttcatctgcctcatctttgtggctgccaagaccagcattgtaggcgcttatatctgcatttttgttggagagacactgctgttttctaactgggccatcactgcagacatcctcatgtatgtggtcatccccactcggcgagccactgctgtggccctgcagagcttcacctcccatctgctgggggacgctggaagcccctacctcattggctttatctcggacctaatccgccagagcaccaaggactccccgctctgggagttcctgagcctgggctatgccctcatgctgtgcccttttgtcgtggtcctgggtggcatgttcttccttgccactgctctcttcttcctcagcgaccgtgccaaggctgagcagcaggtgaaccagctggtgatgcctcctgcatccgtgaaagtctga

SEQ ID NO: 21 - DNA, 17 bp, synthetic construct
  misc_feature 1..17: note = M13
  source 1..17: mol_type = other DNA
gtaaaacgacggccagt

SEQ ID NO: 22 - protein, 8 aa, synthetic construct
  REGION 1..8: note = Flag tag
DYKDDDDK

SEQ ID NO: 23 - DNA, 59 bp, synthetic construct
  misc_feature 1..59: note = Homo sapiens
  source 1..59: mol_type = other DNA
aagcttgaattcatggattacaaggatgacgacgataagatgatgtgcctggaatgcgc

SEQ ID NO: 24 - DNA, 29 bp, synthetic construct
  misc_feature 1..29: note = Homo sapiens
  source 1..29: mol_type = other DNA
agcggccgctcagactttcacagatgcgg

SEQ ID NO: 25 - DNA, 32 bp, synthetic construct
  misc_feature 1..32: note = Homo Sapiens
  source 1..32: mol_type = other DNA
aagcttgaattcatgatgtgcctggaatgcgc

SEQ ID NO: 26 - DNA, 52 bp, synthetic construct
  misc_feature 1..52: note = Homo Sapiens
  source 1..52: mol_type = other DNA
gcggccgctcacttatcgtcgtcatccttgtaatcgactttcacagatgcgg

SEQ ID NO: 27 - protein, 558 aa, synthetic construct
  REGION 1..558: note = N' Flag
MDYKDDDDKMMCLECASAAAGGAEEEEADAERRRRRRGAQRGAGGSGCCGARGAGGAGVSAAGDEVQTLSGSVRRAPTGPPGTPGTPGCAATAKGPGAQQPKPASLGRGRGAAAAILSLGNVLNYLDRYTVAGVLLDIQQHFGVKDRGAGLLQSVFICSFMVAAPIFGYLGDRFNRKVILSCGIFFWSAVTFSSSFIPQQYFWLLVLSRGLVGIGEASYSTIAPTIIGDLFTKNTRTLMLSVFYFAIPLGSGLGYITGSSVKQAAGDWHWALRVSPVLGMITGTLILILVPATKRGHADQLGDQLKARTSWLRDMKALIRNRSYVFSSLATSAVSFATGALGMWIPLYLHRAQVVQKTAETCNSPPCGAKDSLIFGAITCFTGFLGVVTGAGATRWCRLKTQRADPLVCAVGMLGSAIFICLIFVAAKSSIVGAYICIFVGETLLFSNWAITADILMYVVIPTRRATAVALQSFTSHLLGDAGSPYLIGFISDLIRQSTKDSPLWEFLSLGYALMLCPFVVVLGGMFFLATALFFVSDRARAEQQVNQLAMPPASVKV

SEQ ID NO: 28 - DNA, 1677 bp, synthetic construct
  misc_feature 1..1677: note = N' Flag
  source 1..1677: mol_type = other DNA
atggattacaaggatgacgacgataagatgatgtgcctggaatgcgcctcggcggcggcgggcggcgcggaggaggaggaggcggacgcggagcggcggcgccggcgccggggggcgcagcgaggggctggcggtagcggttgctgcggggcgcggggcgcgggcggcgctggagtctcggccgcgggcgatgaggtgcagacgctgtcgggcagcgtaaggcgggccccgaccggaccccccggcacccccggcacccccggctgcgcagctactgcaaagggccccggcgctcagcagcccaaaccggccagcttgggccgcgggcggggggcagccgccgccatcctcagcttgggcaacgtgctcaactacctggacaggtacaccgtggcaggcgtccttctggacatccagcagcactttggggtcaaggaccgaggcgccggcctgctgcagtcagtgttcatctgtagcttcatggtggctgcccccatcttcggctacctgggcgaccgcttcaacaggaaggtgattctcagctgcggcattttcttctggtcggccgtcaccttctccagctccttcattccccagcagtacttctggctgctggtcctgtcccgggggctggtgggcatcggggaggccagctactccaccatcgcccccactatcattggcgacctcttcaccaagaacacgcgtacgctcatgctgtccgtcttctacttcgccatcccactgggcagtggcctgggctacattactggctccagcgtgaagcaggcagccggagactggcactgggcattgcgggtgtcccctgtcctgggcatgatcacaggaacactcatcctcattctggtcccagccactaaaaggggtcatgccgaccagctcggggaccagctcaaggcccggacctcatggctccgagatatgaaggccctgattcgaaaccgcagctacgtcttctcctccctggccacgtcggctgtctccttcgccacgggggccctgggcatgtggatcccgctctacctgcaccgcgcccaagttgtgcagaagacagcagagacgtgcaacagcccgccctgtggggccaaggacagcctcatctttggggccatcacctgctttacgggatttctgggcgtggtcacgggggcaggagccacgcgctggtgccgcctgaagacccagcgggccgacccactggtgtgtgccgtgggcatgctgggctctgccatcttcatctgcctgatcttcgtggctgccaagagcagcatcgtaggagcctatatctgtatcttcgtcggggagacgctgctgttttctaactgggccatcactgcagacatcctcatgtacgtggtcatccccacgcggcgcgccactgccgtggccttgcagagcttcacctcccacctgctgggggacgccgggagcccctacctcattggctttatctcagacctgatccgccagagcactaaggactccccgctctgggagttcctgagcctgggctacgcgctcatgctctgccctttcgtcgtggtcctgggcggcatgttcttcctcgccactgcgctcttcttcgtcagcgaccgcgccagggctgagcagcaggtgaaccagctggcgatgccgcccgcatctgtgaaagtctga

SEQ ID NO: 29 - protein, 557 aa, synthetic construct
  REGION 1..557: note = C' Flag
MMCLECASAAAGGAEEEEADAERRRRRRGAQRGAGGSGCCGARGAGGAGVSAAGDEVQTLSGSVRRAPTGPPGTPGTPGCAATAKGPGAQQPKPASLGRGRGAAAAILSLGNVLNYLDRYTVAGVLLDIQQHFGVKDRGAGLLQSVFICSFMVAAPIFGYLGDRFNRKVILSCGIFFWSAVTFSSSFIPQQYFWLLVLSRGLVGIGEASYSTIAPTIIGDLFTKNTRTLMLSVFYFAIPLGSGLGYITGSSVKQAAGDWHWALRVSPVLGMITGTLILILVPATKRGHADQLGDQLKARTSWLRDMKALIRNRSYVFSSLATSAVSFATGALGMWIPLYLHRAQVVQKTAETCNSPPCGAKDSLIFGAITCFTGFLGVVTGAGATRWCRLKTQRADPLVCAVGMLGSAIFICLIFVAAKSSIVGAYICIFVGETLLFSNWAITADILMYVVIPTRRATAVALQSFTSHLLGDAGSPYLIGFISDLIRQSTKDSPLWEFLSLGYALMLCPFVVVLGGMFFLATALFFVSDRARAEQQVNQLAMPPASVKVDYKDDDDK

SEQ ID NO: 30 - DNA, 1674 bp, synthetic construct
  misc_feature 1..1674: note = C' Flag
  source 1..1674: mol_type = other DNA
atgatgtgcctggaatgcgcctcggcggcggcgggcggcgcggaggaggaggaggcggacgcggagcggcggcgccggcgccggggggcgcagcgaggggctggcggtagcggttgctgcggggcgcggggcgcgggcggcgctggagtctcggccgcgggcgatgaggtgcagacgctgtcgggcagcgtaaggcgggccccgaccggaccccccggcacccccggcacccccggctgcgcagctactgcaaagggccccggcgctcagcagcccaaaccggccagcttgggccgcgggcggggggcagccgccgccatcctcagcttgggcaacgtgctcaactacctggacaggtacaccgtggcaggcgtccttctggacatccagcagcactttggggtcaaggaccgaggcgccggcctgctgcagtcagtgttcatctgtagcttcatggtggctgcccccatcttcggctacctgggcgaccgcttcaacaggaaggtgattctcagctgcggcattttcttctggtcggccgtcaccttctccagctccttcattccccagcagtacttctggctgctggtcctgtcccgggggctggtgggcatcggggaggccagctactccaccatcgcccccactatcattggcgacctcttcaccaagaacacgcgtacgctcatgctgtccgtcttctacttcgccatcccactgggcagtggcctgggctacattactggctccagcgtgaagcaggcagccggagactggcactgggcattgcgggtgtcccctgtcctgggcatgatcacaggaacactcatcctcattctggtcccagccactaaaaggggtcatgccgaccagctcggggaccagctcaaggcccggacctcatggctccgagatatgaaggccctgattcgaaaccgcagctacgtcttctcctccctggccacgtcggctgtctccttcgccacgggggccctgggcatgtggatcccgctctacctgcaccgcgcccaagttgtgcagaagacagcagagacgtgcaacagcccgccctgtggggccaaggacagcctcatctttggggccatcacctgctttacgggatttctgggcgtggtcacgggggcaggagccacgcgctggtgccgcctgaagacccagcgggccgacccactggtgtgtgccgtgggcatgctgggctctgccatcttcatctgcctgatcttcgtggctgccaagagcagcatcgtaggagcctatatctgtatcttcgtcggggagacgctgctgttttctaactgggccatcactgcagacatcctcatgtacgtggtcatccccacgcggcgcgccactgccgtggccttgcagagcttcacctcccacctgctgggggacgccgggagcccctacctcattggctttatctcagacctgatccgccagagcactaaggactccccgctctgggagttcctgagcctgggctacgcgctcatgctctgccctttcgtcgtggtcctgggcggcatgttcttcctcgccactgcgctcttcttcgtcagcgaccgcgccagggctgagcagcaggtgaaccagctggcgatgccgcccgcatctgtgaaagtcgattacaaggatgacgacgataagtga

SEQ ID NO: 31 - protein, 549 aa, Macaca mulatta
MMCLECASAAAGGAEEEEADAERRRRRRGAQRGAGGSGCCGARGAGGAGVSAADDEVQTLSGSVRRAPTGPPGTPGTPGCAATAKGPGAQQPKPASLGRGRGAAAAILSLGNVLNYLDRYTVAGVLLDIQQHFGVKDRGAGLLQSVFICSFMVAAPIFGYLGDRFNRKVILSCGIFFWSAVTFSSSFIPQQYFWLLVLSRGLVGIGEASYSTIAPTIIGDLFTKNTRTLMLSVFYFAIPLGSGLGYITGSSVKQAAGDWHWALRVSPVLGMITGTLILILVPATKRGHADQLGDQLKTRTSWLRDMKALIRNRSYVFSSLATSAVSFATGALGMWIPLYLHRAQVVQKTAETCNSPPCGAKDSLIFGAITCFTGFLGVVTGAGATRWCRLKTQRADPLVCAVGMLGSAIFICLIFVAAKSSIVGAYICIFVGETLLFSNWAITADILMYVVIPTRRATAVALQSFTSHLLGDAGSPYLIGFISDLIRQSTKDSPLWEFLSLGYALMLCPFVVVLGGMFFLATALFFLSDRAKAEQQVNQLVMPPASVKV

SEQ ID NO: 32 - protein, 549 aa, Cavia porcellus
MMCLECASAAAGGAEEEEADAERRRRRRGAQRGASGSGCCGTRDTGGAGVAAVNDEVQTLSGSVRRAPAGPSSIPGTPGCAAAAKSPCAQQPKPASLGRGRGAAAAILSLGNVLNYLDRYTVAGVLLDIQQHFGVKDRGAGLLQSVFICSFMVAAPIFGYLGDRFNRKVILSCGIFFWSAVTFSSSFIPQQYFWLLVLSRGLVGIGEASYSTIAPTIIGDLFTKNTRTLMLSVFYFAIPLGSGLGYITGSSVKQAAGDWHWALRVSPVLGMITGTLILILVPATKRGHADQLGGQLKARTSWLRDMKALIRNRSYVFSSLATSAVSFATGALGMWIPLYLHRAQVVQKTAETCHSPPCGAKDSLIFGAITCFTGFLGVVTGAGATRWCRLRTQRADPLVCAVGMLGSAIFICLIFVAAKSSIVGAYICIFVGETLLFSNWAITADILMCVVIPTRRATAVALQSFTSHLLGDAGSPYLIGFISDLIRQSTKDSPLWEFLSLGYALMLCPFVVVLGGMFFLATALFFLSDRAKAEQQVNQLVLPRPPMKV

SEQ ID NO: 33 - protein, 549 aa, Rattus norvegicus
MMCLECASAAAGGAEEEEADAERRRRRRGAQPGAGGSACCGARGVGGAGVVSADEEVQTLSGSVRRVPSGLPSIPSTPGCAAAAKGPGAPQPKPASLGRGRGAAAAILSLGNVLNYLDRYTVAGVLLDIQQHFGVKDRGAGLLQSVFICSFMVAAPIFGYLGDRFNRKVILSCGIFFWSAVTFSSSFIPQQYFWLLVLSRGLVGIGEASYSTIAPTIIGDLFTKNTRTLMLSVFYFAIPLGSGLGYITGSSVKQAAGDWHWALRVSPVLGMITGTLILILVPATKRGHADQLGGQLKARTSWLRDMKALIRNRSYVFSSLATSAVSFATGALGMWIPLYLHRAQVVQKTAETCNSPPCGAKDSLIFGAITCFTGFLGVVTGAGATRWCRLRTQRADPLVCAVGMLGSAIFICLIFVAAKTSIVGAYICIFVGETLLFSNWAITADILMYVVIPTRRATAVALQSFTSHLLGDAGSPYLIGFISDLIRQSTKDSPLWEFLSLGYALMLCPFVVVLGGMFFLATALFFLSDRAKAEQQVNQLVMPPASVKI

SEQ ID NO: 34 - protein, 121 aa, Rattus norvegicus
AVQLVGSGGGLVQPGRSMKLSCEASGFTFSNHYMAWVRQAPTRGLEWVATISTGGGNTYYRDSVKGRFTISRDNTRSTLSLQMDSLRSEDTATYYCTRQDYTNYMGGFAYWGQGTLVTVSS

SEQ ID NO: 35 - DNA, 363 bp, Rattus norvegicus
  source 1..363: mol_type = genomic DNA
gcggtgcagctggtggggtctgggggaggcttagtgcagcctggaaggtccatgaaactctcctgtgaagcctcaggattcactttcagtaaccattacatggcctgggtccgccaggcaccaacaaggggtctggagtgggtcgcgaccattagtactggtggtggtaatacttactatcgcgactccgtgaagggccgattcactatctccagagataatacaagaagcaccctatccctgcagatggacagtctgaggtctgaggacacggccacttattactgtacaagacaagattatactaactatatgggggggtttgcttactggggccagggcactctggtcactgtctcttca

SEQ ID NO: 36 - protein, 119 aa, Rattus norvegicus
EVQLVESGGGLVRPGGSMKLSCGASGFIFDNYYMTWVRQAPTKGLEWVASISSSGGNTYYRDSVRGRFTISRDNAGNTLSLQMGSLRAEDTATYHCAKEGYRGRYFDYWGQGVMVTVSS

SEQ ID NO: 37 - DNA, 357 bp, Rattus norvegicus
  source 1..357: mol_type = genomic DNA
gaggtgcaactggtggagtctgggggaggcttagtgcggcctggggggtccatgaaactctcctgtggagcctcaggattcattttcgataactattacatgacctgggtccgccaggctccaacgaagggtctggagtgggtcgcatccattagttctagtggtggtaacacttactatcgagattccgtgaggggccggttcactatctccagagataatgcaggaaacaccctatccctgcaaatgggcagtctgagggctgaggacacggccacttatcactgtgcgaaagagggctacaggggtcggtactttgattactggggccaaggagtcatggtcacagtctcctca

SEQ ID NO: 38 - protein, 115 aa, Rattus norvegicus
EVHLQQSGAALVRPRASVKLSCKVSGDSISRYYVHFVKQRPGQGLEWIGRIDPEDDTTKYSEKFKNRATLTADASSDTASLILSGLTSDDTATYFCSTLTGLDYWGQGVMVTVSS

SEQ ID NO: 39 - DNA, 345 bp, Rattus norvegicus
  source 1..345: mol_type = genomic DNA
gaagtccacctgcagcagtctggggctgcgcttgtgagacctagggcctctgtgaagttatcttgcaaagtttctggcgattccatttcaagatactacgtgcactttgtgaagcaaaggcctggacagggtctggaatggataggaaggattgatcctgaggatgatactactaagtattctgagaagttcaaaaacagggcgacactcactgcagatgcatcctccgacacagcctccctgattctcagcggcctgacctctgacgacactgcaacctatttttgtagcactctaactggccttgattactggggccaaggagtcatggtcacggtctcctca

SEQ ID NO: 40 - protein, 121 aa, Rattus norvegicus
EVQLVESGGGLVQPGRSMKLSCAASGFTFSNHYMAWVRQAPTKGLEWVASISTGGGNTYYRDSVKGRFTISRDNAKSTLYLQMDSLRSEDTATYYCARQDYSNYMGGFAYWGQGTLVTVSS

SEQ ID NO: 41 - DNA, 363 bp, Rattus norvegicus
  source 1..363: mol_type = genomic DNA
gaggtgcagctggtggagtctgggggaggcttagtgcagcctggaaggtccatgaagctctcctgtgcagcctcaggattcactttcagtaaccattacatggcctgggtccgccaggcaccaacaaagggtctggagtgggtcgcgtccattagtactggtggtggtaatacttattatcgagactccgtgaagggccgattcactatctccagagataatgcaaaaagcaccctttatctgcaaatggacagtctgaggtctgaggacacggccacttattattgtgccagacaagactatagtaactatatgggggggtttgcttactggggccaaggcactctggtcactgtctcttca

SEQ ID NO: 42 - protein, 121 aa, Rattus norvegicus
EVQLVGSGGGLVQPGRSMKLSCEASGFTFSNHYMAWVRQAPTKGLEWVATISTGGGNTYYRDSVKGRFTISRDNARSTLSLQMDSLRSEDTATYYCARQDYSNYMGGFAYWGQGTLVTVSS

SEQ ID NO: 43 - DNA, 363 bp, Rattus norvegicus
  source 1..363: mol_type = genomic DNA
gaggtgcagctggtggggtctgggggaggcttagtgcagcctggaaggtccatgaaactctcctgtgaagcctcaggattcactttcagtaaccattacatggcctgggtccgccaggcaccaacaaagggtctggagtgggtcgcgaccattagtactggtggtggtaatacttactatcgcgactccgtgaagggccgattcactatctccagagataatgcaagaagcaccctatccctgcagatggacagtctgaggtctgaggacacggccacttattactgtgcaagacaagattatagtaactatatgggggggtttgcttactggggccagggcactctggtcactgtctcttca

SEQ ID NO: 44 - protein, 115 aa, Rattus norvegicus
EVQLQQSGAELVRPRTSVKLSCKVSGDSITRYYVHFVKQRPGQGLEWIGRIDPEDDTTKYSEKFKKKATLTADASSNTAYLIFSGLTSEDTATYFCSTLTGLDYWGQGVMVTVSS

SEQ ID NO: 45 - DNA, 345 bp, Rattus norvegicus
  source 1..345: mol_type = genomic DNA
gaagtccagctgcagcagtctggggctgagcttgtgagacctaggacctctgtgaagttatcttgcaaagtttctggcgattccattacaagatactacgtgcactttgtgaagcaaaggcctggacagggtctggaatggataggaaggattgatcctgaggatgatactactaagtattctgagaagttcaaaaagaaggcgacactcactgcagatgcatcctccaacacagcctacctgattttcagcggcctgacctctgaggacactgcaacctatttttgtagcactctaactggccttgattactggggccaaggagtcatggtcacggtctcctca

SEQ ID NO: 46 - protein, 118 aa, Rattus norvegicus
EVQVVESGGGLVQPGRSMKLSCAALGFTFRDYYMAWVRQTPTKGLEWVAAISTGGGNTYYRDSVKGRFTISRDNAKSTLYLQMDSLRSDDTATYYCARNPYGNYFDYWGQGVMVTVSS

SEQ ID NO: 47 - DNA, 354 bp, Rattus norvegicus
  source 1..354: mol_type = genomic DNA
gaggtgcaggtggtggagtctgggggaggcttagtgcagcctggaaggtccatgaaactctcctgtgcagccttaggattcactttccgtgactattacatggcctgggtccgccagacaccaacaaagggtctggagtgggtcgcagccattagtactggtggtggaaacacttactatcgagactccgtgaagggccgattcactatctccagagataatgcaaaaagcaccctttatctgcaaatggacagtctgaggtctgacgacacggccacttattactgtgcaagaaacccctacggcaactactttgattattggggccaaggagtcatggtcacagtctcctct

SEQ ID NO: 48 - protein, 115 aa, Rattus norvegicus
EVHLVESGGGLVQPGRSMKLSCTASGFTFNNYYMAWVRQAPTKGLEWVASISTGGGYTYYRDSVKGRFTISRDNTGNTLYLQMDSLRSEDTATYYCARCWELPYWGQGVMVTVSS

SEQ ID NO: 49 - DNA, 345 bp, Rattus norvegicus
  source 1..345: mol_type = genomic DNA
gaggtgcacctggtggagtctgggggaggcttagtgcagcctggaaggtccatgaaactctcctgtacagcctcaggattcactttcaataactattacatggcctgggtccgtcaggctccaacgaagggtctggagtgggtcgcgtccattagtactggtggtggttacacttactatcgagactccgtgaagggccgatttactatctccagagataatacaggaaacaccctgtatctgcaaatggacagtctgaggtctgaggacacggccacttattactgtgcaagatgttgggagctgccttattggggccaaggagtcatggtcacagtctcctca

SEQ ID NO: 50 - protein, 125 aa, Rattus norvegicus
EVQLVETGGGLVQPGSSLKLSCSTSGFTFSETWMSWVRQAPGKGLEWVGLIKDKNSNYEANYAESVKGRFTISRDDSKRRVYLQMYTLRDQDTATYYCTSHEDFYYYSSYYFDYWGQGVMVTVSS

SEQ ID NO: 51 - DNA, 375 bp, Rattus norvegicus
  source 1..375: mol_type = genomic DNA
gaggtgcagctcgtggagacaggaggaggcttggtgcagcctgggagttctctaaaactctcctgttcaacctctggatttacattcagtgaaacctggatgagctgggttcgccaggctccagggaaggggctcgagtgggttggtctaattaaagataaaaatagtaattatgaagcaaactatgcagagtctgtcaaaggcagattcaccatctcaagagacgattcgaaacgcagagtctacttacagatgtacaccttaagggatcaggacactgccacttattactgtacaagtcacgaggatttttattactacagcagctattactttgattactggggccaaggagtcatggtcacagtctcctca

SEQ ID NO: 52 - protein, 115 aa, Rattus norvegicus
EVQLQQSGPEFVRPGTSVKFSCKVSGGSITSYFIHFVKQRPGQGLEWIGKIDPEDDSTKYGEKFKNKATLTADTSSNTAFLKLSSLTSEDTAIYFCTTLTGLDYWGQGVMVTVSS

SEQ ID NO: 53 - DNA, 345 bp, Rattus norvegicus
  source 1..345: mol_type = genomic DNA
gaagtccagctgcagcagtctgggcctgagtttgtgaggcctgggacctctgtgaagttttcttgcaaagtctctggcggttccattacatcatacttcatacactttgtgaaacaaaggcctggacagggtctggaatggataggaaagattgatcctgaggatgatagtactaaatatggtgagaagttcaaaaacaaggcgacactcactgccgatacatcctccaacacagccttcctgaagctcagcagcctgacctctgaggacactgcaatctatttttgcaccactctaactggccttgattactggggccaaggagtcatggtcacagtctcctca

SEQ ID NO: 54 - protein, 118 aa, Rattus norvegicus
EVQVVESGGGLVQPGRSMKLSCAALGFTFRDYYMAWVRQTPTKGLEWVAAISTGGGNTYYRDSVKGRFTISRDNAKSTLYLKMDSLRSDDTATYYCARNPYGNYFDYWGQGVMVTVSS

SEQ ID NO: 55 - DNA, 354 bp, Rattus norvegicus
  source 1..354: mol_type = genomic DNA
gaggtgcaggtggtggagtctgggggaggcttagtgcagcctggaaggtccatgaaactctcctgtgcagccttaggattcactttccgtgactattacatggcctgggtccgccagacaccaacaaagggtctggagtgggtcgcagccattagtactggtggtggaaacacttactatcgagactccgtgaagggccgattcactatctccagagataatgcaaaaagcaccctttatctgaaaatggacagtctgaggtctgacgacacggccacttattactgtgcaagaaacccctacggcaactactttgattattggggccaaggagtcatggtcacagtctcctct

SEQ ID NO: 56 - protein, 121 aa, Rattus norvegicus
EVQLVGSGGGLVQPGRSMKLSCEASGFTFSNHYMAWVRQAPTKGLEWVATISTGGGNTYYRDSVKGRFTISRDNARSILSLQMDSLRSEDTATYYCARQDYSNYMGGFAYWGQGTLVTVSS

SEQ ID NO: 57 - DNA, 363 bp, Rattus norvegicus
  source 1..363: mol_type = genomic DNA
gaggtgcagctggtggggtctgggggaggcttagtgcagcctggaaggtccatgaaactctcctgtgaagcctcaggattcactttcagtaaccattacatggcctgggtccgccaggcaccaacaaagggtctggagtgggtcgcgaccattagtactggtggtggtaatacttactatcgagactccgtgaagggccgattcactatctccagagataatgcaagaagcattctatccctacagatggacagtctgaggtctgaggacacggccacttattactgtgcaagacaagattatagtaactatatgggggggtttgcttactggggccagggcactctggtcactgtctcttca

SEQ ID NO: 58 - protein, 125 aa, Rattus norvegicus
EVQLVETGGGLVQPGSSLKLSCATSGFTFSDTWMSWVRQAPGKGLEWVALIKDKNSNYEANYAESVKGRFTISRDDSKRRVYLQMFTLRDQDTATYYCTSHEDFYYYSSYYFDYWGHGVMVTVSS

SEQ ID NO: 59 - DNA, 375 bp, Rattus norvegicus
  source 1..375: mol_type = genomic DNA
gaggtgcagctcgtggagacaggaggaggcttggtgcagcctgggagttctctaaaactctcctgtgcaacctctggatttacattcagtgacacctggatgagctgggttcgccaggctccagggaaggggctcgagtgggttgctctaattaaagataaaaatagtaattatgaagcaaactatgcagagtctgtaaaaggcagattcaccatctcaagagacgattcgaaacgcagagtctacttacagatgttcaccttacgggatcaggacactgccacttattactgtacaagtcacgaggatttttattactatagcagctattactttgattactggggccacggagtcatggtcacagtctcctca

SEQ ID NO: 60 - protein, 115 aa, Rattus norvegicus
EVQLQQSGAGLVRPRTSVRLSCKISGDSITAYYVHFVKQRPGQGLEWIGRIDPEDDSTKYSEKFKNKATLTADVSSSTAYLILSSLTSDDSATYFCSTLTGLDYWGQGVMVTVSS

SEQ ID NO: 61 - DNA, 345 bp, Rattus norvegicus
  source 1..345: mol_type = genomic DNA
gaagtccagctgcagcagtctggggctggacttgtgagacctaggacctctgtgaggttatcttgcaaaatttctggcgattccattacagcatattacgtgcactttgtgaaacaaaggcctggacagggtctggaatggataggaagaattgatcctgaggatgatagtactaaatattctgagaagttcaaaaacaaggcgacactcactgcagatgtatcctccagcacagcctacctgattctcagcagcctgacctctgacgactctgcaacctatttttgttccactctgactggccttgattactggggccagggagtcatggtcacggtctcctca

SEQ ID NO: 62 - protein, 125 aa, Rattus norvegicus
EVQLVETGGGLVRPGSSLKLSCATSGFTFSDTWMSWVRQAPGKGLEWVALIKDKNSNSEANYAESIKGRFTISRDDSKSRVYLQMNTLRDQDTATYYCTRHEDFYYYSGYYFDYWGQGVMVTVSS

SEQ ID NO: 63 - DNA, 375 bp, Rattus norvegicus
  source 1..375: mol_type = genomic DNA
gaggtgcagctcgtggagacaggaggaggcttggtgcggcctgggagttctctaaaactctcctgtgcaacctctggatttacattcagtgacacctggatgagctgggttcgccaggctccagggaaggggctcgagtgggttgctctaattaaagataaaaatagtaattctgaagcaaactatgcagagtctataaaaggcagattcaccatctcaagagacgattcgaaaagcagagtctacttacagatgaacaccttaagggatcaggacactgccacttattactgtacaaggcacgaggatttttattactatagtggctattactttgattactggggccaaggagtcatggtcacagtctcctca

SEQ ID NO: 64 - protein, 118 aa, Rattus norvegicus
QVQLQQSGVELAKPGSSVKISCKASGNTFTSNYITWIKQTPGQGLEYIGYINTGSGKTYYNEKFKGKATLTADKSSSTAFMQLSSLTPDDSAVYFCASLTGVDYFDDWGQGVMVTVSS

SEQ ID NO: 65 - DNA, 354 bp, Rattus norvegicus
  source 1..354: mol_type = genomic DNA
caggtccagctgcagcagtctggagttgagctggcaaagcctggctcttcagtgaagatctcctgtaaggcctctggcaacaccttcaccagcaattatataacctggataaagcagacgcctggacagggccttgagtatattggatatattaatacgggaagtggaaaaacttactacaatgagaagttcaagggcaaggccacattgactgcagacaaatcctccagcacagccttcatgcaactcagcagcctgacacctgacgactctgcggtctatttctgtgcaagtctaactggggtcgactactttgatgactggggccaaggagtcatggtcacagtctcctca

SEQ ID NO: 66 - protein, 110 aa, Rattus norvegicus
QFVLTQPNSVSTNLGSTVKLSCTRSIGNIGNNYVNWYKQYEGRSPTTLIYRDDERPDGVPDRFSGSIDRSSNSALLTINSVQTEDGADYFCQSFSSGIFIFGGGTTLTVL

SEQ ID NO: 67 - DNA, 330 bp, Rattus norvegicus
  source 1..330: mol_type = genomic DNA
cagtttgtacttacgcagccaaactctgtgtctacgaatctcggaagcacagtcaaactgtcttgcacgcgcagcattggtaacattggaaacaattatgtgaactggtacaagcagtatgagggaagatctcccaccactctgatttatagggatgatgagagaccagatggagttcctgacaggttctctggctccattgacagatcttccaactcagccctcctgacaatcaatagtgtgcagactgaagatggagctgactacttctgtcagtctttcagtagtggtatctttatttttggcggtggaaccacgctcactgtcctg

SEQ ID NO: 68 - protein, 109 aa, Rattus norvegicus
QVVLTQPNSVSTNLGSTVKLSCKRTTGNIGSNYVNWYQQHEGRSPTTMIYRDDERPDGVPDRFSGSIDRSSNSALLTINNVQTEDEAEYFCQSYSSGIIFGGGTKLTVL

SEQ ID NO: 69 - DNA, 327 bp, Rattus norvegicus
  source 1..327: mol_type = genomic DNA
caggtggtgcttactcagccaaactctgtgtctacgaatctcggaagcacagtcaaactgtcttgcaagcgcaccactggtaacattggtagcaattatgtgaactggtatcagcagcatgagggaagatctcccaccactatgatttatagggatgatgagagaccagatggagttcctgacaggttctctggctccattgacagatcgtccaactcagccctcctgacaatcaataatgtgcagactgaagatgaagctgaatacttctgtcagtcttacagtagtggtattattttcggcggtggaaccaagctcactgtccta

SEQ ID NO: 70 - protein, 107 aa, Rattus norvegicus
DIQMTQSPPVLSTSVGDRVTLRCKPSQNVHSKLDWYQQKHGEAPKLLIYYTHNLQTGIPSRFSGSGSGTDYTLTISSLQPEDVATYYCFQYYSGWTFGGGTKLEMKR

SEQ ID NO: 71 - DNA, 321 bp, Rattus norvegicus
  source 1..321: mol_type = genomic DNA
gacatccagatgacccagtctcctccagtcctgtctacatctgtgggagacagagtcactctcaggtgcaaaccaagtcagaatgttcatagcaagttagactggtatcagcagaaacatggagaggctccgaaactcctgatatattatacacacaatttgcaaacgggcatcccatcaaggttcagtggcagtggatccggtacagattacaccctcaccatcagcagcctgcagcctgaagatgttgccacatattactgttttcaatattacagtgggtggacgttcggtggaggcaccaagctggaaatgaaacgg

SEQ ID NO: 72 - protein, 110 aa, Rattus norvegicus
QFVLTQPNSVSTNLGSTVKLSCKRSTGNIGNNYVNWYQQYEGRSPTTMIYRDDERPDGVPDRFSGSIDRSSNSALLTINNVQTEDEADYFCQSFSNGMFIFAGGTQLTVL

SEQ ID NO: 73 - DNA, 330 bp, Rattus norvegicus
  source 1..330: mol_type = genomic DNA
cagtttgtacttactcagccaaactctgtgtctacgaatctcggaagcacagtcaaactgtcttgcaagcgcagcactggtaacattggaaacaattatgtgaactggtaccagcagtatgagggaagatctcccactactatgatttatagggatgatgagagaccagatggagttcctgacaggttctctggctccattgacagatcttccaactcagccctcctgacaatcaataatgtgcagactgaggatgaagctgactacttctgtcagtctttcagtaacggtatgtttatttttgccggtggaacccagctcactgtccta

SEQ ID NO: 74 - protein, 110 aa, Rattus norvegicus
QFVLTQPNSVSTNLGSTVKLSCTRSIGNIGNNYVNWYKQYEGRSPTTMIYRDDERPDGVPDRFSGSIDRSSNSALLTINSVQTEDEADYFCQSFSSGIFIFGGGTKLTVL

SEQ ID NO: 75 - DNA, 330 bp, Rattus norvegicus
  source 1..330: mol_type = genomic DNA
cagtttgtacttacgcagccaaactctgtgtctacgaatctcggaagcacagtcaaactgtcttgcacgcgcagcattggtaacattggaaacaattatgtgaattggtacaagcagtatgagggaagatctcccaccactatgatttatagggatgatgagagaccagatggagttcctgacaggttctctggctccattgacagatcttccaactcagccctcctgacaatcaatagtgtgcagactgaagatgaagctgactacttctgtcagtctttcagtagtggtatctttatttttggcggtggaaccaagctcactgtccta

SEQ ID NO: 76 - protein, 107 aa, Rattus norvegicus
DIQMTQSPPVLSTSVGDRVTLRCKASQNVHSKLDWYQQKHGEAPKLLIYYTHNLQTGIPSRFSGSGSGTDYTLTISSLQPEDVATYYCFQYYSGWTFGGGTKLEMKR

SEQ ID NO: 77 - DNA, 321 bp, Rattus norvegicus
  source 1..321: mol_type = genomic DNA
gacatccagatgacccagtctcctccagtcctgtctacatctgtgggagacagagtcactctcaggtgcaaagcaagtcagaatgttcatagtaagttagactggtatcagcagaaacatggagaggctccgaaactcctgatatattatacacacaatttgcaaacgggcatcccatcaaggttcagtggcagtggatccggtacagattacaccctcaccatcagcagcctgcagcctgaagatgttgccacatattactgttttcaatattacagtgggtggacgttcggtggaggcaccaagctggaaatgaaacgg

SEQ ID NO: 78 - protein, 110 aa, Rattus norvegicus
QFVLSQPNSVSTNLGSTVKLSCKRSTGNIGSNYVHWYQRHEGRSPTTLIYRDDKRPNGVPDRFSGSIDRSSNSALLTINNVQTEDEADYFCQSYSGGMYLFGGGTKLTVL

SEQ ID NO: 79 - DNA, 330 bp, Rattus norvegicus
  source 1..330: mol_type = genomic DNA
cagtttgtgcttagtcagccaaactctgtgtcgacgaatctcggaagcacagtcaaactgtcttgcaagcgcagcactggtaacattggaagcaattatgtgcactggtaccagcgacatgagggaagatctcccaccactctgatttatagggatgataagagaccaaatggagttcctgacaggttttctggctccattgacagatcttccaactcagccctcctgacaatcaataatgtgcagactgaagatgaagctgactacttctgtcagtcttacagtggtggtatgtatcttttcggcggtggaaccaagctcactgtccta

SEQ ID NO: 80 - protein, 110 aa, Rattus norvegicus
QFVLTQPNSVSTNLGSTVKLSCRRSSGNIGNNYVNWYRQHEGRSPTTMIYRDDTRPDGVPNRFSGSIDRSSNSALLTINNVRPEDEAYYFCQSYSGSIYIFGGGTKLTVL

SEQ ID NO: 81 - DNA, 330 bp, Rattus norvegicus
  source 1..330: mol_type = genomic DNA
cagtttgtgcttactcagccaaactctgtgtctacgaatctcggaagcacagtcaaactgtcttgcaggcgcagcagtggtaacattggaaacaattatgtaaactggtaccgacagcatgagggaagatctcccaccactatgatttatagggatgatacgagaccagatggagttcctaacaggttctctggctccattgacagatcttccaactcagccctcctgacaatcaataatgtgcggcctgaggatgaagcttactacttctgtcagtcttacagtggtagtatctatattttcggcggtgggaccaagctcactgtcctg

SEQ ID NO: 82 - protein, 108 aa, Rattus norvegicus
DIVLTQSPATLSVTPGESVSLSCRASQGISTSIHWYQQKSNESPRLLIKYASQSMSGIPSRFSGSGSGTDFTLRINRVESEDFSVYYCQQSYNLPLTFGSGTKLEIKR

SEQ ID NO: 83 - DNA, 324 bp, Rattus norvegicus
  source 1..324: mol_type = genomic DNA
gacatcgtgctgactcagtctccagccaccctgtctgtgactccaggagagagtgtgagtctctcgtgcagggccagtcagggtattagtactagcatacactggtatcagcaaaaatcaaatgagtctccaaggcttctcatcaagtatgcttcccagtccatgtctggaatcccctccaggttcagtggcagtggatcagggacagatttcactctcagaatcaacagagtagaatctgaggatttttcagtttattactgtcaacagagttacaacttgcccctcacgttcggctcagggacgaagttggaaataaaacgg

SEQ ID NO: 84 - protein, 107 aa, Rattus norvegicus
DIQMTQSPPVLSAAVGDRVTLSCKASRSLNKNLDWYQQKHGETPKLLIYHTHNLQTGIPSRFSGSGSDTDYTLTISSLQTEDVATYYCYQYHSGWTFGGGTRLELRR

SEQ ID NO: 85 - DNA, 321 bp, Rattus norvegicus
  source 1..321: mol_type = genomic DNA
gacatccagatgacccagtctcctccagtcctgtctgcagctgtgggagacagagtcactctcagctgcaaagcaagtcggagtcttaataagaacttagactggtatcagcaaaagcatggagaaactccaaaactcctgatatatcatacacacaatttgcaaacgggcatcccttcgaggttcagtggcagtggatctgatactgattacacactcaccatcagtagcctgcagactgaagatgttgccacatattactgctatcagtatcacagtgggtggacgttcggtgggggcaccaggctggaattgagacgg

SEQ ID NO: 86 - protein, 110 aa, Rattus norvegicus
QFVLSQPNSVSTNLGSTVKLSCKRSTGNIGSNYVHWYQRHEGRSPTTMIYRDDKRPNGVPDRFSGSIDRSSNSALLTINNVQTEDEADYFCQSYSGGMYLFGGGTTLTVL

SEQ ID NO: 87 - DNA, 330 bp, Rattus norvegicus
  source 1..330: mol_type = genomic DNA
cagtttgtgcttagtcagccaaactctgtgtcgacgaatctcggaagcacagtcaaactgtcttgcaagcgcagcactggtaacattggaagcaattatgtgcactggtaccagcgacatgagggaagatctcccaccactatgatttatagggatgataagagaccaaacggagttcctgacaggttttctggctccattgacagatcttccaactcagccctcctgacaatcaataatgtgcagactgaagatgaagctgactacttctgtcagtcttacagtggtggtatgtatcttttcggcggtggaaccacgctcactgtccta

SEQ ID NO: 88 - protein, 110 aa, Rattus norvegicus
QFVLTQPNSVSTNLGSTVKLSCTRSIGNIGNNYVNWYKQYEGRSPTTMIYRDDERPDGVPDRFSGSIDRSSNSALLTINNVQTEDEADYFCQSFSSGMFIFGGGTKLTVL

SEQ ID NO: 89 - DNA, 330 bp, Rattus norvegicus
  source 1..330: mol_type = genomic DNA
cagtttgtacttacgcagccaaactctgtgtctacgaatctcggaagcacagtcaaactgtcttgcacgcgcagcattggtaacattggaaacaattatgtgaactggtataagcagtatgagggaagatctcccaccactatgatttatagggatgatgagagaccagatggagttcctgacaggttctctggctccattgacagatcttccaactcagccctcctgacaatcaataatgtgcagactgaagatgaagctgactacttctgtcagtctttcagtagtggtatgtttatttttggcggtggaaccaaactcactgtccta

SEQ ID NO: 90 - protein, 108 aa, Rattus norvegicus
DIVLTQSPATLSVTPGESVSLSCRASQGISTSIHWYQQKSNGSPRLLIKYASQSISGIPSRFSGSGSGTDFTLRINRVESEDFSVYYCQQTYSLPLTFGSGTRLEIKR

SEQ ID NO: 91 - DNA, 324 bp, Rattus norvegicus
  source 1..324: mol_type = genomic DNA
gacatcgtgctgactcagtctccagccaccctgtctgtgactccaggagagagtgtgagtctctcctgcagggccagtcagggtattagtactagcattcactggtatcagcaaaaatcaaatgggtctccaaggcttctcatcaagtatgcttcccagtccatctctggaatcccctccaggttcagtggcagtggatcagggacagatttcactctcagaatcaacagagtagaatctgaagatttttcagtttattactgtcaacagacttacagcttgcccctcacgttcggctcagggacgaggttggaaataaaacgg

SEQ ID NO: 92 - protein, 107 aa, Rattus norvegicus
DIQMTQSPPVLSASVGDRVTLSCKASQSVHNKLDWYQQKHGEAPKLLIYYTHNLQTGIPSRFSGSGSGSDYTLTISSLRAEDVATYYCFQYYSGWTFGGGTKLEMKR

SEQ ID NO: 93 - DNA, 321 bp, Rattus norvegicus
  source 1..321: mol_type = genomic DNA
gacatccagatgacccagtctcccccagtcctgtctgcatctgtgggagacagagtcactctcagctgcaaagcaagtcagagtgttcataacaagttagactggtatcagcaaaagcatggagaggctccgaaactcctgatttattatacacacaatttacaaacgggcatcccatcaaggttcagtggcagtggatccggttcagattacacactcaccatcagcagcctgcgggctgaagatgttgccacatattactgttttcaatattacagtgggtggacgttcggtggaggcaccaagctggaaatgaaacgg

SEQ ID NO: 94 - protein, 108 aa, Rattus norvegicus
DIVLTQSPPTLSVTPGESVSLSCRASQGISTSIHWYQQRSNESPRLLIKYASQSIAGIPSRFSGSGSGTDFILSINRVESEDFSVYYCQQTYSLPLTFGPGTKLEVKR

SEQ ID NO: 95 - DNA, 324 bp, Rattus norvegicus
  source 1..324: mol_type = genomic DNA
gacatcgtgctgactcagtctccacccaccctgtctgtgactccaggagagagtgtgagtctctcctgcagggccagtcagggtattagtactagcatacactggtatcaacaaagatcaaatgagtctccaaggcttctcatcaagtatgcttcccagtccattgctggaatcccctccaggttcagtggcagtggatcagggacagatttcatcctcagtatcaacagagtagaatctgaagatttttcagtttattactgtcaacagacttacagcttgcccctcacgttcggcccagggacgaagttggaagtaaaacgg

SEQ ID NO: 96 - protein, 112 aa, Rattus norvegicus
DDIVLTQSPALAPSLGQRATISCRASQSVRMSGYNLMHWYQQKPGQQPKLLIYDASKLASGIPARFSGSGSGTDFTLTIDPVQSDDIATYYCQQSKDDPYTFGAGTKLELRR

SEQ ID NO: 97 - DNA, 336 bp, Rattus norvegicus
  source 1..336: mol_type = genomic DNA
gatgacattgtgctgacccagtctccagctttggctccgtctctagggcagagggccacaatctcctgtagagccagccaaagtgtcaggatgtctggctataatctcatgcactggtaccaacagaaaccaggacaacagcccaaactcctcatctatgatgcatccaagctagcatctgggatccctgccaggttcagtggcagtgggtctgggacagacttcaccctcaccattgatcctgtgcagtctgatgatattgcaacctattactgtcagcagagtaaggatgatccgtacacgtttggagctgggaccaagctggaactgcgacgg

SEQ ID NO: 98 - protein, 5 aa, Rattus norvegicus
NHYMA

SEQ ID NO: 99 - protein, 5 aa, Rattus norvegicus
NYYMT

SEQ ID NO: 100 - protein, 5 aa, Rattus norvegicus
RYYVH

SEQ ID NO: 101 - protein, 5 aa, Rattus norvegicus
DYYMA

SEQ ID NO: 102 - protein, 5 aa, Rattus norvegicus
NYYMA

SEQ ID NO: 103 - protein, 5 aa, Rattus norvegicus
ETWMS

SEQ ID NO: 104 - protein, 5 aa, Rattus norvegicus
SYFIH

SEQ ID NO: 105 - protein, 5 aa, Rattus norvegicus
DTWMS

SEQ ID NO: 106 - protein, 5 aa, Rattus norvegicus
AYYVH

SEQ ID NO: 107 - protein, 5 aa, Rattus norvegicus
SNYIT

SEQ ID NO: 108 - protein, 17 aa, Rattus norvegicus
TISTGGGNTYYRDSVKG

SEQ ID NO: 109 - protein, 17 aa, Rattus norvegicus
SISSSGGNTYYRDSVRG

SEQ ID NO: 110 - protein, 17 aa, Rattus norvegicus
RIDPEDDTTKYSEKFKN

SEQ ID NO: 111 - protein, 17 aa, Rattus norvegicus
SISTGGGNTYYRDSVKG

SEQ ID NO: 112 - protein, 17 aa, Rattus norvegicus
RIDPEDDTTKYSEKFKK

SEQ ID NO: 113 - protein, 17 aa, Rattus norvegicus
AISTGGGNTYYRDSVKG

SEQ ID NO: 114 - protein, 17 aa, Rattus norvegicus
SISTGGGYTYYRDSVKG

SEQ ID NO: 115 - protein, 19 aa, Rattus norvegicus
LIKDKNSNYEANYAESVKG

SEQ ID NO: 116 - protein, 17 aa, Rattus norvegicus
KIDPEDDSTKYGEKFKN

SEQ ID NO: 117 - protein, 17 aa, Rattus norvegicus
RIDPEDDSTKYSEKFKN

SEQ ID NO: 118 - protein, 19 aa, Rattus norvegicus
LIKDKNSNSEANYAESIKG

SEQ ID NO: 119 - protein, 17 aa, Rattus norvegicus
YINTGSGKTYYNEKFKG

SEQ ID NO: 120 - protein, 12 aa, Rattus norvegicus
QDYTNYMGGFAY

SEQ ID NO: 121 - protein, 10 aa, Rattus norvegicus
EGYRGRYFDY

SEQ ID NO: 122 - protein, 6 aa, Rattus norvegicus
LTGLDY

SEQ ID NO: 123 - protein, 12 aa, Rattus norvegicus
QDYSNYMGGFAY

SEQ ID NO: 124 - protein, 9 aa, Rattus norvegicus
NPYGNYFDY

SEQ ID NO: 125 - protein, 6 aa, Rattus norvegicus
CWELPY

SEQ ID NO: 126 - protein, 14 aa, Rattus norvegicus
HEDFYYYSSYYFDY

SEQ ID NO: 127 - protein, 14 aa, Rattus norvegicus
HEDFYYYSGYYFDY

SEQ ID NO: 128 - protein, 9 aa, Rattus norvegicus
LTGVDYFDD

SEQ ID NO: 129 - protein, 13 aa, Rattus norvegicus
TRSIGNIGNNYVN

SEQ ID NO: 130 - protein, 13 aa, Rattus norvegicus
KRTTGNIGSNYVN

SEQ ID NO: 131 - protein, 11 aa, Rattus norvegicus
KPSQNVHSKLD

SEQ ID NO: 132 - protein, 13 aa, Rattus norvegicus
KRSTGNIGNNYVN

SEQ ID NO: 133 - protein, 11 aa, Rattus norvegicus
KASQNVHSKLD

SEQ ID NO: 134 - protein, 13 aa, Rattus norvegicus
KRSTGNIGSNYVH

SEQ ID NO: 135 - protein, 13 aa, Rattus norvegicus
RRSSGNIGNNYVN

SEQ ID NO: 136 - protein, 11 aa, Rattus norvegicus
RASQGISTSIH

SEQ ID NO: 137 - protein, 11 aa, Rattus norvegicus
KASRSLNKNLD

SEQ ID NO: 138 - protein, 11 aa, Rattus norvegicus
KASQSVHNKLD

SEQ ID NO: 139 - protein, 15 aa, Rattus norvegicus
RASQSVRMSGYNLMH

SEQ ID NO: 140 - protein, 7 aa, Rattus norvegicus
RDDERPD

SEQ ID NO: 141 - protein, 7 aa, Rattus norvegicus
YTHNLQT

SEQ ID NO: 142 - protein, 7 aa, Rattus norvegicus
RDDKRPN

SEQ ID NO: 143 - protein, 7 aa, Rattus norvegicus
RDDTRPD

SEQ ID NO: 144 - protein, 7 aa, Rattus norvegicus
YASQSMS

SEQ ID NO: 145 - protein, 7 aa, Rattus norvegicus
HTHNLQT

SEQ ID NO: 146 - protein, 7 aa, Rattus norvegicus
YASQSIS

SEQ ID NO: 147 - protein, 7 aa, Rattus norvegicus
YASQSIA

SEQ ID NO: 148 - protein, 7 aa, Rattus norvegicus
DASKLAS

SEQ ID NO: 149 - protein, 9 aa, Rattus norvegicus
QSFSSGIFI

SEQ ID NO: 150 - protein, 8 aa, Rattus norvegicus
QSYSSGII

SEQ ID NO: 151 - protein, 9 aa, Rattus norvegicus
FQYYSGWTF

SEQ ID NO: 152 - protein, 9 aa, Rattus norvegicus
QSFSNGMFI

SEQ ID NO: 153 - protein, 9 aa, Rattus norvegicus
QSYSGGMYL

SEQ ID NO: 154 - protein, 9 aa, Rattus norvegicus
QSYSGSIYI

SEQ ID NO: 155 - protein, 9 aa, Rattus norvegicus
QQSYNLPLT

SEQ ID NO: 156 - protein, 9 aa, Rattus norvegicus
YQYHSGWTF

SEQ ID NO: 157 - protein, 9 aa, Rattus norvegicus
QSFSSGMFI

SEQ ID NO: 158 - protein, 9 aa, Rattus norvegicus
QQTYSLPLT

SEQ ID NO: 159 - protein, 9 aa, Rattus norvegicus
QQSKDDPYT

SEQ ID NO: 160 - protein, 557 aa, synthetic construct
  REGION 1..557: note = Homo sapiens
MMCLECASAAAGGAEEEEADAERRRRRRGAQRGAGGSGCCGARGAGGAGVSAAGDEVQTLSGSVRRAPTGPPGTPGTPGCAATAKGPGAQQPKPASLGRGRGAAAAILSLGNVLNYLDRYTVAGVLLDIQQHFDYKDDDDKGVKDRGAGLLQSVFICSFMVAAPIFGYLGDRFNRKVILSCGIFFWSAVTFSSSFIPQQYFWLLVLSRGLVGIGEASYSTIAPTIIGDLFTKNTRTLMLSVFYFAIPLGSGLGYITGSSVKQAAGDWHWALRVSPVLGMITGTLILILVPATKRGHADQLGDQLKARTSWLRDMKALIRNRSYVFSSLATSAVSFATGALGMWIPLYLHRAQVVQKTAETCNSPPCGAKDSLIFGAITCFTGFLGVVTGAGATRWCRLKTQRADPLVCAVGMLGSAIFICLIFVAAKSSIVGAYICIFVGETLLFSNWAITADILMYVVIPTRRATAVALQSFTSHLLGDAGSPYLIGFISDLIRQSTKDSPLWEFLSLGYALMLCPFVVVLGGMFFLATALFFVSDRARAEQQVNQLAMPPASVKV

SEQ ID NO: 161 - DNA, 1674 bp, synthetic construct
  misc_feature 1..1674: note = Homo sapiens
  source 1..1674: mol_type = other DNA
atgatgtgcctggaatgcgcctcggcggcggcgggcggcgcggaggaggaggaggcggacgcggagcggcggcgccggcgccggggggcgcagcgaggggctggcggtagcggttgctgcggggcgcggggcgcgggcggcgctggagtctcggccgcgggcgatgaggtgcagacgctgtcgggcagcgtaaggcgggccccgaccggaccccccggcacccccggcacccccggctgcgcagctactgcaaagggccccggcgctcagcagcccaaaccggccagcttgggccgcgggcggggggcagccgccgccatcctcagcttgggcaacgtgctcaactacctggacaggtacaccgtggcaggcgtccttctggacatccagcagcactttgattacaaggatgacgacgataagggggtcaaggaccgaggcgccggcctgctgcagtcagtgttcatctgtagcttcatggtggctgcccccatcttcggctacctgggcgaccgcttcaacaggaaggtgattctcagctgcggcattttcttctggtcggccgtcaccttctccagctccttcattccccagcagtacttctggctgctggtcctgtcccgggggctggtgggcatcggggaggccagctactccaccatcgcccccactatcattggcgacctcttcaccaagaacacgcgtacgctcatgctgtccgtcttctacttcgccatcccactgggcagtggcctgggctacattactggctccagcgtgaagcaggcagccggagactggcactgggcattgcgggtgtcccctgtcctgggcatgatcacaggaacactcatcctcattctggtcccagccactaaaaggggtcatgccgaccagctcggggaccagctcaaggcccggacctcatggctccgagatatgaaggccctgattcgaaaccgcagctacgtcttctcctccctggccacgtcggctgtctccttcgccacgggggccctgggcatgtggatcccgctctacctgcaccgcgcccaagttgtgcagaagacagcagagacgtgcaacagcccgccctgtggggccaaggacagcctcatctttggggccatcacctgctttacgggatttctgggcgtggtcacgggggcaggagccacgcgctggtgccgcctgaagacccagcgggccgacccactggtgtgtgccgtgggcatgctgggctctgccatcttcatctgcctgatcttcgtggctgccaagagcagcatcgtaggagcctatatctgtatcttcgtcggggagacgctgctgttttctaactgggccatcactgcagacatcctcatgtacgtggtcatccccacgcggcgcgccactgccgtggccttgcagagcttcacctcccacctgctgggggacgccgggagcccctacctcattggctttatctcagacctgatccgccagagcactaaggactccccgctctgggagttcctgagcctgggctacgcgctcatgctctgccctttcgtcgtggtcctgggcggcatgttcttcctcgccactgcgctcttcttcgtcagcgaccgcgccagggctgagcagcaggtgaaccagctggcgatgccgcccgcatctgtgaaagtctga

SEQ ID NO: 162 - protein, 557 aa, synthetic construct
  REGION 1..557: note = Homo sapiens
MMCLECASAAAGGAEEEEADAERRRRRRGAQRGAGGSGCCGARGAGGAGVSAAGDEVQTLSGSVRRAPTGPPGTPGTPGCAATAKGPGAQQPKPASLGRGRGAAAAILSLGNVLNYLDRYTVAGVLLDIQQHFGVKDRGAGLLQSVFICSFMVAAPIFGYLGDRFNRKVILSCGIFFWSAVTFSSSFIPQQYFWLDYKDDDDKLVLSRGLVGIGEASYSTIAPTIIGDLFTKNTRTLMLSVFYFAIPLGSGLGYITGSSVKQAAGDWHWALRVSPVLGMITGTLILILVPATKRGHADQLGDQLKARTSWLRDMKALIRNRSYVFSSLATSAVSFATGALGMWIPLYLHRAQVVQKTAETCNSPPCGAKDSLIFGAITCFTGFLGVVTGAGATRWCRLKTQRADPLVCAVGMLGSAIFICLIFVAAKSSIVGAYICIFVGETLLFSNWAITADILMYVVIPTRRATAVALQSFTSHLLGDAGSPYLIGFISDLIRQSTKDSPLWEFLSLGYALMLCPFVVVLGGMFFLATALFFVSDRARAEQQVNQLAMPPASVKV

SEQ ID NO: 163 - DNA, 1674 bp, synthetic construct
  misc_feature 1..1674: note = Homo sapiens
  source 1..1674: mol_type = other DNA
atgatgtgcctggaatgcgcctcggcggcggcgggcggcgcggaggaggaggaggcggacgcggagcggcggcgccggcgccggggggcgcagcgaggggctggcggtagcggttgctgcggggcgcggggcgcgggcggcgctggagtctcggccgcgggcgatgaggtgcagacgctgtcgggcagcgtaaggcgggccccgaccggaccccccggcacccccggcacccccggctgcgcagctactgcaaagggccccggcgctcagcagcccaaaccggccagcttgggccgcgggcggggggcagccgccgccatcctcagcttgggcaacgtgctcaactacctggacaggtacaccgtggcaggcgtccttctggacatccagcagcactttggggtcaaggaccgaggcgccggcctgctgcagtcagtgttcatctgtagcttcatggtggctgcccccatcttcggctacctgggcgaccgcttcaacaggaaggtgattctcagctgcggcattttcttctggtcggccgtcaccttctccagctccttcattccccagcagtacttctggctggattacaaggatgacgacgataagctggtcctgtcccgggggctggtgggcatcggggaggccagctactccaccatcgcccccactatcattggcgacctcttcaccaagaacacgcgtacgctcatgctgtccgtcttctacttcgccatcccactgggcagtggcctgggctacattactggctccagcgtgaagcaggcagccggagactggcactgggcattgcgggtgtcccctgtcctgggcatgatcacaggaacactcatcctcattctggtcccagccactaaaaggggtcatgccgaccagctcggggaccagctcaaggcccggacctcatggctccgagatatgaaggccctgattcgaaaccgcagctacgtcttctcctccctggccacgtcggctgtctccttcgccacgggggccctgggcatgtggatcccgctctacctgcaccgcgcccaagttgtgcagaagacagcagagacgtgcaacagcccgccctgtggggccaaggacagcctcatctttggggccatcacctgctttacgggatttctgggcgtggtcacgggggcaggagccacgcgctggtgccgcctgaagacccagcgggccgacccactggtgtgtgccgtgggcatgctgggctctgccatcttcatctgcctgatcttcgtggctgccaagagcagcatcgtaggagcctatatctgtatcttcgtcggggagacgctgctgttttctaactgggccatcactgcagacatcctcatgtacgtggtcatccccacgcggcgcgccactgccgtggccttgcagagcttcacctcccacctgctgggggacgccgggagcccctacctcattggctttatctcagacctgatccgccagagcactaaggactccccgctctgggagttcctgagcctgggctacgcgctcatgctctgccctttcgtcgtggtcctgggcggcatgttcttcctcgccactgcgctcttcttcgtcagcgaccgcgccagggctgagcagcaggtgaaccagctggcgatgccgcccgcatctgtgaaagtctga

SEQ ID NO: 164 - protein, 557 aa, synthetic construct
  REGION 1..557: note = Homo Sapiens
MMCLECASAAAGGAEEEEADAERRRRRRGAQRGAGGSGCCGARGAGGAGVSAAGDEVQTLSGSVRRAPTGPPGTPGTPGCAATAKGPGAQQPKPASLGRGRGAAAAILSLGNVLNYLDRYTVAGVLLDIQQHFGVKDRGAGLLQSVFICSFMVAAPIFGYLGDRFNRKVILSCGIFFWSAVTFSSSFIPQQYFWLLVLSRGLVGIGEASYSTIAPTIIGDLFTKNTRTLMLSVFYFAIPLGSGLGYITGSSVKQADYKDDDDKAGDWHWALRVSPVLGMITGTLILILVPATKRGHADQLGDQLKARTSWLRDMKALIRNRSYVFSSLATSAVSFATGALGMWIPLYLHRAQVVQKTAETCNSPPCGAKDSLIFGAITCFTGFLGVVTGAGATRWCRLKTQRADPLVCAVGMLGSAIFICLIFVAAKSSIVGAYICIFVGETLLFSNWAITADILMYVVIPTRRATAVALQSFTSHLLGDAGSPYLIGFISDLIRQSTKDSPLWEFLSLGYALMLCPFVVVLGGMFFLATALFFVSDRARAEQQVNQLAMPPASVKV

SEQ ID NO: 165 - DNA, 1674 bp, synthetic construct
  misc_feature 1..1674: note = Homo sapiens
  source 1..1674: mol_type = other DNA
atgatgtgcctggaatgcgcctcggcggcggcgggcggcgcggaggaggaggaggcggacgcggagcggcggcgccggcgccggggggcgcagcgaggggctggcggtagcggttgctgcggggcgcggggcgcgggcggcgctggagtctcggccgcgggcgatgaggtgcagacgctgtcgggcagcgtaaggcgggccccgaccggaccccccggcacccccggcacccccggctgcgcagctactgcaaagggccccggcgctcagcagcccaaaccggccagcttgggccgcgggcggggggcagccgccgccatcctcagcttgggcaacgtgctcaactacctggacaggtacaccgtggcaggcgtccttctggacatccagcagcactttggggtcaaggaccgaggcgccggcctgctgcagtcagtgttcatctgtagcttcatggtggctgcccccatcttcggctacctgggcgaccgcttcaacaggaaggtgattctcagctgcggcattttcttctggtcggccgtcaccttctccagctccttcattccccagcagtacttctggctgctggtcctgtcccgggggctggtgggcatcggggaggccagctactccaccatcgcccccactatcattggcgacctcttcaccaagaacacgcgtacgctcatgctgtccgtcttctacttcgccatcccactgggcagtggcctgggctacattactggctccagcgtgaagcaggcagattacaaggatgacgacgataaggccggagactggcactgggcattgcgggtgtcccctgtcctgggcatgatcacaggaacactcatcctcattctggtcccagccactaaaaggggtcatgccgaccagctcggggaccagctcaaggcccggacctcatggctccgagatatgaaggccctgattcgaaaccgcagctacgtcttctcctccctggccacgtcggctgtctccttcgccacgggggccctgggcatgtggatcccgctctacctgcaccgcgcccaagttgtgcagaagacagcagagacgtgcaacagcccgccctgtggggccaaggacagcctcatctttggggccatcacctgctttacgggatttctgggcgtggtcacgggggcaggagccacgcgctggtgccgcctgaagacccagcgggccgacccactggtgtgtgccgtgggcatgctgggctctgccatcttcatctgcctgatcttcgtggctgccaagagcagcatcgtaggagcctatatctgtatcttcgtcggggagacgctgctgttttctaactgggccatcactgcagacatcctcatgtacgtggtcatccccacgcggcgcgccactgccgtggccttgcagagcttcacctcccacctgctgggggacgccgggagcccctacctcattggctttatctcagacctgatccgccagagcactaaggactccccgctctgggagttcctgagcctgggctacgcgctcatgctctgccctttcgtcgtggtcctgggcggcatgttcttcctcgccactgcgctcttcttcgtcagcgaccgcgccagggctgagcagcaggtgaaccagctggcgatgccgcccgcatctgtgaaagtctga

SEQ ID NO: 166 - protein, 557 aa, synthetic construct
  REGION 1..557: note = Homo sapiens
MMCLECASAAAGGAEEEEADAERRRRRRGAQRGAGGSGCCGARGAGGAGVSAAGDEVQTLSGSVRRAPTGPPGTPGTPGCAATAKGPGAQQPKPASLGRGRGAAAAILSLGNVLNYLDRYTVAGVLLDIQQHFGVKDRGAGLLQSVFICSFMVAAPIFGYLGDRFNRKVILSCGIFFWSAVTFSSSFIPQQYFWLLVLSRGLVGIGEASYSTIAPTIIGDLFTKNTRTLMLSVFYFAIPLGSGLGYITGSSVKQAAGDWHWALRVSPVLGMITGTLILILVPATKRGHADQLGDQLKARTSWLRDMKALIRNRSYVFSSLATSAVSFATGALGMWIPLYLHRAQVVQKTADYKDDDDKETCNSPPCGAKDSLIFGAITCFTGFLGVVTGAGATRWCRLKTQRADPLVCAVGMLGSAIFICLIFVAAKSSIVGAYICIFVGETLLFSNWAITADILMYVVIPTRRATAVALQSFTSHLLGDAGSPYLIGFISDLIRQSTKDSPLWEFLSLGYALMLCPFVVVLGGMFFLATALFFVSDRARAEQQVNQLAMPPASVKV

SEQ ID NO: 167 - DNA, 1674 bp, synthetic construct
  misc_feature 1..1674: note = Homo sapiens
  source 1..1674: mol_type = other DNA
atgatgtgcctggaatgcgcctcggcggcggcgggcggcgcggaggaggaggaggcggacgcggagcggcggcgccggcgccggggggcgcagcgaggggctggcggtagcggttgctgcggggcgcggggcgcgggcggcgctggagtctcggccgcgggcgatgaggtgcagacgctgtcgggcagcgtaaggcgggccccgaccggaccccccggcacccccggcacccccggctgcgcagctactgcaaagggccccggcgctcagcagcccaaaccggccagcttgggccgcgggcggggggcagccgccgccatcctcagcttgggcaacgtgctcaactacctggacaggtacaccgtggcaggcgtccttctggacatccagcagcactttggggtcaaggaccgaggcgccggcctgctgcagtcagtgttcatctgtagcttcatggtggctgcccccatcttcggctacctgggcgaccgcttcaacaggaaggtgattctcagctgcggcattttcttctggtcggccgtcaccttctccagctccttcattccccagcagtacttctggctgctggtcctgtcccgggggctggtgggcatcggggaggccagctactccaccatcgcccccactatcattggcgacctcttcaccaagaacacgcgtacgctcatgctgtccgtcttctacttcgccatcccactgggcagtggcctgggctacattactggctccagcgtgaagcaggcagccggagactggcactgggcattgcgggtgtcccctgtcctgggcatgatcacaggaacactcatcctcattctggtcccagccactaaaaggggtcatgccgaccagctcggggaccagctcaaggcccggacctcatggctccgagatatgaaggccctgattcgaaaccgcagctacgtcttctcctccctggccacgtcggctgtctccttcgccacgggggccctgggcatgtggatcccgctctacctgcaccgcgcccaagttgtgcagaagacagcagattacaaggatgacgacgataaggagacgtgcaacagcccgccctgtggggccaaggacagcctcatctttggggccatcacctgctttacgggatttctgggcgtggtcacgggggcaggagccacgcgctggtgccgcctgaagacccagcgggccgacccactggtgtgtgccgtgggcatgctgggctctgccatcttcatctgcctgatcttcgtggctgccaagagcagcatcgtaggagcctatatctgtatcttcgtcggggagacgctgctgttttctaactgggccatcactgcagacatcctcatgtacgtggtcatccccacgcggcgcgccactgccgtggccttgcagagcttcacctcccacctgctgggggacgccgggagcccctacctcattggctttatctcagacctgatccgccagagcactaaggactccccgctctgggagttcctgagcctgggctacgcgctcatgctctgccctttcgtcgtggtcctgggcggcatgttcttcctcgccactgcgctcttcttcgtcagcgaccgcgccagggctgagcagcaggtgaaccagctggcgatgccgcccgcatctgtgaaagtctga

SEQ ID NO: 168 - protein, 557 aa, synthetic construct
  REGION 1..557: note = Homo sapiens
MMCLECASAAAGGAEEEEADAERRRRRRGAQRGAGGSGCCGARGAGGAGVSAAGDEVQTLSGSVRRAPTGPPGTPGTPGCAATAKGPGAQQPKPASLGRGRGAAAAILSLGNVLNYLDRYTVAGVLLDIQQHFGVKDRGAGLLQSVFICSFMVAAPIFGYLGDRFNRKVILSCGIFFWSAVTFSSSFIPQQYFWLLVLSRGLVGIGEASYSTIAPTIIGDLFTKNTRTLMLSVFYFAIPLGSGLGYITGSSVKQAAGDWHWALRVSPVLGMITGTLILILVPATKRGHADQLGDQLKARTSWLRDMKALIRNRSYVFSSLATSAVSFATGALGMWIPLYLHRAQVVQKTAETCNSPPCGAKDSLIFGAITCFTGFLGVVTGAGATRWCRLKTQRADPLVCAVGMLGSAIFICLIFVAAKDYKDDDDKSSIVGAYICIFVGETLLFSNWAITADILMYVVIPTRRATAVALQSFTSHLLGDAGSPYLIGFISDLIRQSTKDSPLWEFLSLGYALMLCPFVVVLGGMFFLATALFFVSDRARAEQQVNQLAMPPASVKV

SEQ ID NO: 169 - DNA, 1674 bp, synthetic construct
  misc_feature 1..1674: note = Homo sapiens
  source 1..1674: mol_type = other DNA
atgatgtgcctggaatgcgcctcggcggcggcgggcggcgcggaggaggaggaggcggacgcggagcggcggcgccggcgccggggggcgcagcgaggggctggcggtagcggttgctgcggggcgcggggcgcgggcggcgctggagtctcggccgcgggcgatgaggtgcagacgctgtcgggcagcgtaaggcgggccccgaccggaccccccggcacccccggcacccccggctgcgcagctactgcaaagggccccggcgctcagcagcccaaaccggccagcttgggccgcgggcggggggcagccgccgccatcctcagcttgggcaacgtgctcaactacctggacaggtacaccgtggcaggcgtccttctggacatccagcagcactttggggtcaaggaccgaggcgccggcctgctgcagtcagtgttcatctgtagcttcatggtggctgcccccatcttcggctacctgggcgaccgcttcaacaggaaggtgattctcagctgcggcattttcttctggtcggccgtcaccttctccagctccttcattccccagcagtacttctggctgctggtcctgtcccgggggctggtgggcatcggggaggccagctactccaccatcgcccccactatcattggcgacctcttcaccaagaacacgcgtacgctcatgctgtccgtcttctacttcgccatcccactgggcagtggcctgggctacattactggctccagcgtgaagcaggcagccggagactggcactgggcattgcgggtgtcccctgtcctgggcatgatcacaggaacactcatcctcattctggtcccagccactaaaaggggtcatgccgaccagctcggggaccagctcaaggcccggacctcatggctccgagatatgaaggccctgattcgaaaccgcagctacgtcttctcctccctggccacgtcggctgtctccttcgccacgggggccctgggcatgtggatcccgctctacctgcaccgcgcccaagttgtgcagaagacagcagagacgtgcaacagcccgccctgtggggccaaggacagcctcatctttggggccatcacctgctttacgggatttctgggcgtggtcacgggggcaggagccacgcgctggtgccgcctgaagacccagcgggccgacccactggtgtgtgccgtgggcatgctgggctctgccatcttcatctgcctgatcttcgtggctgccaaggattacaaggatgacgacgataagagcagcatcgtaggagcctatatctgtatcttcgtcggggagacgctgctgttttctaactgggccatcactgcagacatcctcatgtacgtggtcatccccacgcggcgcgccactgccgtggccttgcagagcttcacctcccacctgctgggggacgccgggagcccctacctcattggctttatctcagacctgatccgccagagcactaaggactccccgctctgggagttcctgagcctgggctacgcgctcatgctctgccctttcgtcgtggtcctgggcggcatgttcttcctcgccactgcgctcttcttcgtcagcgaccgcgccagggctgagcagcaggtgaaccagctggcgatgccgcccgcatctgtgaaagtctga

SEQ ID NO: 170 - protein, 557 aa, synthetic construct
  REGION 1..557: note = Homo sapiens
MMCLECASAAAGGAEEEEADAERRRRRRGAQRGAGGSGCCGARGAGGAGVSAAGDEVQTLSGSVRRAPTGPPGTPGTPGCAATAKGPGAQQPKPASLGRGRGAAAAILSLGNVLNYLDRYTVAGVLLDIQQHFGVKDRGAGLLQSVFICSFMVAAPIFGYLGDRFNRKVILSCGIFFWSAVTFSSSFIPQQYFWLLVLSRGLVGIGEASYSTIAPTIIGDLFTKNTRTLMLSVFYFAIPLGSGLGYITGSSVKQAAGDWHWALRVSPVLGMITGTLILILVPATKRGHADQLGDQLKARTSWLRDMKALIRNRSYVFSSLATSAVSFATGALGMWIPLYLHRAQVVQKTAETCNSPPCGAKDSLIFGAITCFTGFLGVVTGAGATRWCRLKTQRADPLVCAVGMLGSAIFICLIFVAAKSSIVGAYICIFVGETLLFSNWAITADILMYVVIPTRRATAVALQSFTSHLLGDAGSPYLIGFISDLIRQSTKDSPLWDYKDDDDKEFLSLGYALMLCPFVVVLGGMFFLATALFFVSDRARAEQQVNQLAMPPASVKV

SEQ ID NO: 171 - DNA, 1674 bp, synthetic construct
  misc_feature 1..1674: note = Homo sapiens
  source 1..1674: mol_type = other DNA
atgatgtgcctggaatgcgcctcggcggcggcgggcggcgcggaggaggaggaggcggacgcggagcggcggcgccggcgccggggggcgcagcgaggggctggcggtagcggttgctgcggggcgcggggcgcgggcggcgctggagtctcggccgcgggcgatgaggtgcagacgctgtcgggcagcgtaaggcgggccccgaccggaccccccggcacccccggcacccccggctgcgcagctactgcaaagggccccggcgctcagcagcccaaaccggccagcttgggccgcgggcggggggcagccgccgccatcctcagcttgggcaacgtgctcaactacctggacaggtacaccgtggcaggcgtccttctggacatccagcagcactttggggtcaaggaccgaggcgccggcctgctgcagtcagtgttcatctgtagcttcatggtggctgcccccatcttcggctacctgggcgaccgcttcaacaggaaggtgattctcagctgcggcattttcttctggtcggccgtcaccttctccagctccttcattccccagcagtacttctggctgctggtcctgtcccgggggctggtgggcatcggggaggccagctactccaccatcgcccccactatcattggcgacctcttcaccaagaacacgcgtacgctcatgctgtccgtcttctacttcgccatcccactgggcagtggcctgggctacattactggctccagcgtgaagcaggcagccggagactggcactgggcattgcgggtgtcccctgtcctgggcatgatcacaggaacactcatcctcattctggtcccagccactaaaaggggtcatgccgaccagctcggggaccagctcaaggcccggacctcatggctccgagatatgaaggccctgattcgaaaccgcagctacgtcttctcctccctggccacgtcggctgtctccttcgccacgggggccctgggcatgtggatcccgctctacctgcaccgcgcccaagttgtgcagaagacagcagagacgtgcaacagcccgccctgtggggccaaggacagcctcatctttggggccatcacctgctttacgggatttctgggcgtggtcacgggggcaggagccacgcgctggtgccgcctgaagacccagcgggccgacccactggtgtgtgccgtgggcatgctgggctctgccatcttcatctgcctgatcttcgtggctgccaagagcagcatcgtaggagcctatatctgtatcttcgtcggggagacgctgctgttttctaactgggccatcactgcagacatcctcatgtacgtggtcatccccacgcggcgcgccactgccgtggccttgcagagcttcacctcccacctgctgggggacgccgggagcccctacctcattggctttatctcagacctgatccgccagagcactaaggactccccgctctgggattacaaggatgacgacgataaggagttcctgagcctgggctacgcgctcatgctctgccctttcgtcgtggtcctgggcggcatgttcttcctcgccactgcgctcttcttcgtcagcgaccgcgccagggctgagcagcaggtgaaccagctggcgatgccgcccgcatctgtgaaagtctga

SEQ ID NO: 172 - protein, 549 aa, synthetic construct
  REGION 1..549: note = Homo sapiens
MMCLECASAAAGGAEEEEADAERRRRRRGAQRGAGGSGCCGARGAGGAGVSAAGDEVQTLSGSVRRAPTGPPGTPGTPGCAATAKGPGAQQPKPASLGRGRGAAAAILSLGNVLNYLDRYTVAGVLADIQQHFGVKDRGAGLLQSVFICSFMVAAPIFGYLGDRFNRKVILSCGIFFWSAVTFSSSFIPQQYFWLLVLSRGLVGIGEASYSTIAPTIIGDLFTKNTRTLMLSVFYFAIPLGSGLGYITGSSVKQAAGDWHWALRVSPVLGMITGTLILILVPATKRGHADQLGDQLKARTSWLRDMKALIRNRSYVFSSLATSAVSFATGALGMWIPLYLHRAQVVQKTAETCNSPPCGAKDSLIFGAITCFTGFLGVVTGAGATRWCRLKTQRADPLVCAVGMLGSAIFICLIFVAAKSSIVGAYICIFVGETLLFSNWAITADILMYVVIPTRRATAVALQSFTSHLLGDAGSPYLIGFISDLIRQSTKDSPLWEFLSLGYALMLCPFVVVLGGMFFLATALFFVSDRARAEQQVNQLAMPPASVKV

SEQ ID NO: 173 - protein, 549 aa, synthetic construct
  REGION 1..549: note = Homo sapiens
MMCLECASAAAGGAEEEEADAERRRRRRGAQRGAGGSGCCGARGAGGAGVSAAGDEVQTLSGSVRRAPTGPPGTPGTPGCAATAKGPGAQQPKPASLGRGRGAAAAILSLGNVLNYLDRYTVAGVLLAIQQHFGVKDRGAGLLQSVFICSFMVAAPIFGYLGDRFNRKVILSCGIFFWSAVTFSSSFIPQQYFWLLVLSRGLVGIGEASYSTIAPTIIGDLFTKNTRTLMLSVFYFAIPLGSGLGYITGSSVKQAAGDWHWALRVSPVLGMITGTLILILVPATKRGHADQLGDQLKARTSWLRDMKALIRNRSYVFSSLATSAVSFATGALGMWIPLYLHRAQVVQKTAETCNSPPCGAKDSLIFGAITCFTGFLGVVTGAGATRWCRLKTQRADPLVCAVGMLGSAIFICLIFVAAKSSIVGAYICIFVGETLLFSNWAITADILMYVVIPTRRATAVALQSFTSHLLGDAGSPYLIGFISDLIRQSTKDSPLWEFLSLGYALMLCPFVVVLGGMFFLATALFFVSDRARAEQQVNQLAMPPASVKV

SEQ ID NO: 174 - protein, 549 aa, synthetic construct
  REGION 1..549: note = Homo sapiens
MMCLECASAAAGGAEEEEADAERRRRRRGAQRGAGGSGCCGARGAGGAGVSAAGDEVQTLSGSVRRAPTGPPGTPGTPGCAATAKGPGAQQPKPASLGRGRGAAAAILSLGNVLNYLDRYTVAGVLLDAQQHFGVKDRGAGLLQSVFICSFMVAAPIFGYLGDRFNRKVILSCGIFFWSAVTFSSSFIPQQYFWLLVLSRGLVGIGEASYSTIAPTIIGDLFTKNTRTLMLSVFYFAIPLGSGLGYITGSSVKQAAGDWHWALRVSPVLGMITGTLILILVPATKRGHADQLGDQLKARTSWLRDMKALIRNRSYVFSSLATSAVSFATGALGMWIPLYLHRAQVVQKTAETCNSPPCGAKDSLIFGAITCFTGFLGVVTGAGATRWCRLKTQRADPLVCAVGMLGSAIFICLIFVAAKSSIVGAYICIFVGETLLFSNWAITADILMYVVIPTRRATAVALQSFTSHLLGDAGSPYLIGFISDLIRQSTKDSPLWEFLSLGYALMLCPFVVVLGGMFFLATALFFVSDRARAEQQVNQLAMPPASVKV

SEQ ID NO: 175 - protein, 549 aa, synthetic construct
  REGION 1..549: note = Homo sapiens
MMCLECASAAAGGAEEEEADAERRRRRRGAQRGAGGSGCCGARGAGGAGVSAAGDEVQTLSGSVRRAPTGPPGTPGTPGCAATAKGPGAQQPKPASLGRGRGAAAAILSLGNVLNYLDRYTVAGVLLDIAQHFGVKDRGAGLLQSVFICSFMVAAPIFGYLGDRFNRKVILSCGIFFWSAVTFSSSFIPQQYFWLLVLSRGLVGIGEASYSTIAPTIIGDLFTKNTRTLMLSVFYFAIPLGSGLGYITGSSVKQAAGDWHWALRVSPVLGMITGTLILILVPATKRGHADQLGDQLKARTSWLRDMKALIRNRSYVFSSLATSAVSFATGALGMWIPLYLHRAQVVQKTAETCNSPPCGAKDSLIFGAITCFTGFLGVVTGAGATRWCRLKTQRADPLVCAVGMLGSAIFICLIFVAAKSSIVGAYICIFVGETLLFSNWAITADILMYVVIPTRRATAVALQSFTSHLLGDAGSPYLIGFISDLIRQSTKDSPLWEFLSLGYALMLCPFVVVLGGMFFLATALFFVSDRARAEQQVNQLAMPPASVKV

SEQ ID NO: 176 - protein, 549 aa, synthetic construct
  REGION 1..549: note = Homo sapiens
MMCLECASAAAGGAEEEEADAERRRRRRGAQRGAGGSGCCGARGAGGAGVSAAGDEVQTLSGSVRRAPTGPPGTPGTPGCAATAKGPGAQQPKPASLGRGRGAAAAILSLGNVLNYLDRYTVAGVLLDIQAHFGVKDRGAGLLQSVFICSFMVAAPIFGYLGDRFNRKVILSCGIFFWSAVTFSSSFIPQQYFWLLVLSRGLVGIGEASYSTIAPTIIGDLFTKNTRTLMLSVFYFAIPLGSGLGYITGSSVKQAAGDWHWALRVSPVLGMITGTLILILVPATKRGHADQLGDQLKARTSWLRDMKALIRNRSYVFSSLATSAVSFATGALGMWIPLYLHRAQVVQKTAETCNSPPCGAKDSLIFGAITCFTGFLGVVTGAGATRWCRLKTQRADPLVCAVGMLGSAIFICLIFVAAKSSIVGAYICIFVGETLLFSNWAITADILMYVVIPTRRATAVALQSFTSHLLGDAGSPYLIGFISDLIRQSTKDSPLWEFLSLGYALMLCPFVVVLGGMFFLATALFFVSDRARAEQQVNQLAMPPASVKV

SEQ ID NO: 177 - protein, 549 aa, synthetic construct
  REGION 1..549: note = Homo sapiens
MMCLECASAAAGGAEEEEADAERRRRRRGAQRGAGGSGCCGARGAGGAGVSAAGDEVQTLSGSVRRAPTGPPGTPGTPGCAATAKGPGAQQPKPASLGRGRGAAAAILSLGNVLNYLDRYTVAGVLLDIQQAFGVKDRGAGLLQSVFICSFMVAAPIFGYLGDRFNRKVILSCGIFFWSAVTFSSSFIPQQYFWLLVLSRGLVGIGEASYSTIAPTIIGDLFTKNTRTLMLSVFYFAIPLGSGLGYITGSSVKQAAGDWHWALRVSPVLGMITGTLILILVPATKRGHADQLGDQLKARTSWLRDMKALIRNRSYVFSSLATSAVSFATGALGMWIPLYLHRAQVVQKTAETCNSPPCGAKDSLIFGAITCFTGFLGVVTGAGATRWCRLKTQRADPLVCAVGMLGSAIFICLIFVAAKSSIVGAYICIFVGETLLFSNWAITADILMYVVIPTRRATAVALQSFTSHLLGDAGSPYLIGFISDLIRQSTKDSPLWEFLSLGYALMLCPFVVVLGGMFFLATALFFVSDRARAEQQVNQLAMPPASVKV

SEQ ID NO: 178 - protein, 549 aa, synthetic construct
  REGION 1..549: note = Homo sapiens
MMCLECASAAAGGAEEEEADAERRRRRRGAQRGAGGSGCCGARGAGGAGVSAAGDEVQTLSGSVRRAPTGPPGTPGTPGCAATAKGPGAQQPKPASLGRGRGAAAAILSLGNVLNYLDRYTVAGVLLDIQQHAGVKDRGAGLLQSVFICSFMVAAPIFGYLGDRFNRKVILSCGIFFWSAVTFSSSFIPQQYFWLLVLSRGLVGIGEASYSTIAPTIIGDLFTKNTRTLMLSVFYFAIPLGSGLGYITGSSVKQAAGDWHWALRVSPVLGMITGTLILILVPATKRGHADQLGDQLKARTSWLRDMKALIRNRSYVFSSLATSAVSFATGALGMWIPLYLHRAQVVQKTAETCNSPPCGAKDSLIFGAITCFTGFLGVVTGAGATRWCRLKTQRADPLVCAVGMLGSAIFICLIFVAAKSSIVGAYICIFVGETLLFSNWAITADILMYVVIPTRRATAVALQSFTSHLLGDAGSPYLIGFISDLIRQSTKDSPLWEFLSLGYALMLCPFVVVLGGMFFLATALFFVSDRARAEQQVNQLAMPPASVKV

SEQ ID NO: 179 - protein, 549 aa, synthetic construct
  REGION 1..549: note = Homo sapiens
MMCLECASAAAGGAEEEEADAERRRRRRGAQRGAGGSGCCGARGAGGAGVSAAGDEVQTLSGSVRRAPTGPPGTPGTPGCAATAKGPGAQQPKPASLGRGRGAAAAILSLGNVLNYLDRYTVAGVLLDIQQHFAVKDRGAGLLQSVFICSFMVAAPIFGYLGDRFNRKVILSCGIFFWSAVTFSSSFIPQQYFWLLVLSRGLVGIGEASYSTIAPTIIGDLFTKNTRTLMLSVFYFAIPLGSGLGYITGSSVKQAAGDWHWALRVSPVLGMITGTLILILVPATKRGHADQLGDQLKARTSWLRDMKALIRNRSYVFSSLATSAVSFATGALGMWIPLYLHRAQVVQKTAETCNSPPCGAKDSLIFGAITCFTGFLGVVTGAGATRWCRLKTQRADPLVCAVGMLGSAIFICLIFVAAKSSIVGAYICIFVGETLLFSNWAITADILMYVVIPTRRATAVALQSFTSHLLGDAGSPYLIGFISDLIRQSTKDSPLWEFLSLGYALMLCPFVVVLGGMFFLATALFFVSDRARAEQQVNQLAMPPASVKV

SEQ ID NO: 180 - protein, 549 aa, synthetic construct
  REGION 1..549: note = Homo sapiens
MMCLECASAAAGGAEEEEADAERRRRRRGAQRGAGGSGCCGARGAGGAGVSAAGDEVQTLSGSVRRAPTGPPGTPGTPGCAATAKGPGAQQPKPASLGRGRGAAAAILSLGNVLNYLDRYTVAGVLLDIQQHFGAKDRGAGLLQSVFICSFMVAAPIFGYLGDRFNRKVILSCGIFFWSAVTFSSSFIPQQYFWLLVLSRGLVGIGEASYSTIAPTIIGDLFTKNTRTLMLSVFYFAIPLGSGLGYITGSSVKQAAGDWHWALRVSPVLGMITGTLILILVPATKRGHADQLGDQLKARTSWLRDMKALIRNRSYVFSSLATSAVSFATGALGMWIPLYLHRAQVVQKTAETCNSPPCGAKDSLIFGAITCFTGFLGVVTGAGATRWCRLKTQRADPLVCAVGMLGSAIFICLIFVAAKSSIVGAYICIFVGETLLFSNWAITADILMYVVIPTRRATAVALQSFTSHLLGDAGSPYLIGFISDLIRQSTKDSPLWEFLSLGYALMLCPFVVVLGGMFFLATALFFVSDRARAEQQVNQLAMPPASVKV

SEQ ID NO: 181 - protein, 549 aa, synthetic construct
  REGION 1..549: note = Homo sapiens
MMCLECASAAAGGAEEEEADAERRRRRRGAQRGAGGSGCCGARGAGGAGVSAAGDEVQTLSGSVRRAPTGPPGTPGTPGCAATAKGPGAQQPKPASLGRGRGAAAAILSLGNVLNYLDRYTVAGVLLDIQQHFGVADRGAGLLQSVFICSFMVAAPIFGYLGDRFNRKVILSCGIFFWSAVTFSSSFIPQQYFWLLVLSRGLVGIGEASYSTIAPTIIGDLFTKNTRTLMLSVFYFAIPLGSGLGYITGSSVKQAAGDWHWALRVSPVLGMITGTLILILVPATKRGHADQLGDQLKARTSWLRDMKALIRNRSYVFSSLATSAVSFATGALGMWIPLYLHRAQVVQKTAETCNSPPCGAKDSLIFGAITCFTGFLGVVTGAGATRWCRLKTQRADPLVCAVGMLGSAIFICLIFVAAKSSIVGAYICIFVGETLLFSNWAITADILMYVVIPTRRATAVALQSFTSHLLGDAGSPYLIGFISDLIRQSTKDSPLWEFLSLGYALMLCPFVVVLGGMFFLATALFFVSDRARAEQQVNQLAMPPASVKV

SEQ ID NO: 182 - protein, 549 aa, synthetic construct
  REGION 1..549: note = Homo sapiens
MMCLECASAAAGGAEEEEADAERRRRRRGAQRGAGGSGCCGARGAGGAGVSAAGDEVQTLSGSVRRAPTGPPGTPGTPGCAATAKGPGAQQPKPASLGRGRGAAAAILSLGNVLNYLDRYTVAGVLLDIQQHFGVKARGAGLLQSVFICSFMVAAPIFGYLGDRFNRKVILSCGIFFWSAVTFSSSFIPQQYFWLLVLSRGLVGIGEASYSTIAPTIIGDLFTKNTRTLMLSVFYFAIPLGSGLGYITGSSVKQAAGDWHWALRVSPVLGMITGTLILILVPATKRGHADQLGDQLKARTSWLRDMKALIRNRSYVFSSLATSAVSFATGALGMWIPLYLHRAQVVQKTAETCNSPPCGAKDSLIFGAITCFTGFLGVVTGAGATRWCRLKTQRADPLVCAVGMLGSAIFICLIFVAAKSSIVGAYICIFVGETLLFSNWAITADILMYVVIPTRRATAVALQSFTSHLLGDAGSPYLIGFISDLIRQSTKDSPLWEFLSLGYALMLCPFVVVLGGMFFLATALFFVSDRARAEQQVNQLAMPPASVKV

SEQ ID NO: 183 - protein, 549 aa, synthetic construct
  REGION 1..549: note = Homo sapiens
MMCLECASAAAGGAEEEEADAERRRRRRGAQRGAGGSGCCGARGAGGAGVSAAGDEVQTLSGSVRRAPTGPPGTPGTPGCAATAKGPGAQQPKPASLGRGRGAAAAILSLGNVLNYLDRYTVAGVLLDIQQHFGVKDAGAGLLQSVFICSFMVAAPIFGYLGDRFNRKVILSCGIFFWSAVTFSSSFIPQQYFWLLVLSRGLVGIGEASYSTIAPTIIGDLFTKNTRTLMLSVFYFAIPLGSGLGYITGSSVKQAAGDWHWALRVSPVLGMITGTLILILVPATKRGHADQLGDQLKARTSWLRDMKALIRNRSYVFSSLATSAVSFATGALGMWIPLYLHRAQVVQKTAETCNSPPCGAKDSLIFGAITCFTGFLGVVTGAGATRWCRLKTQRADPLVCAVGMLGSAIFICLIFVAAKSSIVGAYICIFVGETLLFSNWAITADILMYVVIPTRRATAVALQSFTSHLLGDAGSPYLIGFISDLIRQSTKDSPLWEFLSLGYALMLCPFVVVLGGMFFLATALFFVSDRARAEQQVNQLAMPPASVKV

SEQ ID NO: 184 - protein, 549 aa, synthetic construct
  REGION 1..549: note = Homo sapiens
MMCLECASAAAGGAEEEEADAERRRRRRGAQRGAGGSGCCGARGAGGAGVSAAGDEVQTLSGSVRRAPTGPPGTPGTPGCAATAKGPGAQQPKPASLGRGRGAAAAILSLGNVLNYLDRYTVAGVLLDIQQHFGVKDRAAGLLQSVFICSFMVAAPIFGYLGDRFNRKVILSCGIFFWSAVTFSSSFIPQQYFWLLVLSRGLVGIGEASYSTIAPTIIGDLFTKNTRTLMLSVFYFAIPLGSGLGYITGSSVKQAAGDWHWALRVSPVLGMITGTLILILVPATKRGHADQLGDQLKARTSWLRDMKALIRNRSYVFSSLATSAVSFATGALGMWIPLYLHRAQVVQKTAETCNSPPCGAKDSLIFGAITCFTGFLGVVTGAGATRWCRLKTQRADPLVCAVGMLGSAIFICLIFVAAKSSIVGAYICIFVGETLLFSNWAITADILMYVVIPTRRATAVALQSFTSHLLGDAGSPYLIGFISDLIRQSTKDSPLWEFLSLGYALMLCPFVVVLGGMFFLATALFFVSDRARAEQQVNQLAMPPASVKV

SEQ ID NO: 185 - protein, 549 aa, synthetic construct
  REGION 1..549: note = Homo sapiens
MMCLECASAAAGGAEEEEADAERRRRRRGAQRGAGGSGCCGARGAGGAGVSAAGDEVQTLSGSVRRAPTGPPGTPGTPGCAATAKGPGAQQPKPASLGRGRGAAAAILSLGNVLNYLDRYTVAGVLLDIQQHFGVKDRGAGLLQSVFICSFMVAAPIFGYLGDRFNRKVILSCGIFFWSAVTFSSSFIAQQYFWLLVLSRGLVGIGEASYSTIAPTIIGDLFTKNTRTLMLSVFYFAIPLGSGLGYITGSSVKQAAGDWHWALRVSPVLGMITGTLILILVPATKRGHADQLGDQLKARTSWLRDMKALIRNRSYVFSSLATSAVSFATGALGMWIPLYLHRAQVVQKTAETCNSPPCGAKDSLIFGAITCFTGFLGVVTGAGATRWCRLKTQRADPLVCAVGMLGSAIFICLIFVAAKSSIVGAYICIFVGETLLFSNWAITADILMYVVIPTRRATAVALQSFTSHLLGDAGSPYLIGFISDLIRQSTKDSPLWEFLSLGYALMLCPFVVVLGGMFFLATALFFVSDRARAEQQVNQLAMPPASVKV

SEQ ID NO: 186 - protein, 549 aa, synthetic construct
  REGION 1..549: note = Homo sapiens
MMCLECASAAAGGAEEEEADAERRRRRRGAQRGAGGSGCCGARGAGGAGVSAAGDEVQTLSGSVRRAPTGPPGTPGTPGCAATAKGPGAQQPKPASLGRGRGAAAAILSLGNVLNYLDRYTVAGVLLDIQQHFGVKDRGAGLLQSVFICSFMVAAPIFGYLGDRFNRKVILSCGIFFWSAVTFSSSFIPAQYFWLLVLSRGLVGIGEASYSTIAPTIIGDLFTKNTRTLMLSVFYFAIPLGSGLGYITGSSVKQAAGDWHWALRVSPVLGMITGTLILILVPATKRGHADQLGDQLKARTSWLRDMKALIRNRSYVFSSLATSAVSFATGALGMWIPLYLHRAQVVQKTAETCNSPPCGAKDSLIFGAITCFTGFLGVVTGAGATRWCRLKTQRADPLVCAVGMLGSAIFICLIFVAAKSSIVGAYICIFVGETLLFSNWAITADILMYVVIPTRRATAVALQSFTSHLLGDAGSPYLIGFISDLIRQSTKDSPLWEFLSLGYALMLCPFVVVLGGMFFLATALFFVSDRARAEQQVNQLAMPPASVKV

SEQ ID NO: 187 - protein, 549 aa, synthetic construct
  REGION 1..549: note = Homo sapiens
MMCLECASAAAGGAEEEEADAERRRRRRGAQRGAGGSGCCGARGAGGAGVSAAGDEVQTLSGSVRRAPTGPPGTPGTPGCAATAKGPGAQQPKPASLGRGRGAAAAILSLGNVLNYLDRYTVAGVLLDIQQHFGVKDRGAGLLQSVFICSFMVAAPIFGYLGDRFNRKVILSCGIFFWSAVTFSSSFIPQAYFWLLVLSRGLVGIGEASYSTIAPTIIGDLFTKNTRTLMLSVFYFAIPLGSGLGYITGSSVKQAAGDWHWALRVSPVLGMITGTLILILVPATKRGHADQLGDQLKARTSWLRDMKALIRNRSYVFSSLATSAVSFATGALGMWIPLYLHRAQVVQKTAETCNSPPCGAKDSLIFGAITCFTGFLGVVTGAGATRWCRLKTQRADPLVCAVGMLGSAIFICLIFVAAKSSIVGAYICIFVGETLLFSNWAITADILMYVVIPTRRATAVALQSFTSHLLGDAGSPYLIGFISDLIRQSTKDSPLWEFLSLGYALMLCPFVVVLGGMFFLATALFFVSDRARAEQQVNQLAMPPASVKV

SEQ ID NO: 188 - protein, 549 aa, synthetic construct
  REGION 1..549: note = Homo sapiens
MMCLECASAAAGGAEEEEADAERRRRRRGAQRGAGGSGCCGARGAGGAGVSAAGDEVQTLSGSVRRAPTGPPGTPGTPGCAATAKGPGAQQPKPASLGRGRGAAAAILSLGNVLNYLDRYTVAGVLLDIQQHFGVKDRGAGLLQSVFICSFMVAAPIFGYLGDRFNRKVILSCGIFFWSAVTFSSSFIPQQAFWLLVLSRGLVGIGEASYSTIAPTIIGDLFTKNTRTLMLSVFYFAIPLGSGLGYITGSSVKQAAGDWHWALRVSPVLGMITGTLILILVPATKRGHADQLGDQLKARTSWLRDMKALIRNRSYVFSSLATSAVSFATGALGMWIPLYLHRAQVVQKTAETCNSPPCGAKDSLIFGAITCFTGFLGVVTGAGATRWCRLKTQRADPLVCAVGMLGSAIFICLIFVAAKSSIVGAYICIFVGETLLFSNWAITADILMYVVIPTRRATAVALQSFTSHLLGDAGSPYLIGFISDLIRQSTKDSPLWEFLSLGYALMLCPFVVVLGGMFFLATALFFVSDRARAEQQVNQLAMPPASVKV

SEQ ID NO: 189 - protein, 549 aa, synthetic construct
  REGION 1..549: note = Homo sapiens
MMCLECASAAAGGAEEEEADAERRRRRRGAQRGAGGSGCCGARGAGGAGVSAAGDEVQTLSGSVRRAPTGPPGTPGTPGCAATAKGPGAQQPKPASLGRGRGAAAAILSLGNVLNYLDRYTVAGVLLDIQQHFGVKDRGAGLLQSVFICSFMVAAPIFGYLGDRFNRKVILSCGIFFWSAVTFSSSFIPQQYAWLLVLSRGLVGIGEASYSTIAPTIIGDLFTKNTRTLMLSVFYFAIPLGSGLGYITGSSVKQAAGDWHWALRVSPVLGMITGTLILILVPATKRGHADQLGDQLKARTSWLRDMKALIRNRSYVFSSLATSAVSFATGALGMWIPLYLHRAQVVQKTAETCNSPPCGAKDSLIFGAITCFTGFLGVVTGAGATRWCRLKTQRADPLVCAVGMLGSAIFICLIFVAAKSSIVGAYICIFVGETLLFSNWAITADILMYVVIPTRRATAVALQSFTSHLLGDAGSPYLIGFISDLIRQSTKDSPLWEFLSLGYALMLCPFVVVLGGMFFLATALFFVSDRARAEQQVNQLAMPPASVKV

SEQ ID NO: 190 - protein, 549 aa, synthetic construct
  REGION 1..549: note = Homo sapiens
MMCLECASAAAGGAEEEEADAERRRRRRGAQRGAGGSGCCGARGAGGAGVSAAGDEVQTLSGSVRRAPTGPPGTPGTPGCAATAKGPGAQQPKPASLGRGRGAAAAILSLGNVLNYLDRYTVAGVLLDIQQHFGVKDRGAGLLQSVFICSFMVAAPIFGYLGDRFNRKVILSCGIFFWSAVTFSSSFIPQQYFALLVLSRGLVGIGEASYSTIAPTIIGDLFTKNTRTLMLSVFYFAIPLGSGLGYITGSSVKQAAGDWHWALRVSPVLGMITGTLILILVPATKRGHADQLGDQLKARTSWLRDMKALIRNRSYVFSSLATSAVSFATGALGMWIPLYLHRAQVVQKTAETCNSPPCGAKDSLIFGAITCFTGFLGVVTGAGATRWCRLKTQRADPLVCAVGMLGSAIFICLIFVAAKSSIVGAYICIFVGETLLFSNWAITADILMYVVIPTRRATAVALQSFTSHLLGDAGSPYLIGFISDLIRQSTKDSPLWEFLSLGYALMLCPFVVVLGGMFFLATALFFVSDRARAEQQVNQLAMPPASVKV

SEQ ID NO: 191 - protein, 549 aa, synthetic construct
  REGION 1..549: note = Homo sapiens
MMCLECASAAAGGAEEEEADAERRRRRRGAQRGAGGSGCCGARGAGGAGVSAAGDEVQTLSGSVRRAPTGPPGTPGTPGCAATAKGPGAQQPKPASLGRGRGAAAAILSLGNVLNYLDRYTVAGVLLDIQQHFGVKDRGAGLLQSVFICSFMVAAPIFGYLGDRFNRKVILSCGIFFWSAVTFSSSFIPQQYFWALVLSRGLVGIGEASYSTIAPTIIGDLFTKNTRTLMLSVFYFAIPLGSGLGYITGSSVKQAAGDWHWALRVSPVLGMITGTLILILVPATKRGHADQLGDQLKARTSWLRDMKALIRNRSYVFSSLATSAVSFATGALGMWIPLYLHRAQVVQKTAETCNSPPCGAKDSLIFGAITCFTGFLGVVTGAGATRWCRLKTQRADPLVCAVGMLGSAIFICLIFVAAKSSIVGAYICIFVGETLLFSNWAITADILMYVVIPTRRATAVALQSFTSHLLGDAGSPYLIGFISDLIRQSTKDSPLWEFLSLGYALMLCPFVVVLGGMFFLATALFFVSDRARAEQQVNQLAMPPASVKV

SEQ ID NO: 192 - protein, 549 aa, synthetic construct
  REGION 1..549: note = Homo sapiens
MMCLECASAAAGGAEEEEADAERRRRRRGAQRGAGGSGCCGARGAGGAGVSAAGDEVQTLSGSVRRAPTGPPGTPGTPGCAATAKGPGAQQPKPASLGRGRGAAAAILSLGNVLNYLDRYTVAGVLLDIQQHFGVKDRGAGLLQSVFICSFMVAAPIFGYLGDRFNRKVILSCGIFFWSAVTFSSSFIPQQYFWLAVLSRGLVGIGEASYSTIAPTIIGDLFTKNTRTLMLSVFYFAIPLGSGLGYITGSSVKQAAGDWHWALRVSPVLGMITGTLILILVPATKRGHADQLGDQLKARTSWLRDMKALIRNRSYVFSSLATSAVSFATGALGMWIPLYLHRAQVVQKTAETCNSPPCGAKDSLIFGAITCFTGFLGVVTGAGATRWCRLKTQRADPLVCAVGMLGSAIFICLIFVAAKSSIVGAYICIFVGETLLFSNWAITADILMYVVIPTRRATAVALQSFTSHLLGDAGSPYLIGFISDLIRQSTKDSPLWEFLSLGYALMLCPFVVVLGGMFFLATALFFVSDRARAEQQVNQLAMPPASVKV

SEQ ID NO: 193 - protein, 549 aa, synthetic construct
  REGION 1..549: note = Homo sapiens
MMCLECASAAAGGAEEEEADAERRRRRRGAQRGAGGSGCCGARGAGGAGVSAAGDEVQTLSGSVRRAPTGPPGTPGTPGCAATAKGPGAQQPKPASLGRGRGAAAAILSLGNVLNYLDRYTVAGVLLDIQQHFGVKDRGAGLLQSVFICSFMVAAPIFGYLGDRFNRKVILSCGIFFWSAVTFSSSFIPQQYFWLLALSRGLVGIGEASYSTIAPTIIGDLFTKNTRTLMLSVFYFAIPLGSGLGYITGSSVKQAAGDWHWALRVSPVLGMITGTLILILVPATKRGHADQLGDQLKARTSWLRDMKALIRNRSYVFSSLATSAVSFATGALGMWIPLYLHRAQVVQKTAETCNSPPCGAKDSLIFGAITCFTGFLGVVTGAGATRWCRLKTQRADPLVCAVGMLGSAIFICLIFVAAKSSIVGAYICIFVGETLLFSNWAITADILMYVVIPTRRATAVALQSFTSHLLGDAGSPYLIGFISDLIRQSTKDSPLWEFLSLGYALMLCPFVVVLGGMFFLATALFFVSDRARAEQQVNQLAMPPASVKV

SEQ ID NO: 194 - protein, 549 aa, synthetic construct
  REGION 1..549: note = Homo sapiens
MMCLECASAAAGGAEEEEADAERRRRRRGAQRGAGGSGCCGARGAGGAGVSAAGDEVQTLSGSVRRAPTGPPGTPGTPGCAATAKGPGAQQPKPASLGRGRGAAAAILSLGNVLNYLDRYTVAGVLLDIQQHFGVKDRGAGLLQSVFICSFMVAAPIFGYLGDRFNRKVILSCGIFFWSAVTFSSSFIPQQYFWLLVASRGLVGIGEASYSTIAPTIIGDLFTKNTRTLMLSVFYFAIPLGSGLGYITGSSVKQAAGDWHWALRVSPVLGMITGTLILILVPATKRGHADQLGDQLKARTSWLRDMKALIRNRSYVFSSLATSAVSFATGALGMWIPLYLHRAQVVQKTAETCNSPPCGAKDSLIFGAITCFTGFLGVVTGAGATRWCRLKTQRADPLVCAVGMLGSAIFICLIFVAAKSSIVGAYICIFVGETLLFSNWAITADILMYVVIPTRRATAVALQSFTSHLLGDAGSPYLIGFISDLIRQSTKDSPLWEFLSLGYALMLCPFVVVLGGMFFLATALFFVSDRARAEQQVNQLAMPPASVKV

SEQ ID NO: 195 - protein, 549 aa, synthetic construct
  REGION 1..549: note = Homo sapiens
MMCLECASAAAGGAEEEEADAERRRRRRGAQRGAGGSGCCGARGAGGAGVSAAGDEVQTLSGSVRRAPTGPPGTPGTPGCAATAKGPGAQQPKPASLGRGRGAAAAILSLGNVLNYLDRYTVAGVLLDIQQHFGVKDRGAGLLQSVFICSFMVAAPIFGYLGDRFNRKVILSCGIFFWSAVTFSSSFIPQQYFWLLVLARGLVGIGEASYSTIAPTIIGDLFTKNTRTLMLSVFYFAIPLGSGLGYITGSSVKQAAGDWHWALRVSPVLGMITGTLILILVPATKRGHADQLGDQLKARTSWLRDMKALIRNRSYVFSSLATSAVSFATGALGMWIPLYLHRAQVVQKTAETCNSPPCGAKDSLIFGAITCFTGFLGVVTGAGATRWCRLKTQRADPLVCAVGMLGSAIFICLIFVAAKSSIVGAYICIFVGETLLFSNWAITADILMYVVIPTRRATAVALQSFTSHLLGDAGSPYLIGFISDLIRQSTKDSPLWEFLSLGYALMLCPFVVVLGGMFFLATALFFVSDRARAEQQVNQLAMPPASVKV

SEQ ID NO: 196 - protein, 549 aa, synthetic construct
  REGION 1..549: note = Homo sapiens
MMCLECASAAAGGAEEEEADAERRRRRRGAQRGAGGSGCCGARGAGGAGVSAAGDEVQTLSGSVRRAPTGPPGTPGTPGCAATAKGPGAQQPKPASLGRGRGAAAAILSLGNVLNYLDRYTVAGVLLDIQQHFGVKDRGAGLLQSVFICSFMVAAPIFGYLGDRFNRKVILSCGIFFWSAVTFSSSFIPQQYFWLLVLSAGLVGIGEASYSTIAPTIIGDLFTKNTRTLMLSVFYFAIPLGSGLGYITGSSVKQAAGDWHWALRVSPVLGMITGTLILILVPATKRGHADQLGDQLKARTSWLRDMKALIRNRSYVFSSLATSAVSFATGALGMWIPLYLHRAQVVQKTAETCNSPPCGAKDSLIFGAITCFTGFLGVVTGAGATRWCRLKTQRADPLVCAVGMLGSAIFICLIFVAAKSSIVGAYICIFVGETLLFSNWAITADILMYVVIPTRRATAVALQSFTSHLLGDAGSPYLIGFISDLIRQSTKDSPLWEFLSLGYALMLCPFVVVLGGMFFLATALFFVSDRARAEQQVNQLAMPPASVKV

SEQ ID NO: 197 - protein, 549 aa, synthetic construct
  REGION 1..549: note = Homo sapiens
MMCLECASAAAGGAEEEEADAERRRRRRGAQRGAGGSGCCGARGAGGAGVSAAGDEVQTLSGSVRRAPTGPPGTPGTPGCAATAKGPGAQQPKPASLGRGRGAAAAILSLGNVLNYLDRYTVAGVLLDIQQHFGVKDRGAGLLQSVFICSFMVAAPIFGYLGDRFNRKVILSCGIFFWSAVTFSSSFIPQQYFWLLVLSRALVGIGEASYSTIAPTIIGDLFTKNTRTLMLSVFYFAIPLGSGLGYITGSSVKQAAGDWHWALRVSPVLGMITGTLILILVPATKRGHADQLGDQLKARTSWLRDMKALIRNRSYVFSSLATSAVSFATGALGMWIPLYLHRAQVVQKTAETCNSPPCGAKDSLIFGAITCFTGFLGVVTGAGATRWCRLKTQRADPLVCAVGMLGSAIFICLIFVAAKSSIVGAYICIFVGETLLFSNWAITADILMYVVIPTRRATAVALQSFTSHLLGDAGSPYLIGFISDLIRQSTKDSPLWEFLSLGYALMLCPFVVVLGGMFFLATALFFVSDRARAEQQVNQLAMPPASVKV

SEQ ID NO: 198 - protein, 549 aa, synthetic construct
  REGION 1..549: note = Homo sapiens
MMCLECASAAAGGAEEEEADAERRRRRRGAQRGAGGSGCCGARGAGGAGVSAAGDEVQTLSGSVRRAPTGPPGTPGTPGCAATAKGPGAQQPKPASLGRGRGAAAAILSLGNVLNYLDRYTVAGVLLDIQQHFGVKDRGAGLLQSVFICSFMVAAPIFGYLGDRFNRKVILSCGIFFWSAVTFSSSFIPQQYFWLLVLSRGAVGIGEASYSTIAPTIIGDLFTKNTRTLMLSVFYFAIPLGSGLGYITGSSVKQAAGDWHWALRVSPVLGMITGTLILILVPATKRGHADQLGDQLKARTSWLRDMKALIRNRSYVFSSLATSAVSFATGALGMWIPLYLHRAQVVQKTAETCNSPPCGAKDSLIFGAITCFTGFLGVVTGAGATRWCRLKTQRADPLVCAVGMLGSAIFICLIFVAAKSSIVGAYICIFVGETLLFSNWAITADILMYVVIPTRRATAVALQSFTSHLLGDAGSPYLIGFISDLIRQSTKDSPLWEFLSLGYALMLCPFVVVLGGMFFLATALFFVSDRARAEQQVNQLAMPPASVKV

SEQ ID NO: 199 - protein, 549 aa, synthetic construct
  REGION 1..549: note = Homo sapiens
MMCLECASAAAGGAEEEEADAERRRRRRGAQRGAGGSGCCGARGAGGAGVSAAGDEVQTLSGSVRRAPTGPPGTPGTPGCAATAKGPGAQQPKPASLGRGRGAAAAILSLGNVLNYLDRYTVAGVLLDIQQHFGVKDRGAGLLQSVFICSFMVAAPIFGYLGDRFNRKVILSCGIFFWSAVTFSSSFIPQQYFWLLVLSRGLVGIGEASYSTIAPTIIGDLFTKNTRTLMLSVFYFAIPLGSGLGYITGSSAKQAAGDWHWALRVSPVLGMITGTLILILVPATKRGHADQLGDQLKARTSWLRDMKALIRNRSYVFSSLATSAVSFATGALGMWIPLYLHRAQVVQKTAETCNSPPCGAKDSLIFGAITCFTGFLGVVTGAGATRWCRLKTQRADPLVCAVGMLGSAIFICLIFVAAKSSIVGAYICIFVGETLLFSNWAITADILMYVVIPTRRATAVALQSFTSHLLGDAGSPYLIGFISDLIRQSTKDSPLWEFLSLGYALMLCPFVVVLGGMFFLATALFFVSDRARAEQQVNQLAMPPASVKV

SEQ ID NO: 200 - protein, 549 aa, synthetic construct
  REGION 1..549: note = Homo sapiens
MMCLECASAAAGGAEEEEADAERRRRRRGAQRGAGGSGCCGARGAGGAGVSAAGDEVQTLSGSVRRAPTGPPGTPGTPGCAATAKGPGAQQPKPASLGRGRGAAAAILSLGNVLNYLDRYTVAGVLLDIQQHFGVKDRGAGLLQSVFICSFMVAAPIFGYLGDRFNRKVILSCGIFFWSAVTFSSSFIPQQYFWLLVLSRGLVGIGEASYSTIAPTIIGDLFTKNTRTLMLSVFYFAIPLGSGLGYITGSSVAQAAGDWHWALRVSPVLGMITGTLILILVPATKRGHADQLGDQLKARTSWLRDMKALIRNRSYVFSSLATSAVSFATGALGMWIPLYLHRAQVVQKTAETCNSPPCGAKDSLIFGAITCFTGFLGVVTGAGATRWCRLKTQRADPLVCAVGMLGSAIFICLIFVAAKSSIVGAYICIFVGETLLFSNWAITADILMYVVIPTRRATAVALQSFTSHLLGDAGSPYLIGFISDLIRQSTKDSPLWEFLSLGYALMLCPFVVVLGGMFFLATALFFVSDRARAEQQVNQLAMPPASVKV

SEQ ID NO: 201 - protein, 549 aa, synthetic construct
  REGION 1..549: note = Homo sapiens
MMCLECASAAAGGAEEEEADAERRRRRRGAQRGAGGSGCCGARGAGGAGVSAAGDEVQTLSGSVRRAPTGPPGTPGTPGCAATAKGPGAQQPKPASLGRGRGAAAAILSLGNVLNYLDRYTVAGVLLDIQQHFGVKDRGAGLLQSVFICSFMVAAPIFGYLGDRFNRKVILSCGIFFWSAVTFSSSFIPQQYFWLLVLSRGLVGIGEASYSTIAPTIIGDLFTKNTRTLMLSVFYFAIPLGSGLGYITGSSVKAAAGDWHWALRVSPVLGMITGTLILILVPATKRGHADQLGDQLKARTSWLRDMKALIRNRSYVFSSLATSAVSFATGALGMWIPLYLHRAQVVQKTAETCNSPPCGAKDSLIFGAITCFTGFLGVVTGAGATRWCRLKTQRADPLVCAVGMLGSAIFICLIFVAAKSSIVGAYICIFVGETLLFSNWAITADILMYVVIPTRRATAVALQSFTSHLLGDAGSPYLIGFISDLIRQSTKDSPLWEFLSLGYALMLCPFVVVLGGMFFLATALFFVSDRARAEQQVNQLAMPPASVKV

SEQ ID NO: 202 - protein, 549 aa, synthetic construct
  REGION 1..549: note = Homo sapiens
MMCLECASAAAGGAEEEEADAERRRRRRGAQRGAGGSGCCGARGAGGAGVSAAGDEVQTLSGSVRRAPTGPPGTPGTPGCAATAKGPGAQQPKPASLGRGRGAAAAILSLGNVLNYLDRYTVAGVLLDIQQHFGVKDRGAGLLQSVFICSFMVAAPIFGYLGDRFNRKVILSCGIFFWSAVTFSSSFIPQQYFWLLVLSRGLVGIGEASYSTIAPTIIGDLFTKNTRTLMLSVFYFAIPLGSGLGYITGSSVKQAAADWHWALRVSPVLGMITGTLILILVPATKRGHADQLGDQLKARTSWLRDMKALIRNRSYVFSSLATSAVSFATGALGMWIPLYLHRAQVVQKTAETCNSPPCGAKDSLIFGAITCFTGFLGVVTGAGATRWCRLKTQRADPLVCAVGMLGSAIFICLIFVAAKSSIVGAYICIFVGETLLFSNWAITADILMYVVIPTRRATAVALQSFTSHLLGDAGSPYLIGFISDLIRQSTKDSPLWEFLSLGYALMLCPFVVVLGGMFFLATALFFVSDRARAEQQVNQLAMPPASVKV

SEQ ID NO: 203 - protein, 549 aa, synthetic construct
  REGION 1..549: note = Homo sapiens
MMCLECASAAAGGAEEEEADAERRRRRRGAQRGAGGSGCCGARGAGGAGVSAAGDEVQTLSGSVRRAPTGPPGTPGTPGCAATAKGPGAQQPKPASLGRGRGAAAAILSLGNVLNYLDRYTVAGVLLDIQQHFGVKDRGAGLLQSVFICSFMVAAPIFGYLGDRFNRKVILSCGIFFWSAVTFSSSFIPQQYFWLLVLSRGLVGIGEASYSTIAPTIIGDLFTKNTRTLMLSVFYFAIPLGSGLGYITGSSVKQAAGAWHWALRVSPVLGMITGTLILILVPATKRGHADQLGDQLKARTSWLRDMKALIRNRSYVFSSLATSAVSFATGALGMWIPLYLHRAQVVQKTAETCNSPPCGAKDSLIFGAITCFTGFLGVVTGAGATRWCRLKTQRADPLVCAVGMLGSAIFICLIFVAAKSSIVGAYICIFVGETLLFSNWAITADILMYVVIPTRRATAVALQSFTSHLLGDAGSPYLIGFISDLIRQSTKDSPLWEFLSLGYALMLCPFVVVLGGMFFLATALFFVSDRARAEQQVNQLAMPPASVKV

SEQ ID NO: 204 - protein, 549 aa, synthetic construct
  REGION 1..549: note = Homo sapiens
MMCLECASAAAGGAEEEEADAERRRRRRGAQRGAGGSGCCGARGAGGAGVSAAGDEVQTLSGSVRRAPTGPPGTPGTPGCAATAKGPGAQQPKPASLGRGRGAAAAILSLGNVLNYLDRYTVAGVLLDIQQHFGVKDRGAGLLQSVFICSFMVAAPIFGYLGDRFNRKVILSCGIFFWSAVTFSSSFIPQQYFWLLVLSRGLVGIGEASYSTIAPTIIGDLFTKNTRTLMLSVFYFAIPLGSGLGYITGSSVKQAAGDAHWALRVSPVLGMITGTLILILVPATKRGHADQLGDQLKARTSWLRDMKALIRNRSYVFSSLATSAVSFATGALGMWIPLYLHRAQVVQKTAETCNSPPCGAKDSLIFGAITCFTGFLGVVTGAGATRWCRLKTQRADPLVCAVGMLGSAIFICLIFVAAKSSIVGAYICIFVGETLLFSNWAITADILMYVVIPTRRATAVALQSFTSHLLGDAGSPYLIGFISDLIRQSTKDSPLWEFLSLGYALMLCPFVVVLGGMFFLATALFFVSDRARAEQQVNQLAMPPASVKV

SEQ ID NO: 205 - protein, 549 aa, synthetic construct
  REGION 1..549: note = Homo sapiens
MMCLECASAAAGGAEEEEADAERRRRRRGAQRGAGGSGCCGARGAGGAGVSAAGDEVQTLSGSVRRAPTGPPGTPGTPGCAATAKGPGAQQPKPASLGRGRGAAAAILSLGNVLNYLDRYTVAGVLLDIQQHFGVKDRGAGLLQSVFICSFMVAAPIFGYLGDRFNRKVILSCGIFFWSAVTFSSSFIPQQYFWLLVLSRGLVGIGEASYSTIAPTIIGDLFTKNTRTLMLSVFYFAIPLGSGLGYITGSSVKQAAGDWAWALRVSPVLGMITGTLILILVPATKRGHADQLGDQLKARTSWLRDMKALIRNRSYVFSSLATSAVSFATGALGMWIPLYLHRAQVVQKTAETCNSPPCGAKDSLIFGAITCFTGFLGVVTGAGATRWCRLKTQRADPLVCAVGMLGSAIFICLIFVAAKSSIVGAYICIFVGETLLFSNWAITADILMYVVIPTRRATAVALQSFTSHLLGDAGSPYLIGFISDLIRQSTKDSPLWEFLSLGYALMLCPFVVVLGGMFFLATALFFVSDRARAEQQVNQLAMPPASVKV

SEQ ID NO: 206 - protein, 549 aa, synthetic construct
  REGION 1..549: note = Homo sapiens
MMCLECASAAAGGAEEEEADAERRRRRRGAQRGAGGSGCCGARGAGGAGVSAAGDEVQTLSGSVRRAPTGPPGTPGTPGCAATAKGPGAQQPKPASLGRGRGAAAAILSLGNVLNYLDRYTVAGVLLDIQQHFGVKDRGAGLLQSVFICSFMVAAPIFGYLGDRFNRKVILSCGIFFWSAVTFSSSFIPQQYFWLLVLSRGLVGIGEASYSTIAPTIIGDLFTKNTRTLMLSVFYFAIPLGSGLGYITGSSVKQFAGDWHWALRVSPVLGMITGTLILILVPATKRGHADQLGDQLKARTSWLRDMKALIRNRSYVFSSLATSAVSFATGALGMWIPLYLHRAQVVQKTAETCNSPPCGAKDSLIFGAITCFTGFLGVVTGAGATRWCRLKTQRADPLVCAVGMLGSAIFICLIFVAAKSSIVGAYICIFVGETLLFSNWAITADILMYVVIPTRRATAVALQSFTSHLLGDAGSPYLIGFISDLIRQSTKDSPLWEFLSLGYALMLCPFVVVLGGMFFLATALFFVSDRARAEQQVNQLAMPPASVKV

SEQ ID NO: 207 - protein, 549 aa, synthetic construct
  REGION 1..549: note = Homo sapiens
MMCLECASAAAGGAEEEEADAERRRRRRGAQRGAGGSGCCGARGAGGAGVSAAGDEVQTLSGSVRRAPTGPPGTPGTPGCAATAKGPGAQQPKPASLGRGRGAAAAILSLGNVLNYLDRYTVAGVLLDIQQHFGVKDRGAGLLQSVFICSFMVAAPIFGYLGDRFNRKVILSCGIFFWSAVTFSSSFIPQQYFWLLVLSRGLVGIGEASYSTIAPTIIGDLFTKNTRTLMLSVFYFAIPLGSGLGYITGSSVKQAFGDWHWALRVSPVLGMITGTLILILVPATKRGHADQLGDQLKARTSWLRDMKALIRNRSYVFSSLATSAVSFATGALGMWIPLYLHRAQVVQKTAETCNSPPCGAKDSLIFGAITCFTGFLGVVTGAGATRWCRLKTQRADPLVCAVGMLGSAIFICLIFVAAKSSIVGAYICIFVGETLLFSNWAITADILMYVVIPTRRATAVALQSFTSHLLGDAGSPYLIGFISDLIRQSTKDSPLWEFLSLGYALMLCPFVVVLGGMFFLATALFFVSDRARAEQQVNQLAMPPASVKV

SEQ ID NO: 208 - DNA, 1650 bp, synthetic construct
  misc_feature 1..1650: note = Homo sapiens
  source 1..1650: mol_type = other DNA
atgatgtgcctggaatgcgcctcggcggcggcgggcggcgcggaggaggaggaggcggacgcggagcggcggcgccggcgccggggggcgcagcgaggggctggcggtagcggttgctgcggggcgcggggcgcgggcggcgctggagtctcggccgcgggcgatgaggtgcagacgctgtcgggcagcgtaaggcgggccccgaccggaccccccggcacccccggcacccccggctgcgcagctactgcaaagggccccggcgctcagcagcccaaaccggccagcttgggccgcgggcggggggcagccgccgccatcctcagcttgggcaacgtgctcaactacctggacaggtacaccgtggcaggcgtccttgccgacatccagcagcactttggggtcaaggaccgaggcgccggcctgctgcagtcagtgttcatctgtagcttcatggtggctgcccccatcttcggctacctgggcgaccgcttcaacaggaaggtgattctcagctgcggcattttcttctggtcggccgtcaccttctccagctccttcattccccagcagtacttctggctgctggtcctgtcccgggggctggtgggcatcggggaggccagctactccaccatcgcccccactatcattggcgacctcttcaccaagaacacgcgtacgctcatgctgtccgtcttctacttcgccatcccactgggcagtggcctgggctacattactggctccagcgtgaagcaggcagccggagactggcactgggcattgcgggtgtcccctgtcctgggcatgatcacaggaacactcatcctcattctggtcccagccactaaaaggggtcatgccgaccagctcggggaccagctcaaggcccggacctcatggctccgagatatgaaggccctgattcgaaaccgcagctacgtcttctcctccctggccacgtcggctgtctccttcgccacgggggccctgggcatgtggatcccgctctacctgcaccgcgcccaagttgtgcagaagacagcagagacgtgcaacagcccgccctgtggggccaaggacagcctcatctttggggccatcacctgctttacgggatttctgggcgtggtcacgggggcaggagccacgcgctggtgccgcctgaagacccagcgggccgacccactggtgtgtgccgtgggcatgctgggctctgccatcttcatctgcctgatcttcgtggctgccaagagcagcatcgtaggagcctatatctgtatcttcgtcggggagacgctgctgttttctaactgggccatcactgcagacatcctcatgtacgtggtcatccccacgcggcgcgccactgccgtggccttgcagagcttcacctcccacctgctgggggacgccgggagcccctacctcattggctttatctcagacctgatccgccagagcactaaggactccccgctctgggagttcctgagcctgggctacgcgctcatgctctgccctttcgtcgtggtcctgggcggcatgttcttcctcgccactgcgctcttcttcgtcagcgaccgcgccagggctgagcagcaggtgaaccagctggcgatgccgcccgcatctgtgaaagtctga

SEQ ID NO: 209 - DNA, 1650 bp, synthetic construct
  misc_feature 1..1650: note = Homo sapiens
  source 1..1650: mol_type = other DNA
atgatgtgcctggaatgcgcctcggcggcggcgggcggcgcggaggaggaggaggcggacgcggagcggcggcgccggcgccggggggcgcagcgaggggctggcggtagcggttgctgcggggcgcggggcgcgggcggcgctggagtctcggccgcgggcgatgaggtgcagacgctgtcgggcagcgtaaggcgggccccgaccggaccccccggcacccccggcacccccggctgcgcagctactgcaaagggccccggcgctcagcagcccaaaccggccagcttgggccgcgggcggggggcagccgccgccatcctcagcttgggcaacgtgctcaactacctggacaggtacaccgtggcaggcgtccttctggccatccagcagcactttggggtcaaggaccgaggcgccggcctgctgcagtcagtgttcatctgtagcttcatggtggctgcccccatcttcggctacctgggcgaccgcttcaacaggaaggtgattctcagctgcggcattttcttctggtcggccgtcaccttctccagctccttcattccccagcagtacttctggctgctggtcctgtcccgggggctggtgggcatcggggaggccagctactccaccatcgcccccactatcattggcgacctcttcaccaagaacacgcgtacgctcatgctgtccgtcttctacttcgccatcccactgggcagtggcctgggctacattactggctccagcgtgaagcaggcagccggagactggcactgggcattgcgggtgtcccctgtcctgggcatgatcacaggaacactcatcctcattctggtcccagccactaaaaggggtcatgccgaccagctcggggaccagctcaaggcccggacctcatggctccgagatatgaaggccctgattcgaaaccgcagctacgtcttctcctccctggccacgtcggctgtctccttcgccacgggggccctgggcatgtggatcccgctctacctgcaccgcgcccaagttgtgcagaagacagcagagacgtgcaacagcccgccctgtggggccaaggacagcctcatctttggggccatcacctgctttacgggatttctgggcgtggtcacgggggcaggagccacgcgctggtgccgcctgaagacccagcgggccgacccactggtgtgtgccgtgggcatgctgggctctgccatcttcatctgcctgatcttcgtggctgccaagagcagcatcgtaggagcctatatctgtatcttcgtcggggagacgctgctgttttctaactgggccatcactgcagacatcctcatgtacgtggtcatccccacgcggcgcgccactgccgtggccttgcagagcttcacctcccacctgctgggggacgccgggagcccctacctcattggctttatctcagacctgatccgccagagcactaaggactccccgctctgggagttcctgagcctgggctacgcgctcatgctctgccctttcgtcgtggtcctgggcggcatgttcttcctcgccactgcgctcttcttcgtcagcgaccgcgccagggctgagcagcaggtgaaccagctggcgatgccgcccgcatctgtgaaagtctga

SEQ ID NO: 210 - DNA, 1650 bp, synthetic construct
  misc_feature 1..1650: note = Homo sapiens
  source 1..1650: mol_type = other DNA
atgatgtgcctggaatgcgcctcggcggcggcgggcggcgcggaggaggaggaggcggacgcggagcggcggcgccggcgccggggggcgcagcgaggggctggcggtagcggttgctgcggggcgcggggcgcgggcggcgctggagtctcggccgcgggcgatgaggtgcagacgctgtcgggcagcgtaaggcgggccccgaccggaccccccggcacccccggcacccccggctgcgcagctactgcaaagggccccggcgctcagcagcccaaaccggccagcttgggccgcgggcggggggcagccgccgccatcctcagcttgggcaacgtgctcaactacctggacaggtacaccgtggcaggcgtccttctggacgcccagcagcactttggggtcaaggaccgaggcgccggcctgctgcagtcagtgttcatctgtagcttcatggtggctgcccccatcttcggctacctgggcgaccgcttcaacaggaaggtgattctcagctgcggcattttcttctggtcggccgtcaccttctccagctccttcattccccagcagtacttctggctgctggtcctgtcccgggggctggtgggcatcggggaggccagctactccaccatcgcccccactatcattggcgacctcttcaccaagaacacgcgtacgctcatgctgtccgtcttctacttcgccatcccactgggcagtggcctgggctacattactggctccagcgtgaagcaggcagccggagactggcactgggcattgcgggtgtcccctgtcctgggcatgatcacaggaacactcatcctcattctggtcccagccactaaaaggggtcatgccgaccagctcggggaccagctcaaggcccggacctcatggctccgagatatgaaggccctgattcgaaaccgcagctacgtcttctcctccctggccacgtcggctgtctccttcgccacgggggccctgggcatgtggatcccgctctacctgcaccgcgcccaagttgtgcagaagacagcagagacgtgcaacagcccgccctgtggggccaaggacagcctcatctttggggccatcacctgctttacgggatttctgggcgtggtcacgggggcaggagccacgcgctggtgccgcctgaagacccagcgggccgacccactggtgtgtgccgtgggcatgctgggctctgccatcttcatctgcctgatcttcgtggctgccaagagcagcatcgtaggagcctatatctgtatcttcgtcggggagacgctgctgttttctaactgggccatcactgcagacatcctcatgtacgtggtcatccccacgcggcgcgccactgccgtggccttgcagagcttcacctcccacctgctgggggacgccgggagcccctacctcattggctttatctcagacctgatccgccagagcactaaggactccccgctctgggagttcctgagcctgggctacgcgctcatgctctgccctttcgtcgtggtcctgggcggcatgttcttcctcgccactgcgctcttcttcgtcagcgaccgcgccagggctgagcagcaggtgaaccagctggcgatgccgcccgcatctgtgaaagtctga

SEQ ID NO: 211 - DNA, 1650 bp, synthetic construct
  misc_feature 1..1650: note = Homo sapiens
  source 1..1650: mol_type = other DNA
atgatgtgcctggaatgcgcctcggcggcggcgggcggcgcggaggaggaggaggcggacgcggagcggcggcgccggcgccggggggcgcagcgaggggctggcggtagcggttgctgcggggcgcggggcgcgggcggcgctggagtctcggccgcgggcgatgaggtgcagacgctgtcgggcagcgtaaggcgggccccgaccggaccccccggcacccccggcacccccggctgcgcagctactgcaaagggccccggcgctcagcagcccaaaccggccagcttgggccgcgggcggggggcagccgccgccatcctcagcttgggcaacgtgctcaactacctggacaggtacaccgtggcaggcgtccttctggacatcgcccagcactttggggtcaaggaccgaggcgccggcctgctgcagtcagtgttcatctgtagcttcatggtggctgcccccatcttcggctacctgggcgaccgcttcaacaggaaggtgattctcagctgcggcattttcttctggtcggccgtcaccttctccagctccttcattccccagcagtacttctggctgctggtcctgtcccgggggctggtgggcatcggggaggccagctactccaccatcgcccccactatcattggcgacctcttcaccaagaacacgcgtacgctcatgctgtccgtcttctacttcgccatcccactgggcagtggcctgggctacattactggctccagcgtgaagcaggcagccggagactggcactgggcattgcgggtgtcccctgtcctgggcatgatcacaggaacactcatcctcattctggtcccagccactaaaaggggtcatgccgaccagctcggggaccagctcaaggcccggacctcatggctccgagatatgaaggccctgattcgaaaccgcagctacgtcttctcctccctggccacgtcggctgtctccttcgccacgggggccctgggcatgtggatcccgctctacctgcaccgcgcccaagttgtgcagaagacagcagagacgtgcaacagcccgccctgtggggccaaggacagcctcatctttggggccatcacctgctttacgggatttctgggcgtggtcacgggggcaggagccacgcgctggtgccgcctgaagacccagcgggccgacccactggtgtgtgccgtgggcatgctgggctctgccatcttcatctgcctgatcttcgtggctgccaagagcagcatcgtaggagcctatatctgtatcttcgtcggggagacgctgctgttttctaactgggccatcactgcagacatcctcatgtacgtggtcatccccacgcggcgcgccactgccgtggccttgcagagcttcacctcccacctgctgggggacgccgggagcccctacctcattggctttatctcagacctgatccgccagagcactaaggactccccgctctgggagttcctgagcctgggctacgcgctcatgctctgccctttcgtcgtggtcctgggcggcatgttcttcctcgccactgcgctcttcttcgtcagcgaccgcgccagggctgagcagcaggtgaaccagctggcgatgccgcccgcatctgtgaaagtctga

SEQ ID NO: 212 - DNA, 1650 bp, synthetic construct
  misc_feature 1..1650: note = Homo sapiens
  source 1..1650: mol_type = other DNA
atgatgtgcctggaatgcgcctcggcggcggcgggcggcgcggaggaggaggaggcggacgcggagcggcggcgccggcgccggggggcgcagcgaggggctggcggtagcggttgctgcggggcgcggggcgcgggcggcgctggagtctcggccgcgggcgatgaggtgcagacgctgtcgggcagcgtaaggcgggccccgaccggaccccccggcacccccggcacccccggctgcgcagctactgcaaagggccccggcgctcagcagcccaaaccggccagcttgggccgcgggcggggggcagccgccgccatcctcagcttgggcaacgtgctcaactacctggacaggtacaccgtggcaggcgtccttctggacatccaggcccactttggggtcaaggaccgaggcgccggcctgctgcagtcagtgttcatctgtagcttcatggtggctgcccccatcttcggctacctgggcgaccgcttcaacaggaaggtgattctcagctgcggcattttcttctggtcggccgtcaccttctccagctccttcattccccagcagtacttctggctgctggtcctgtcccgggggctggtgggcatcggggaggccagctactccaccatcgcccccactatcattggcgacctcttcaccaagaacacgcgtacgctcatgctgtccgtcttctacttcgccatcccactgggcagtggcctgggctacattactggctccagcgtgaagcaggcagccggagactggcactgggcattgcgggtgtcccctgtcctgggcatgatcacaggaacactcatcctcattctggtcccagccactaaaaggggtcatgccgaccagctcggggaccagctcaaggcccggacctcatggctccgagatatgaaggccctgattcgaaaccgcagctacgtcttctcctccctggccacgtcggctgtctccttcgccacgggggccctgggcatgtggatcccgctctacctgcaccgcgcccaagttgtgcagaagacagcagagacgtgcaacagcccgccctgtggggccaaggacagcctcatctttggggccatcacctgctttacgggatttctgggcgtggtcacgggggcaggagccacgcgctggtgccgcctgaagacccagcgggccgacccactggtgtgtgccgtgggcatgctgggctctgccatcttcatctgcctgatcttcgtggctgccaagagcagcatcgtaggagcctatatctgtatcttcgtcggggagacgctgctgttttctaactgggccatcactgcagacatcctcatgtacgtggtcatccccacgcggcgcgccactgccgtggccttgcagagcttcacctcccacctgctgggggacgccgggagcccctacctcattggctttatctcagacctgatccgccagagcactaaggactccccgctctgggagttcctgagcctgggctacgcgctcatgctctgccctttcgtcgtggtcctgggcggcatgttcttcctcgccactgcgctcttcttcgtcagcgaccgcgccagggctgagcagcaggtgaaccagctggcgatgccgcccgcatctgtgaaagtctga

SEQ ID NO: 213 - DNA, 1650 bp, synthetic construct
  misc_feature 1..1650: note = Homo sapiens
  source 1..1650: mol_type = other DNA
atgatgtgcctggaatgcgcctcggcggcggcgggcggcgcggaggaggaggaggcggacgcggagcggcggcgccggcgccggggggcgcagcgaggggctggcggtagcggttgctgcggggcgcggggcgcgggcggcgctggagtctcggccgcgggcgatgaggtgcagacgctgtcgggcagcgtaaggcgggccccgaccggaccccccggcacccccggcacccccggctgcgcagctactgcaaagggccccggcgctcagcagcccaaaccggccagcttgggccgcgggcggggggcagccgccgccatcctcagcttgggcaacgtgctcaactacctggacaggtacaccgtggcaggcgtccttctggacatccagcaggcctttggggtcaaggaccgaggcgccggcctgctgcagtcagtgttcatctgtagcttcatggtggctgcccccatcttcggctacctgggcgaccgcttcaacaggaaggtgattctcagctgcggcattttcttctggtcggccgtcaccttctccagctccttcattccccagcagtacttctggctgctggtcctgtcccgggggctggtgggcatcggggaggccagctactccaccatcgcccccactatcattggcgacctcttcaccaagaacacgcgtacgctcatgctgtccgtcttctacttcgccatcccactgggcagtggcctgggctacattactggctccagcgtgaagcaggcagccggagactggcactgggcattgcgggtgtcccctgtcctgggcatgatcacaggaacactcatcctcattctggtcccagccactaaaaggggtcatgccgaccagctcggggaccagctcaaggcccggacctcatggctccgagatatgaaggccctgattcgaaaccgcagctacgtcttctcctccctggccacgtcggctgtctccttcgccacgggggccctgggcatgtggatcccgctctacctgcaccgcgcccaagttgtgcagaagacagcagagacgtgcaacagcccgccctgtggggccaaggacagcctcatctttggggccatcacctgctttacgggatttctgggcgtggtcacgggggcaggagccacgcgctggtgccgcctgaagacccagcgggccgacccactggtgtgtgccgtgggcatgctgggctctgccatcttcatctgcctgatcttcgtggctgccaagagcagcatcgtaggagcctatatctgtatcttcgtcggggagacgctgctgttttctaactgggccatcactgcagacatcctcatgtacgtggtcatccccacgcggcgcgccactgccgtggccttgcagagcttcacctcccacctgctgggggacgccgggagcccctacctcattggctttatctcagacctgatccgccagagcactaaggactccccgctctgggagttcctgagcctgggctacgcgctcatgctctgccctttcgtcgtggtcctgggcggcatgttcttcctcgccactgcgctcttcttcgtcagcgaccgcgccagggctgagcagcaggtgaaccagctggcgatgccgcccgcatctgtgaaagtctga

SEQ ID NO: 214 - DNA, 1650 bp, synthetic construct
  misc_feature 1..1650: note = Homo sapiens
  source 1..1650: mol_type = other DNA
atgatgtgcctggaatgcgcctcggcggcggcgggcggcgcggaggaggaggaggcggacgcggagcggcggcgccggcgccggggggcgcagcgaggggctggcggtagcggttgctgcggggcgcggggcgcgggcggcgctggagtctcggccgcgggcgatgaggtgcagacgctgtcgggcagcgtaaggcgggccccgaccggaccccccggcacccccggcacccccggctgcgcagctactgcaaagggccccggcgctcagcagcccaaaccggccagcttgggccgcgggcggggggcagccgccgccatcctcagcttgggcaacgtgctcaactacctggacaggtacaccgtggcaggcgtccttctggacatccagcagcacgccggggtcaaggaccgaggcgccggcctgctgcagtcagtgttcatctgtagcttcatggtggctgcccccatcttcggctacctgggcgaccgcttcaacaggaaggtgattctcagctgcggcattttcttctggtcggccgtcaccttctccagctccttcattccccagcagtacttctggctgctggtcctgtcccgggggctggtgggcatcggggaggccagctactccaccatcgcccccactatcattggcgacctcttcaccaagaacacgcgtacgctcatgctgtccgtcttctacttcgccatcccactgggcagtggcctgggctacattactggctccagcgtgaagcaggcagccggagactggcactgggcattgcgggtgtcccctgtcctgggcatgatcacaggaacactcatcctcattctggtcccagccactaaaaggggtcatgccgaccagctcggggaccagctcaaggcccggacctcatggctccgagatatgaaggccctgattcgaaaccgcagctacgtcttctcctccctggccacgtcggctgtctccttcgccacgggggccctgggcatgtggatcccgctctacctgcaccgcgcccaagttgtgcagaagacagcagagacgtgcaacagcccgccctgtggggccaaggacagcctcatctttggggccatcacctgctttacgggatttctgggcgtggtcacgggggcaggagccacgcgctggtgccgcctgaagacccagcgggccgacccactggtgtgtgccgtgggcatgctgggctctgccatcttcatctgcctgatcttcgtggctgccaagagcagcatcgtaggagcctatatctgtatcttcgtcggggagacgctgctgttttctaactgggccatcactgcagacatcctcatgtacgtggtcatccccacgcggcgcgccactgccgtggccttgcagagcttcacctcccacctgctgggggacgccgggagcccctacctcattggctttatctcagacctgatccgccagagcactaaggactccccgctctgggagttcctgagcctgggctacgcgctcatgctctgccctttcgtcgtggtcctgggcggcatgttcttcctcgccactgcgctcttcttcgtcagcgaccgcgccagggctgagcagcaggtgaaccagctggcgatgccgcccgcatctgtgaaagtctga

SEQ ID NO: 215 - DNA, 1650 bp, synthetic construct
  misc_feature 1..1650: note = Homo sapiens
  source 1..1650: mol_type = other DNA
atgatgtgcctggaatgcgcctcggcggcggcgggcggcgcggaggaggaggaggcggacgcggagcggcggcgccggcgccggggggcgcagcgaggggctggcggtagcggttgctgcggggcgcggggcgcgggcggcgctggagtctcggccgcgggcgatgaggtgcagacgctgtcgggcagcgtaaggcgggccccgaccggaccccccggcacccccggcacccccggctgcgcagctactgcaaagggccccggcgctcagcagcccaaaccggccagcttgggccgcgggcggggggcagccgccgccatcctcagcttgggcaacgtgctcaactacctggacaggtacaccgtggcaggcgtccttctggacatccagcagcactttgccgtcaaggaccgaggcgccggcctgctgcagtcagtgttcatctgtagcttcatggtggctgcccccatcttcggctacctgggcgaccgcttcaacaggaaggtgattctcagctgcggcattttcttctggtcggccgtcaccttctccagctccttcattccccagcagtacttctggctgctggtcctgtcccgggggctggtgggcatcggggaggccagctactccaccatcgcccccactatcattggcgacctcttcaccaagaacacgcgtacgctcatgctgtccgtcttctacttcgccatcccactgggcagtggcctgggctacattactggctccagcgtgaagcaggcagccggagactggcactgggcattgcgggtgtcccctgtcctgggcatgatcacaggaacactcatcctcattctggtcccagccactaaaaggggtcatgccgaccagctcggggaccagctcaaggcccggacctcatggctccgagatatgaaggccctgattcgaaaccgcagctacgtcttctcctccctggccacgtcggctgtctccttcgccacgggggccctgggcatgtggatcccgctctacctgcaccgcgcccaagttgtgcagaagacagcagagacgtgcaacagcccgccctgtggggccaaggacagcctcatctttggggccatcacctgctttacgggatttctgggcgtggtcacgggggcaggagccacgcgctggtgccgcctgaagacccagcgggccgacccactggtgtgtgccgtgggcatgctgggctctgccatcttcatctgcctgatcttcgtggctgccaagagcagcatcgtaggagcctatatctgtatcttcgtcggggagacgctgctgttttctaactgggccatcactgcagacatcctcatgtacgtggtcatccccacgcggcgcgccactgccgtggccttgcagagcttcacctcccacctgctgggggacgccgggagcccctacctcattggctttatctcagacctgatccgccagagcactaaggactccccgctctgggagttcctgagcctgggctacgcgctcatgctctgccctttcgtcgtggtcctgggcggcatgttcttcctcgccactgcgctcttcttcgtcagcgaccgcgccagggctgagcagcaggtgaaccagctggcgatgccgcccgcatctgtgaaagtctga

SEQ ID NO: 216 - DNA, 1650 bp, synthetic construct
  misc_feature 1..1650: note = Homo sapiens
  source 1..1650: mol_type = other DNA
atgatgtgcctggaatgcgcctcggcggcggcgggcggcgcggaggaggaggaggcggacgcggagcggcggcgccggcgccggggggcgcagcgaggggctggcggtagcggttgctgcggggcgcggggcgcgggcggcgctggagtctcggccgcgggcgatgaggtgcagacgctgtcgggcagcgtaaggcgggccccgaccggaccccccggcacccccggcacccccggctgcgcagctactgcaaagggccccggcgctcagcagcccaaaccggccagcttgggccgcgggcggggggcagccgccgccatcctcagcttgggcaacgtgctcaactacctggacaggtacaccgtggcaggcgtccttctggacatccagcagcactttggggccaaggaccgaggcgccggcctgctgcagtcagtgttcatctgtagcttcatggtggctgcccccatcttcggctacctgggcgaccgcttcaacaggaaggtgattctcagctgcggcattttcttctggtcggccgtcaccttctccagctccttcattccccagcagtacttctggctgctggtcctgtcccgggggctggtgggcatcggggaggccagctactccaccatcgcccccactatcattggcgacctcttcaccaagaacacgcgtacgctcatgctgtccgtcttctacttcgccatcccactgggcagtggcctgggctacattactggctccagcgtgaagcaggcagccggagactggcactgggcattgcgggtgtcccctgtcctgggcatgatcacaggaacactcatcctcattctggtcccagccactaaaaggggtcatgccgaccagctcggggaccagctcaaggcccggacctcatggctccgagatatgaaggccctgattcgaaaccgcagctacgtcttctcctccctggccacgtcggctgtctccttcgccacgggggccctgggcatgtggatcccgctctacctgcaccgcgcccaagttgtgcagaagacagcagagacgtgcaacagcccgccctgtggggccaaggacagcctcatctttggggccatcacctgctttacgggatttctgggcgtggtcacgggggcaggagccacgcgctggtgccgcctgaagacccagcgggccgacccactggtgtgtgccgtgggcatgctgggctctgccatcttcatctgcctgatcttcgtggctgccaagagcagcatcgtaggagcctatatctgtatcttcgtcggggagacgctgctgttttctaactgggccatcactgcagacatcctcatgtacgtggtcatccccacgcggcgcgccactgccgtggccttgcagagcttcacctcccacctgctgggggacgccgggagcccctacctcattggctttatctcagacctgatccgccagagcactaaggactccccgctctgggagttcctgagcctgggctacgcgctcatgctctgccctttcgtcgtggtcctgggcggcatgttcttcctcgccactgcgctcttcttcgtcagcgaccgcgccagggctgagcagcaggtgaaccagctggcgatgccgcccgcatctgtgaaagtctga

SEQ ID NO: 217 - DNA, 1650 bp, synthetic construct
  misc_feature 1..1650: note = Homo sapiens
  source 1..1650: mol_type = other DNA
atgatgtgcctggaatgcgcctcggcggcggcgggcggcgcggaggaggaggaggcggacgcggagcggcggcgccggcgccggggggcgcagcgaggggctggcggtagcggttgctgcggggcgcggggcgcgggcggcgctggagtctcggccgcgggcgatgaggtgcagacgctgtcgggcagcgtaaggcgggccccgaccggaccccccggcacccccggcacccccggctgcgcagctactgcaaagggccccggcgctcagcagcccaaaccggccagcttgggccgcgggcggggggcagccgccgccatcctcagcttgggcaacgtgctcaactacctggacaggtacaccgtggcaggcgtccttctggacatccagcagcactttggggtcgccgaccgaggcgccggcctgctgcagtcagtgttcatctgtagcttcatggtggctgcccccatcttcggctacctgggcgaccgcttcaacaggaaggtgattctcagctgcggcattttcttctggtcggccgtcaccttctccagctccttcattccccagcagtacttctggctgctggtcctgtcccgggggctggtgggcatcggggaggccagctactccaccatcgcccccactatcattggcgacctcttcaccaagaacacgcgtacgctcatgctgtccgtcttctacttcgccatcccactgggcagtggcctgggctacattactggctccagcgtgaagcaggcagccggagactggcactgggcattgcgggtgtcccctgtcctgggcatgatcacaggaacactcatcctcattctggtcccagccactaaaaggggtcatgccgaccagctcggggaccagctcaaggcccggacctcatggctccgagatatgaaggccctgattcgaaaccgcagctacgtcttctcctccctggccacgtcggctgtctccttcgccacgggggccctgggcatgtggatcccgctctacctgcaccgcgcccaagttgtgcagaagacagcagagacgtgcaacagcccgccctgtggggccaaggacagcctcatctttggggccatcacctgctttacgggatttctgggcgtggtcacgggggcaggagccacgcgctggtgccgcctgaagacccagcgggccgacccactggtgtgtgccgtgggcatgctgggctctgccatcttcatctgcctgatcttcgtggctgccaagagcagcatcgtaggagcctatatctgtatcttcgtcggggagacgctgctgttttctaactgggccatcactgcagacatcctcatgtacgtggtcatccccacgcggcgcgccactgccgtggccttgcagagcttcacctcccacctgctgggggacgccgggagcccctacctcattggctttatctcagacctgatccgccagagcactaaggactccccgctctgggagttcctgagcctgggctacgcgctcatgctctgccctttcgtcgtggtcctgggcggcatgttcttcctcgccactgcgctcttcttcgtcagcgaccgcgccagggctgagcagcaggtgaaccagctggcgatgccgcccgcatctgtgaaagtctga

SEQ ID NO: 218 - DNA, 1650 bp, synthetic construct
  misc_feature 1..1650: note = Homo sapiens
  source 1..1650: mol_type = other DNA
atgatgtgcctggaatgcgcctcggcggcggcgggcggcgcggaggaggaggaggcggacgcggagcggcggcgccggcgccggggggcgcagcgaggggctggcggtagcggttgctgcggggcgcggggcgcgggcggcgctggagtctcggccgcgggcgatgaggtgcagacgctgtcgggcagcgtaaggcgggccccgaccggaccccccggcacccccggcacccccggctgcgcagctactgcaaagggccccggcgctcagcagcccaaaccggccagcttgggccgcgggcggggggcagccgccgccatcctcagcttgggcaacgtgctcaactacctggacaggtacaccgtggcaggcgtccttctggacatccagcagcactttggggtcaaggcccgaggcgccggcctgctgcagtcagtgttcatctgtagcttcatggtggctgcccccatcttcggctacctgggcgaccgcttcaacaggaaggtgattctcagctgcggcattttcttctggtcggccgtcaccttctccagctccttcattccccagcagtacttctggctgctggtcctgtcccgggggctggtgggcatcggggaggccagctactccaccatcgcccccactatcattggcgacctcttcaccaagaacacgcgtacgctcatgctgtccgtcttctacttcgccatcccactgggcagtggcctgggctacattactggctccagcgtgaagcaggcagccggagactggcactgggcattgcgggtgtcccctgtcctgggcatgatcacaggaacactcatcctcattctggtcccagccactaaaaggggtcatgccgaccagctcggggaccagctcaaggcccggacctcatggctccgagatatgaaggccctgattcgaaaccgcagctacgtcttctcctccctggccacgtcggctgtctccttcgccacgggggccctgggcatgtggatcccgctctacctgcaccgcgcccaagttgtgcagaagacagcagagacgtgcaacagcccgccctgtggggccaaggacagcctcatctttggggccatcacctgctttacgggatttctgggcgtggtcacgggggcaggagccacgcgctggtgccgcctgaagacccagcgggccgacccactggtgtgtgccgtgggcatgctgggctctgccatcttcatctgcctgatcttcgtggctgccaagagcagcatcgtaggagcctatatctgtatcttcgtcggggagacgctgctgttttctaactgggccatcactgcagacatcctcatgtacgtggtcatccccacgcggcgcgccactgccgtggccttgcagagcttcacctcccacctgctgggggacgccgggagcccctacctcattggctttatctcagacctgatccgccagagcactaaggactccccgctctgggagttcctgagcctgggctacgcgctcatgctctgccctttcgtcgtggtcctgggcggcatgttcttcctcgccactgcgctcttcttcgtcagcgaccgcgccagggctgagcagcaggtgaaccagctggcgatgccgcccgcatctgtgaaagtctga

SEQ ID NO: 219 - DNA, 1650 bp, synthetic construct
  misc_feature 1..1650: note = Homo sapiens
  source 1..1650: mol_type = other DNA
atgatgtgcctggaatgcgcctcggcggcggcgggcggcgcggaggaggaggaggcggacgcggagcggcggcgccggcgccggggggcgcagcgaggggctggcggtagcggttgctgcggggcgcggggcgcgggcggcgctggagtctcggccgcgggcgatgaggtgcagacgctgtcgggcagcgtaaggcgggccccgaccggaccccccggcacccccggcacccccggctgcgcagctactgcaaagggccccggcgctcagcagcccaaaccggccagcttgggccgcgggcggggggcagccgccgccatcctcagcttgggcaacgtgctcaactacctggacaggtacaccgtggcaggcgtccttctggacatccagcagcactttggggtcaaggacgccggcgccggcctgctgcagtcagtgttcatctgtagcttcatggtggctgcccccatcttcggctacctgggcgaccgcttcaacaggaaggtgattctcagctgcggcattttcttctggtcggccgtcaccttctccagctccttcattccccagcagtacttctggctgctggtcctgtcccgggggctggtgggcatcggggaggccagctactccaccatcgcccccactatcattggcgacctcttcaccaagaacacgcgtacgctcatgctgtccgtcttctacttcgccatcccactgggcagtggcctgggctacattactggctccagcgtgaagcaggcagccggagactggcactgggcattgcgggtgtcccctgtcctgggcatgatcacaggaacactcatcctcattctggtcccagccactaaaaggggtcatgccgaccagctcggggaccagctcaaggcccggacctcatggctccgagatatgaaggccctgattcgaaaccgcagctacgtcttctcctccctggccacgtcggctgtctccttcgccacgggggccctgggcatgtggatcccgctctacctgcaccgcgcccaagttgtgcagaagacagcagagacgtgcaacagcccgccctgtggggccaaggacagcctcatctttggggccatcacctgctttacgggatttctgggcgtggtcacgggggcaggagccacgcgctggtgccgcctgaagacccagcgggccgacccactggtgtgtgccgtgggcatgctgggctctgccatcttcatctgcctgatcttcgtggctgccaagagcagcatcgtaggagcctatatctgtatcttcgtcggggagacgctgctgttttctaactgggccatcactgcagacatcctcatgtacgtggtcatccccacgcggcgcgccactgccgtggccttgcagagcttcacctcccacctgctgggggacgccgggagcccctacctcattggctttatctcagacctgatccgccagagcactaaggactccccgctctgggagttcctgagcctgggctacgcgctcatgctctgccctttcgtcgtggtcctgggcggcatgttcttcctcgccactgcgctcttcttcgtcagcgaccgcgccagggctgagcagcaggtgaaccagctggcgatgccgcccgcatctgtgaaagtctga

SEQ ID NO: 220 - DNA, 1650 bp, synthetic construct
  misc_feature 1..1650: note = Homo sapiens
  source 1..1650: mol_type = other DNA
atgatgtgcctggaatgcgcctcggcggcggcgggcggcgcggaggaggaggaggcggacgcggagcggcggcgccggcgccggggggcgcagcgaggggctggcggtagcggttgctgcggggcgcggggcgcgggcggcgctggagtctcggccgcgggcgatgaggtgcagacgctgtcgggcagcgtaaggcgggccccgaccggaccccccggcacccccggcacccccggctgcgcagctactgcaaagggccccggcgctcagcagcccaaaccggccagcttgggccgcgggcggggggcagccgccgccatcctcagcttgggcaacgtgctcaactacctggacaggtacaccgtggcaggcgtccttctggacatccagcagcactttggggtcaaggaccgagccgccggcctgctgcagtcagtgttcatctgtagcttcatggtggctgcccccatcttcggctacctgggcgaccgcttcaacaggaaggtgattctcagctgcggcattttcttctggtcggccgtcaccttctccagctccttcattccccagcagtacttctggctgctggtcctgtcccgggggctggtgggcatcggggaggccagctactccaccatcgcccccactatcattggcgacctcttcaccaagaacacgcgtacgctcatgctgtccgtcttctacttcgccatcccactgggcagtggcctgggctacattactggctccagcgtgaagcaggcagccggagactggcactgggcattgcgggtgtcccctgtcctgggcatgatcacaggaacactcatcctcattctggtcccagccactaaaaggggtcatgccgaccagctcggggaccagctcaaggcccggacctcatggctccgagatatgaaggccctgattcgaaaccgcagctacgtcttctcctccctggccacgtcggctgtctccttcgccacgggggccctgggcatgtggatcccgctctacctgcaccgcgcccaagttgtgcagaagacagcagagacgtgcaacagcccgccctgtggggccaaggacagcctcatctttggggccatcacctgctttacgggatttctgggcgtggtcacgggggcaggagccacgcgctggtgccgcctgaagacccagcgggccgacccactggtgtgtgccgtgggcatgctgggctctgccatcttcatctgcctgatcttcgtggctgccaagagcagcatcgtaggagcctatatctgtatcttcgtcggggagacgctgctgttttctaactgggccatcactgcagacatcctcatgtacgtggtcatccccacgcggcgcgccactgccgtggccttgcagagcttcacctcccacctgctgggggacgccgggagcccctacctcattggctttatctcagacctgatccgccagagcactaaggactccccgctctgggagttcctgagcctgggctacgcgctcatgctctgccctttcgtcgtggtcctgggcggcatgttcttcctcgccactgcgctcttcttcgtcagcgaccgcgccagggctgagcagcaggtgaaccagctggcgatgccgcccgcatctgtgaaagtctga

SEQ ID NO: 221 - DNA, 1650 bp, synthetic construct
  misc_feature 1..1650: note = Homo sapiens
  source 1..1650: mol_type = other DNA
atgatgtgcctggaatgcgcctcggcggcggcgggcggcgcggaggaggaggaggcggacgcggagcggcggcgccggcgccggggggcgcagcgaggggctggcggtagcggttgctgcggggcgcggggcgcgggcggcgctggagtctcggccgcgggcgatgaggtgcagacgctgtcgggcagcgtaaggcgggccccgaccggaccccccggcacccccggcacccccggctgcgcagctactgcaaagggccccggcgctcagcagcccaaaccggccagcttgggccgcgggcggggggcagccgccgccatcctcagcttgggcaacgtgctcaactacctggacaggtacaccgtggcaggcgtccttctggacatccagcagcactttggggtcaaggaccgaggcgccggcctgctgcagtcagtgttcatctgtagcttcatggtggctgcccccatcttcggctacctgggcgaccgcttcaacaggaaggtgattctcagctgcggcattttcttctggtcggccgtcaccttctccagctccttcattgcccagcagtacttctggctgctggtcctgtcccgggggctggtgggcatcggggaggccagctactccaccatcgcccccactatcattggcgacctcttcaccaagaacacgcgtacgctcatgctgtccgtcttctacttcgccatcccactgggcagtggcctgggctacattactggctccagcgtgaagcaggcagccggagactggcactgggcattgcgggtgtcccctgtcctgggcatgatcacaggaacactcatcctcattctggtcccagccactaaaaggggtcatgccgaccagctcggggaccagctcaaggcccggacctcatggctccgagatatgaaggccctgattcgaaaccgcagctacgtcttctcctccctggccacgtcggctgtctccttcgccacgggggccctgggcatgtggatcccgctctacctgcaccgcgcccaagttgtgcagaagacagcagagacgtgcaacagcccgccctgtggggccaaggacagcctcatctttggggccatcacctgctttacgggatttctgggcgtggtcacgggggcaggagccacgcgctggtgccgcctgaagacccagcgggccgacccactggtgtgtgccgtgggcatgctgggctctgccatcttcatctgcctgatcttcgtggctgccaagagcagcatcgtaggagcctatatctgtatcttcgtcggggagacgctgctgttttctaactgggccatcactgcagacatcctcatgtacgtggtcatccccacgcggcgcgccactgccgtggccttgcagagcttcacctcccacctgctgggggacgccgggagcccctacctcattggctttatctcagacctgatccgccagagcactaaggactccccgctctgggagttcctgagcctgggctacgcgctcatgctctgccctttcgtcgtggtcctgggcggcatgttcttcctcgccactgcgctcttcttcgtcagcgaccgcgccagggctgagcagcaggtgaaccagctggcgatgccgcccgcatctgtgaaagtctga

SEQ ID NO: 222 - DNA, 1650 bp, synthetic construct
  misc_feature 1..1650: note = Homo sapiens
  source 1..1650: mol_type = other DNA
atgatgtgcctggaatgcgcctcggcggcggcgggcggcgcggaggaggaggaggcggacgcggagcggcggcgccggcgccggggggcgcagcgaggggctggcggtagcggttgctgcggggcgcggggcgcgggcggcgctggagtctcggccgcgggcgatgaggtgcagacgctgtcgggcagcgtaaggcgggccccgaccggaccccccggcacccccggcacccccggctgcgcagctactgcaaagggccccggcgctcagcagcccaaaccggccagcttgggccgcgggcggggggcagccgccgccatcctcagcttgggcaacgtgctcaactacctggacaggtacaccgtggcaggcgtccttctggacatccagcagcactttggggtcaaggaccgaggcgccggcctgctgcagtcagtgttcatctgtagcttcatggtggctgcccccatcttcggctacctgggcgaccgcttcaacaggaaggtgattctcagctgcggcattttcttctggtcggccgtcaccttctccagctccttcattcccgcccagtacttctggctgctggtcctgtcccgggggctggtgggcatcggggaggccagctactccaccatcgcccccactatcattggcgacctcttcaccaagaacacgcgtacgctcatgctgtccgtcttctacttcgccatcccactgggcagtggcctgggctacattactggctccagcgtgaagcaggcagccggagactggcactgggcattgcgggtgtcccctgtcctgggcatgatcacaggaacactcatcctcattctggtcccagccactaaaaggggtcatgccgaccagctcggggaccagctcaaggcccggacctcatggctccgagatatgaaggccctgattcgaaaccgcagctacgtcttctcctccctggccacgtcggctgtctccttcgccacgggggccctgggcatgtggatcccgctctacctgcaccgcgcccaagttgtgcagaagacagcagagacgtgcaacagcccgccctgtggggccaaggacagcctcatctttggggccatcacctgctttacgggatttctgggcgtggtcacgggggcaggagccacgcgctggtgccgcctgaagacccagcgggccgacccactggtgtgtgccgtgggcatgctgggctctgccatcttcatctgcctgatcttcgtggctgccaagagcagcatcgtaggagcctatatctgtatcttcgtcggggagacgctgctgttttctaactgggccatcactgcagacatcctcatgtacgtggtcatccccacgcggcgcgccactgccgtggccttgcagagcttcacctcccacctgctgggggacgccgggagcccctacctcattggctttatctcagacctgatccgccagagcactaaggactccccgctctgggagttcctgagcctgggctacgcgctcatgctctgccctttcgtcgtggtcctgggcggcatgttcttcctcgccactgcgctcttcttcgtcagcgaccgcgccagggctgagcagcaggtgaaccagctggcgatgccgcccgcatctgtgaaagtctga

SEQ ID NO: 223 - DNA, 1650 bp, synthetic construct
  misc_feature 1..1650: note = Homo sapiens
  source 1..1650: mol_type = other DNA
atgatgtgcctggaatgcgcctcggcggcggcgggcggcgcggaggaggaggaggcggacgcggagcggcggcgccggcgccggggggcgcagcgaggggctggcggtagcggttgctgcggggcgcggggcgcgggcggcgctggagtctcggccgcgggcgatgaggtgcagacgctgtcgggcagcgtaaggcgggccccgaccggaccccccggcacccccggcacccccggctgcgcagctactgcaaagggccccggcgctcagcagcccaaaccggccagcttgggccgcgggcggggggcagccgccgccatcctcagcttgggcaacgtgctcaactacctggacaggtacaccgtggcaggcgtccttctggacatccagcagcactttggggtcaaggaccgaggcgccggcctgctgcagtcagtgttcatctgtagcttcatggtggctgcccccatcttcggctacctgggcgaccgcttcaacaggaaggtgattctcagctgcggcattttcttctggtcggccgtcaccttctccagctccttcattccccaggcctacttctggctgctggtcctgtcccgggggctggtgggcatcggggaggccagctactccaccatcgcccccactatcattggcgacctcttcaccaagaacacgcgtacgctcatgctgtccgtcttctacttcgccatcccactgggcagtggcctgggctacattactggctccagcgtgaagcaggcagccggagactggcactgggcattgcgggtgtcccctgtcctgggcatgatcacaggaacactcatcctcattctggtcccagccactaaaaggggtcatgccgaccagctcggggaccagctcaaggcccggacctcatggctccgagatatgaaggccctgattcgaaaccgcagctacgtcttctcctccctggccacgtcggctgtctccttcgccacgggggccctgggcatgtggatcccgctctacctgcaccgcgcccaagttgtgcagaagacagcagagacgtgcaacagcccgccctgtggggccaaggacagcctcatctttggggccatcacctgctttacgggatttctgggcgtggtcacgggggcaggagccacgcgctggtgccgcctgaagacccagcgggccgacccactggtgtgtgccgtgggcatgctgggctctgccatcttcatctgcctgatcttcgtggctgccaagagcagcatcgtaggagcctatatctgtatcttcgtcggggagacgctgctgttttctaactgggccatcactgcagacatcctcatgtacgtggtcatccccacgcggcgcgccactgccgtggccttgcagagcttcacctcccacctgctgggggacgccgggagcccctacctcattggctttatctcagacctgatccgccagagcactaaggactccccgctctgggagttcctgagcctgggctacgcgctcatgctctgccctttcgtcgtggtcctgggcggcatgttcttcctcgccactgcgctcttcttcgtcagcgaccgcgccagggctgagcagcaggtgaaccagctggcgatgccgcccgcatctgtgaaagtctga

SEQ ID NO: 224 - DNA, 1650 bp, synthetic construct
  misc_feature 1..1650: note = Homo sapiens
  source 1..1650: mol_type = other DNA
atgatgtgcctggaatgcgcctcggcggcggcgggcggcgcggaggaggaggaggcggacgcggagcggcggcgccggcgccggggggcgcagcgaggggctggcggtagcggttgctgcggggcgcggggcgcgggcggcgctggagtctcggccgcgggcgatgaggtgcagacgctgtcgggcagcgtaaggcgggccccgaccggaccccccggcacccccggcacccccggctgcgcagctactgcaaagggccccggcgctcagcagcccaaaccggccagcttgggccgcgggcggggggcagccgccgccatcctcagcttgggcaacgtgctcaactacctggacaggtacaccgtggcaggcgtccttctggacatccagcagcactttggggtcaaggaccgaggcgccggcctgctgcagtcagtgttcatctgtagcttcatggtggctgcccccatcttcggctacctgggcgaccgcttcaacaggaaggtgattctcagctgcggcattttcttctggtcggccgtcaccttctccagctccttcattccccagcaggccttctggctgctggtcctgtcccgggggctggtgggcatcggggaggccagctactccaccatcgcccccactatcattggcgacctcttcaccaagaacacgcgtacgctcatgctgtccgtcttctacttcgccatcccactgggcagtggcctgggctacattactggctccagcgtgaagcaggcagccggagactggcactgggcattgcgggtgtcccctgtcctgggcatgatcacaggaacactcatcctcattctggtcccagccactaaaaggggtcatgccgaccagctcggggaccagctcaaggcccggacctcatggctccgagatatgaaggccctgattcgaaaccgcagctacgtcttctcctccctggccacgtcggctgtctccttcgccacgggggccctgggcatgtggatcccgctctacctgcaccgcgcccaagttgtgcagaagacagcagagacgtgcaacagcccgccctgtggggccaaggacagcctcatctttggggccatcacctgctttacgggatttctgggcgtggtcacgggggcaggagccacgcgctggtgccgcctgaagacccagcgggccgacccactggtgtgtgccgtgggcatgctgggctctgccatcttcatctgcctgatcttcgtggctgccaagagcagcatcgtaggagcctatatctgtatcttcgtcggggagacgctgctgttttctaactgggccatcactgcagacatcctcatgtacgtggtcatccccacgcggcgcgccactgccgtggccttgcagagcttcacctcccacctgctgggggacgccgggagcccctacctcattggctttatctcagacctgatccgccagagcactaaggactccccgctctgggagttcctgagcctgggctacgcgctcatgctctgccctttcgtcgtggtcctgggcggcatgttcttcctcgccactgcgctcttcttcgtcagcgaccgcgccagggctgagcagcaggtgaaccagctggcgatgccgcccgcatctgtgaaagtctga

SEQ ID NO: 225 - DNA, 1650 bp, synthetic construct
  misc_feature 1..1650: note = Homo sapiens
  source 1..1650: mol_type = other DNA
atgatgtgcctggaatgcgcctcggcggcggcgggcggcgcggaggaggaggaggcggacgcggagcggcggcgccggcgccggggggcgcagcgaggggctggcggtagcggttgctgcggggcgcggggcgcgggcggcgctggagtctcggccgcgggcgatgaggtgcagacgctgtcgggcagcgtaaggcgggccccgaccggaccccccggcacccccggcacccccggctgcgcagctactgcaaagggccccggcgctcagcagcccaaaccggccagcttgggccgcgggcggggggcagccgccgccatcctcagcttgggcaacgtgctcaactacctggacaggtacaccgtggcaggcgtccttctggacatccagcagcactttggggtcaaggaccgaggcgccggcctgctgcagtcagtgttcatctgtagcttcatggtggctgcccccatcttcggctacctgggcgaccgcttcaacaggaaggtgattctcagctgcggcattttcttctggtcggccgtcaccttctccagctccttcattccccagcagtacgcctggctgctggtcctgtcccgggggctggtgggcatcggggaggccagctactccaccatcgcccccactatcattggcgacctcttcaccaagaacacgcgtacgctcatgctgtccgtcttctacttcgccatcccactgggcagtggcctgggctacattactggctccagcgtgaagcaggcagccggagactggcactgggcattgcgggtgtcccctgtcctgggcatgatcacaggaacactcatcctcattctggtcccagccactaaaaggggtcatgccgaccagctcggggaccagctcaaggcccggacctcatggctccgagatatgaaggccctgattcgaaaccgcagctacgtcttctcctccctggccacgtcggctgtctccttcgccacgggggccctgggcatgtggatcccgctctacctgcaccgcgcccaagttgtgcagaagacagcagagacgtgcaacagcccgccctgtggggccaaggacagcctcatctttggggccatcacctgctttacgggatttctgggcgtggtcacgggggcaggagccacgcgctggtgccgcctgaagacccagcgggccgacccactggtgtgtgccgtgggcatgctgggctctgccatcttcatctgcctgatcttcgtggctgccaagagcagcatcgtaggagcctatatctgtatcttcgtcggggagacgctgctgttttctaactgggccatcactgcagacatcctcatgtacgtggtcatccccacgcggcgcgccactgccgtggccttgcagagcttcacctcccacctgctgggggacgccgggagcccctacctcattggctttatctcagacctgatccgccagagcactaaggactccccgctctgggagttcctgagcctgggctacgcgctcatgctctgccctttcgtcgtggtcctgggcggcatgttcttcctcgccactgcgctcttcttcgtcagcgaccgcgccagggctgagcagcaggtgaaccagctggcgatgccgcccgcatctgtgaaagtctga

SEQ ID NO: 226 - DNA, 1650 bp, synthetic construct
  misc_feature 1..1650: note = Homo sapiens
  source 1..1650: mol_type = other DNA
atgatgtgcctggaatgcgcctcggcggcggcgggcggcgcggaggaggaggaggcggacgcggagcggcggcgccggcgccggggggcgcagcgaggggctggcggtagcggttgctgcggggcgcggggcgcgggcggcgctggagtctcggccgcgggcgatgaggtgcagacgctgtcgggcagcgtaaggcgggccccgaccggaccccccggcacccccggcacccccggctgcgcagctactgcaaagggccccggcgctcagcagcccaaaccggccagcttgggccgcgggcggggggcagccgccgccatcctcagcttgggcaacgtgctcaactacctggacaggtacaccgtggcaggcgtccttctggacatccagcagcactttggggtcaaggaccgaggcgccggcctgctgcagtcagtgttcatctgtagcttcatggtggctgcccccatcttcggctacctgggcgaccgcttcaacaggaaggtgattctcagctgcggcattttcttctggtcggccgtcaccttctccagctccttcattccccagcagtacttcgccctgctggtcctgtcccgggggctggtgggcatcggggaggccagctactccaccatcgcccccactatcattggcgacctcttcaccaagaacacgcgtacgctcatgctgtccgtcttctacttcgccatcccactgggcagtggcctgggctacattactggctccagcgtgaagcaggcagccggagactggcactgggcattgcgggtgtcccctgtcctgggcatgatcacaggaacactcatcctcattctggtcccagccactaaaaggggtcatgccgaccagctcggggaccagctcaaggcccggacctcatggctccgagatatgaaggccctgattcgaaaccgcagctacgtcttctcctccctggccacgtcggctgtctccttcgccacgggggccctgggcatgtggatcccgctctacctgcaccgcgcccaagttgtgcagaagacagcagagacgtgcaacagcccgccctgtggggccaaggacagcctcatctttggggccatcacctgctttacgggatttctgggcgtggtcacgggggcaggagccacgcgctggtgccgcctgaagacccagcgggccgacccactggtgtgtgccgtgggcatgctgggctctgccatcttcatctgcctgatcttcgtggctgccaagagcagcatcgtaggagcctatatctgtatcttcgtcggggagacgctgctgttttctaactgggccatcactgcagacatcctcatgtacgtggtcatccccacgcggcgcgccactgccgtggccttgcagagcttcacctcccacctgctgggggacgccgggagcccctacctcattggctttatctcagacctgatccgccagagcactaaggactccccgctctgggagttcctgagcctgggctacgcgctcatgctctgccctttcgtcgtggtcctgggcggcatgttcttcctcgccactgcgctcttcttcgtcagcgaccgcgccagggctgagcagcaggtgaaccagctggcgatgccgcccgcatctgtgaaagtctga

SEQ ID NO: 227 - DNA, 1650 bp, synthetic construct
  misc_feature 1..1650: note = Homo sapiens
  source 1..1650: mol_type = other DNA
atgatgtgcctggaatgcgcctcggcggcggcgggcggcgcggaggaggaggaggcggacgcggagcggcggcgccggcgccggggggcgcagcgaggggctggcggtagcggttgctgcggggcgcggggcgcgggcggcgctggagtctcggccgcgggcgatgaggtgcagacgctgtcgggcagcgtaaggcgggccccgaccggaccccccggcacccccggcacccccggctgcgcagctactgcaaagggccccggcgctcagcagcccaaaccggccagcttgggccgcgggcggggggcagccgccgccatcctcagcttgggcaacgtgctcaactacctggacaggtacaccgtggcaggcgtccttctggacatccagcagcactttggggtcaaggaccgaggcgccggcctgctgcagtcagtgttcatctgtagcttcatggtggctgcccccatcttcggctacctgggcgaccgcttcaacaggaaggtgattctcagctgcggcattttcttctggtcggccgtcaccttctccagctccttcattccccagcagtacttctgggccctggtcctgtcccgggggctggtgggcatcggggaggccagctactccaccatcgcccccactatcattggcgacctcttcaccaagaacacgcgtacgctcatgctgtccgtcttctacttcgccatcccactgggcagtggcctgggctacattactggctccagcgtgaagcaggcagccggagactggcactgggcattgcgggtgtcccctgtcctgggcatgatcacaggaacactcatcctcattctggtcccagccactaaaaggggtcatgccgaccagctcggggaccagctcaaggcccggacctcatggctccgagatatgaaggccctgattcgaaaccgcagctacgtcttctcctccctggccacgtcggctgtctccttcgccacgggggccctgggcatgtggatcccgctctacctgcaccgcgcccaagttgtgcagaagacagcagagacgtgcaacagcccgccctgtggggccaaggacagcctcatctttggggccatcacctgctttacgggatttctgggcgtggtcacgggggcaggagccacgcgctggtgccgcctgaagacccagcgggccgacccactggtgtgtgccgtgggcatgctgggctctgccatcttcatctgcctgatcttcgtggctgccaagagcagcatcgtaggagcctatatctgtatcttcgtcggggagacgctgctgttttctaactgggccatcactgcagacatcctcatgtacgtggtcatccccacgcggcgcgccactgccgtggccttgcagagcttcacctcccacctgctgggggacgccgggagcccctacctcattggctttatctcagacctgatccgccagagcactaaggactccccgctctgggagttcctgagcctgggctacgcgctcatgctctgccctttcgtcgtggtcctgggcggcatgttcttcctcgccactgcgctcttcttcgtcagcgaccgcgccagggctgagcagcaggtgaaccagctggcgatgccgcccgcatctgtgaaagtctga

SEQ ID NO: 228 - DNA, 1650 bp, synthetic construct
  misc_feature 1..1650: note = Homo sapiens
  source 1..1650: mol_type = other DNA
atgatgtgcctggaatgcgcctcggcggcggcgggcggcgcggaggaggaggaggcggacgcggagcggcggcgccggcgccggggggcgcagcgaggggctggcggtagcggttgctgcggggcgcggggcgcgggcggcgctggagtctcggccgcgggcgatgaggtgcagacgctgtcgggcagcgtaaggcgggccccgaccggaccccccggcacccccggcacccccggctgcgcagctactgcaaagggccccggcgctcagcagcccaaaccggccagcttgggccgcgggcggggggcagccgccgccatcctcagcttgggcaacgtgctcaactacctggacaggtacaccgtggcaggcgtccttctggacatccagcagcactttggggtcaaggaccgaggcgccggcctgctgcagtcagtgttcatctgtagcttcatggtggctgcccccatcttcggctacctgggcgaccgcttcaacaggaaggtgattctcagctgcggcattttcttctggtcggccgtcaccttctccagctccttcattccccagcagtacttctggctggccgtcctgtcccgggggctggtgggcatcggggaggccagctactccaccatcgcccccactatcattggcgacctcttcaccaagaacacgcgtacgctcatgctgtccgtcttctacttcgccatcccactgggcagtggcctgggctacattactggctccagcgtgaagcaggcagccggagactggcactgggcattgcgggtgtcccctgtcctgggcatgatcacaggaacactcatcctcattctggtcccagccactaaaaggggtcatgccgaccagctcggggaccagctcaaggcccggacctcatggctccgagatatgaaggccctgattcgaaaccgcagctacgtcttctcctccctggccacgtcggctgtctccttcgccacgggggccctgggcatgtggatcccgctctacctgcaccgcgcccaagttgtgcagaagacagcagagacgtgcaacagcccgccctgtggggccaaggacagcctcatctttggggccatcacctgctttacgggatttctgggcgtggtcacgggggcaggagccacgcgctggtgccgcctgaagacccagcgggccgacccactggtgtgtgccgtgggcatgctgggctctgccatcttcatctgcctgatcttcgtggctgccaagagcagcatcgtaggagcctatatctgtatcttcgtcggggagacgctgctgttttctaactgggccatcactgcagacatcctcatgtacgtggtcatccccacgcggcgcgccactgccgtggccttgcagagcttcacctcccacctgctgggggacgccgggagcccctacctcattggctttatctcagacctgatccgccagagcactaaggactccccgctctgggagttcctgagcctgggctacgcgctcatgctctgccctttcgtcgtggtcctgggcggcatgttcttcctcgccactgcgctcttcttcgtcagcgaccgcgccagggctgagcagcaggtgaaccagctggcgatgccgcccgcatctgtgaaagtctga

SEQ ID NO: 229 - DNA, 1650 bp, synthetic construct
  misc_feature 1..1650: note = Homo sapiens
  source 1..1650: mol_type = other DNA
atgatgtgcctggaatgcgcctcggcggcggcgggcggcgcggaggaggaggaggcggacgcggagcggcggcgccggcgccggggggcgcagcgaggggctggcggtagcggttgctgcggggcgcggggcgcgggcggcgctggagtctcggccgcgggcgatgaggtgcagacgctgtcgggcagcgtaaggcgggccccgaccggaccccccggcacccccggcacccccggctgcgcagctactgcaaagggccccggcgctcagcagcccaaaccggccagcttgggccgcgggcggggggcagccgccgccatcctcagcttgggcaacgtgctcaactacctggacaggtacaccgtggcaggcgtccttctggacatccagcagcactttggggtcaaggaccgaggcgccggcctgctgcagtcagtgttcatctgtagcttcatggtggctgcccccatcttcggctacctgggcgaccgcttcaacaggaaggtgattctcagctgcggcattttcttctggtcggccgtcaccttctccagctccttcattccccagcagtacttctggctgctggccctgtcccgggggctggtgggcatcggggaggccagctactccaccatcgcccccactatcattggcgacctcttcaccaagaacacgcgtacgctcatgctgtccgtcttctacttcgccatcccactgggcagtggcctgggctacattactggctccagcgtgaagcaggcagccggagactggcactgggcattgcgggtgtcccctgtcctgggcatgatcacaggaacactcatcctcattctggtcccagccactaaaaggggtcatgccgaccagctcggggaccagctcaaggcccggacctcatggctccgagatatgaaggccctgattcgaaaccgcagctacgtcttctcctccctggccacgtcggctgtctccttcgccacgggggccctgggcatgtggatcccgctctacctgcaccgcgcccaagttgtgcagaagacagcagagacgtgcaacagcccgccctgtggggccaaggacagcctcatctttggggccatcacctgctttacgggatttctgggcgtggtcacgggggcaggagccacgcgctggtgccgcctgaagacccagcgggccgacccactggtgtgtgccgtgggcatgctgggctctgccatcttcatctgcctgatcttcgtggctgccaagagcagcatcgtaggagcctatatctgtatcttcgtcggggagacgctgctgttttctaactgggccatcactgcagacatcctcatgtacgtggtcatccccacgcggcgcgccactgccgtggccttgcagagcttcacctcccacctgctgggggacgccgggagcccctacctcattggctttatctcagacctgatccgccagagcactaaggactccccgctctgggagttcctgagcctgggctacgcgctcatgctctgccctttcgtcgtggtcctgggcggcatgttcttcctcgccactgcgctcttcttcgtcagcgaccgcgccagggctgagcagcaggtgaaccagctggcgatgccgcccgcatctgtgaaagtctga

SEQ ID NO: 230 - DNA, 1650 bp, synthetic construct
  misc_feature 1..1650: note = Homo sapiens
  source 1..1650: mol_type = other DNA
atgatgtgcctggaatgcgcctcggcggcggcgggcggcgcggaggaggaggaggcggacgcggagcggcggcgccggcgccggggggcgcagcgaggggctggcggtagcggttgctgcggggcgcggggcgcgggcggcgctggagtctcggccgcgggcgatgaggtgcagacgctgtcgggcagcgtaaggcgggccccgaccggaccccccggcacccccggcacccccggctgcgcagctactgcaaagggccccggcgctcagcagcccaaaccggccagcttgggccgcgggcggggggcagccgccgccatcctcagcttgggcaacgtgctcaactacctggacaggtacaccgtggcaggcgtccttctggacatccagcagcactttggggtcaaggaccgaggcgccggcctgctgcagtcagtgttcatctgtagcttcatggtggctgcccccatcttcggctacctgggcgaccgcttcaacaggaaggtgattctcagctgcggcattttcttctggtcggccgtcaccttctccagctccttcattccccagcagtacttctggctgctggtcgcctcccgggggctggtgggcatcggggaggccagctactccaccatcgcccccactatcattggcgacctcttcaccaagaacacgcgtacgctcatgctgtccgtcttctacttcgccatcccactgggcagtggcctgggctacattactggctccagcgtgaagcaggcagccggagactggcactgggcattgcgggtgtcccctgtcctgggcatgatcacaggaacactcatcctcattctggtcccagccactaaaaggggtcatgccgaccagctcggggaccagctcaaggcccggacctcatggctccgagatatgaaggccctgattcgaaaccgcagctacgtcttctcctccctggccacgtcggctgtctccttcgccacgggggccctgggcatgtggatcccgctctacctgcaccgcgcccaagttgtgcagaagacagcagagacgtgcaacagcccgccctgtggggccaaggacagcctcatctttggggccatcacctgctttacgggatttctgggcgtggtcacgggggcaggagccacgcgctggtgccgcctgaagacccagcgggccgacccactggtgtgtgccgtgggcatgctgggctctgccatcttcatctgcctgatcttcgtggctgccaagagcagcatcgtaggagcctatatctgtatcttcgtcggggagacgctgctgttttctaactgggccatcactgcagacatcctcatgtacgtggtcatccccacgcggcgcgccactgccgtggccttgcagagcttcacctcccacctgctgggggacgccgggagcccctacctcattggctttatctcagacctgatccgccagagcactaaggactccccgctctgggagttcctgagcctgggctacgcgctcatgctctgccctttcgtcgtggtcctgggcggcatgttcttcctcgccactgcgctcttcttcgtcagcgaccgcgccagggctgagcagcaggtgaaccagctggcgatgccgcccgcatctgtgaaagtctga

SEQ ID NO: 231 - DNA, 1650 bp, synthetic construct
  misc_feature 1..1650: note = Homo sapiens
  source 1..1650: mol_type = other DNA
atgatgtgcctggaatgcgcctcggcggcggcgggcggcgcggaggaggaggaggcggacgcggagcggcggcgccggcgccggggggcgcagcgaggggctggcggtagcggttgctgcggggcgcggggcgcgggcggcgctggagtctcggccgcgggcgatgaggtgcagacgctgtcgggcagcgtaaggcgggccccgaccggaccccccggcacccccggcacccccggctgcgcagctactgcaaagggccccggcgctcagcagcccaaaccggccagcttgggccgcgggcggggggcagccgccgccatcctcagcttgggcaacgtgctcaactacctggacaggtacaccgtggcaggcgtccttctggacatccagcagcactttggggtcaaggaccgaggcgccggcctgctgcagtcagtgttcatctgtagcttcatggtggctgcccccatcttcggctacctgggcgaccgcttcaacaggaaggtgattctcagctgcggcattttcttctggtcggccgtcaccttctccagctccttcattccccagcagtacttctggctgctggtcctggcccgggggctggtgggcatcggggaggccagctactccaccatcgcccccactatcattggcgacctcttcaccaagaacacgcgtacgctcatgctgtccgtcttctacttcgccatcccactgggcagtggcctgggctacattactggctccagcgtgaagcaggcagccggagactggcactgggcattgcgggtgtcccctgtcctgggcatgatcacaggaacactcatcctcattctggtcccagccactaaaaggggtcatgccgaccagctcggggaccagctcaaggcccggacctcatggctccgagatatgaaggccctgattcgaaaccgcagctacgtcttctcctccctggccacgtcggctgtctccttcgccacgggggccctgggcatgtggatcccgctctacctgcaccgcgcccaagttgtgcagaagacagcagagacgtgcaacagcccgccctgtggggccaaggacagcctcatctttggggccatcacctgctttacgggatttctgggcgtggtcacgggggcaggagccacgcgctggtgccgcctgaagacccagcgggccgacccactggtgtgtgccgtgggcatgctgggctctgccatcttcatctgcctgatcttcgtggctgccaagagcagcatcgtaggagcctatatctgtatcttcgtcggggagacgctgctgttttctaactgggccatcactgcagacatcctcatgtacgtggtcatccccacgcggcgcgccactgccgtggccttgcagagcttcacctcccacctgctgggggacgccgggagcccctacctcattggctttatctcagacctgatccgccagagcactaaggactccccgctctgggagttcctgagcctgggctacgcgctcatgctctgccctttcgtcgtggtcctgggcggcatgttcttcctcgccactgcgctcttcttcgtcagcgaccgcgccagggctgagcagcaggtgaaccagctggcgatgccgcccgcatctgtgaaagtctga

SEQ ID NO: 232 - DNA, 1650 bp, synthetic construct
  misc_feature 1..1650: note = Homo sapiens
  source 1..1650: mol_type = other DNA
atgatgtgcctggaatgcgcctcggcggcggcgggcggcgcggaggaggaggaggcggacgcggagcggcggcgccggcgccggggggcgcagcgaggggctggcggtagcggttgctgcggggcgcggggcgcgggcggcgctggagtctcggccgcgggcgatgaggtgcagacgctgtcgggcagcgtaaggcgggccccgaccggaccccccggcacccccggcacccccggctgcgcagctactgcaaagggccccggcgctcagcagcccaaaccggccagcttgggccgcgggcggggggcagccgccgccatcctcagcttgggcaacgtgctcaactacctggacaggtacaccgtggcaggcgtccttctggacatccagcagcactttggggtcaaggaccgaggcgccggcctgctgcagtcagtgttcatctgtagcttcatggtggctgcccccatcttcggctacctgggcgaccgcttcaacaggaaggtgattctcagctgcggcattttcttctggtcggccgtcaccttctccagctccttcattccccagcagtacttctggctgctggtcctgtccgccgggctggtgggcatcggggaggccagctactccaccatcgcccccactatcattggcgacctcttcaccaagaacacgcgtacgctcatgctgtccgtcttctacttcgccatcccactgggcagtggcctgggctacattactggctccagcgtgaagcaggcagccggagactggcactgggcattgcgggtgtcccctgtcctgggcatgatcacaggaacactcatcctcattctggtcccagccactaaaaggggtcatgccgaccagctcggggaccagctcaaggcccggacctcatggctccgagatatgaaggccctgattcgaaaccgcagctacgtcttctcctccctggccacgtcggctgtctccttcgccacgggggccctgggcatgtggatcccgctctacctgcaccgcgcccaagttgtgcagaagacagcagagacgtgcaacagcccgccctgtggggccaaggacagcctcatctttggggccatcacctgctttacgggatttctgggcgtggtcacgggggcaggagccacgcgctggtgccgcctgaagacccagcgggccgacccactggtgtgtgccgtgggcatgctgggctctgccatcttcatctgcctgatcttcgtggctgccaagagcagcatcgtaggagcctatatctgtatcttcgtcggggagacgctgctgttttctaactgggccatcactgcagacatcctcatgtacgtggtcatccccacgcggcgcgccactgccgtggccttgcagagcttcacctcccacctgctgggggacgccgggagcccctacctcattggctttatctcagacctgatccgccagagcactaaggactccccgctctgggagttcctgagcctgggctacgcgctcatgctctgccctttcgtcgtggtcctgggcggcatgttcttcctcgccactgcgctcttcttcgtcagcgaccgcgccagggctgagcagcaggtgaaccagctggcgatgccgcccgcatctgtgaaagtctga

SEQ ID NO: 233 - DNA, 1650 bp, synthetic construct
  misc_feature 1..1650: note = Homo sapiens
  source 1..1650: mol_type = other DNA
atgatgtgcctggaatgcgcctcggcggcggcgggcggcgcggaggaggaggaggcggacgcggagcggcggcgccggcgccggggggcgcagcgaggggctggcggtagcggttgctgcggggcgcggggcgcgggcggcgctggagtctcggccgcgggcgatgaggtgcagacgctgtcgggcagcgtaaggcgggccccgaccggaccccccggcacccccggcacccccggctgcgcagctactgcaaagggccccggcgctcagcagcccaaaccggccagcttgggccgcgggcggggggcagccgccgccatcctcagcttgggcaacgtgctcaactacctggacaggtacaccgtggcaggcgtccttctggacatccagcagcactttggggtcaaggaccgaggcgccggcctgctgcagtcagtgttcatctgtagcttcatggtggctgcccccatcttcggctacctgggcgaccgcttcaacaggaaggtgattctcagctgcggcattttcttctggtcggccgtcaccttctccagctccttcattccccagcagtacttctggctgctggtcctgtcccgggccctggtgggcatcggggaggccagctactccaccatcgcccccactatcattggcgacctcttcaccaagaacacgcgtacgctcatgctgtccgtcttctacttcgccatcccactgggcagtggcctgggctacattactggctccagcgtgaagcaggcagccggagactggcactgggcattgcgggtgtcccctgtcctgggcatgatcacaggaacactcatcctcattctggtcccagccactaaaaggggtcatgccgaccagctcggggaccagctcaaggcccggacctcatggctccgagatatgaaggccctgattcgaaaccgcagctacgtcttctcctccctggccacgtcggctgtctccttcgccacgggggccctgggcatgtggatcccgctctacctgcaccgcgcccaagttgtgcagaagacagcagagacgtgcaacagcccgccctgtggggccaaggacagcctcatctttggggccatcacctgctttacgggatttctgggcgtggtcacgggggcaggagccacgcgctggtgccgcctgaagacccagcgggccgacccactggtgtgtgccgtgggcatgctgggctctgccatcttcatctgcctgatcttcgtggctgccaagagcagcatcgtaggagcctatatctgtatcttcgtcggggagacgctgctgttttctaactgggccatcactgcagacatcctcatgtacgtggtcatccccacgcggcgcgccactgccgtggccttgcagagcttcacctcccacctgctgggggacgccgggagcccctacctcattggctttatctcagacctgatccgccagagcactaaggactccccgctctgggagttcctgagcctgggctacgcgctcatgctctgccctttcgtcgtggtcctgggcggcatgttcttcctcgccactgcgctcttcttcgtcagcgaccgcgccagggctgagcagcaggtgaaccagctggcgatgccgcccgcatctgtgaaagtctga

SEQ ID NO: 234 - DNA, 1650 bp, synthetic construct
  misc_feature 1..1650: note = Homo sapiens
  source 1..1650: mol_type = other DNA
atgatgtgcctggaatgcgcctcggcggcggcgggcggcgcggaggaggaggaggcggacgcggagcggcggcgccggcgccggggggcgcagcgaggggctggcggtagcggttgctgcggggcgcggggcgcgggcggcgctggagtctcggccgcgggcgatgaggtgcagacgctgtcgggcagcgtaaggcgggccccgaccggaccccccggcacccccggcacccccggctgcgcagctactgcaaagggccccggcgctcagcagcccaaaccggccagcttgggccgcgggcggggggcagccgccgccatcctcagcttgggcaacgtgctcaactacctggacaggtacaccgtggcaggcgtccttctggacatccagcagcactttggggtcaaggaccgaggcgccggcctgctgcagtcagtgttcatctgtagcttcatggtggctgcccccatcttcggctacctgggcgaccgcttcaacaggaaggtgattctcagctgcggcattttcttctggtcggccgtcaccttctccagctccttcattccccagcagtacttctggctgctggtcctgtcccggggggccgtgggcatcggggaggccagctactccaccatcgcccccactatcattggcgacctcttcaccaagaacacgcgtacgctcatgctgtccgtcttctacttcgccatcccactgggcagtggcctgggctacattactggctccagcgtgaagcaggcagccggagactggcactgggcattgcgggtgtcccctgtcctgggcatgatcacaggaacactcatcctcattctggtcccagccactaaaaggggtcatgccgaccagctcggggaccagctcaaggcccggacctcatggctccgagatatgaaggccctgattcgaaaccgcagctacgtcttctcctccctggccacgtcggctgtctccttcgccacgggggccctgggcatgtggatcccgctctacctgcaccgcgcccaagttgtgcagaagacagcagagacgtgcaacagcccgccctgtggggccaaggacagcctcatctttggggccatcacctgctttacgggatttctgggcgtggtcacgggggcaggagccacgcgctggtgccgcctgaagacccagcgggccgacccactggtgtgtgccgtgggcatgctgggctctgccatcttcatctgcctgatcttcgtggctgccaagagcagcatcgtaggagcctatatctgtatcttcgtcggggagacgctgctgttttctaactgggccatcactgcagacatcctcatgtacgtggtcatccccacgcggcgcgccactgccgtggccttgcagagcttcacctcccacctgctgggggacgccgggagcccctacctcattggctttatctcagacctgatccgccagagcactaaggactccccgctctgggagttcctgagcctgggctacgcgctcatgctctgccctttcgtcgtggtcctgggcggcatgttcttcctcgccactgcgctcttcttcgtcagcgaccgcgccagggctgagcagcaggtgaaccagctggcgatgccgcccgcatctgtgaaagtctga

SEQ ID NO: 235 - DNA, 1650 bp, synthetic construct
  misc_feature 1..1650: note = Homo sapiens
  source 1..1650: mol_type = other DNA
atgatgtgcctggaatgcgcctcggcggcggcgggcggcgcggaggaggaggaggcggacgcggagcggcggcgccggcgccggggggcgcagcgaggggctggcggtagcggttgctgcggggcgcggggcgcgggcggcgctggagtctcggccgcgggcgatgaggtgcagacgctgtcgggcagcgtaaggcgggccccgaccggaccccccggcacccccggcacccccggctgcgcagctactgcaaagggccccggcgctcagcagcccaaaccggccagcttgggccgcgggcggggggcagccgccgccatcctcagcttgggcaacgtgctcaactacctggacaggtacaccgtggcaggcgtccttctggacatccagcagcactttggggtcaaggaccgaggcgccggcctgctgcagtcagtgttcatctgtagcttcatggtggctgcccccatcttcggctacctgggcgaccgcttcaacaggaaggtgattctcagctgcggcattttcttctggtcggccgtcaccttctccagctccttcattccccagcagtacttctggctgctggtcctgtcccgggggctggtgggcatcggggaggccagctactccaccatcgcccccactatcattggcgacctcttcaccaagaacacgcgtacgctcatgctgtccgtcttctacttcgccatcccactgggcagtggcctgggctacattactggctccagcgccaagcaggcagccggagactggcactgggcattgcgggtgtcccctgtcctgggcatgatcacaggaacactcatcctcattctggtcccagccactaaaaggggtcatgccgaccagctcggggaccagctcaaggcccggacctcatggctccgagatatgaaggccctgattcgaaaccgcagctacgtcttctcctccctggccacgtcggctgtctccttcgccacgggggccctgggcatgtggatcccgctctacctgcaccgcgcccaagttgtgcagaagacagcagagacgtgcaacagcccgccctgtggggccaaggacagcctcatctttggggccatcacctgctttacgggatttctgggcgtggtcacgggggcaggagccacgcgctggtgccgcctgaagacccagcgggccgacccactggtgtgtgccgtgggcatgctgggctctgccatcttcatctgcctgatcttcgtggctgccaagagcagcatcgtaggagcctatatctgtatcttcgtcggggagacgctgctgttttctaactgggccatcactgcagacatcctcatgtacgtggtcatccccacgcggcgcgccactgccgtggccttgcagagcttcacctcccacctgctgggggacgccgggagcccctacctcattggctttatctcagacctgatccgccagagcactaaggactccccgctctgggagttcctgagcctgggctacgcgctcatgctctgccctttcgtcgtggtcctgggcggcatgttcttcctcgccactgcgctcttcttcgtcagcgaccgcgccagggctgagcagcaggtgaaccagctggcgatgccgcccgcatctgtgaaagtctga

SEQ ID NO: 236 - DNA, 1650 bp, synthetic construct
  misc_feature 1..1650: note = Homo sapiens
  source 1..1650: mol_type = other DNA
atgatgtgcctggaatgcgcctcggcggcggcgggcggcgcggaggaggaggaggcggacgcggagcggcggcgccggcgccggggggcgcagcgaggggctggcggtagcggttgctgcggggcgcggggcgcgggcggcgctggagtctcggccgcgggcgatgaggtgcagacgctgtcgggcagcgtaaggcgggccccgaccggaccccccggcacccccggcacccccggctgcgcagctactgcaaagggccccggcgctcagcagcccaaaccggccagcttgggccgcgggcggggggcagccgccgccatcctcagcttgggcaacgtgctcaactacctggacaggtacaccgtggcaggcgtccttctggacatccagcagcactttggggtcaaggaccgaggcgccggcctgctgcagtcagtgttcatctgtagcttcatggtggctgcccccatcttcggctacctgggcgaccgcttcaacaggaaggtgattctcagctgcggcattttcttctggtcggccgtcaccttctccagctccttcattccccagcagtacttctggctgctggtcctgtcccgggggctggtgggcatcggggaggccagctactccaccatcgcccccactatcattggcgacctcttcaccaagaacacgcgtacgctcatgctgtccgtcttctacttcgccatcccactgggcagtggcctgggctacattactggctccagcgtggcccaggcagccggagactggcactgggcattgcgggtgtcccctgtcctgggcatgatcacaggaacactcatcctcattctggtcccagccactaaaaggggtcatgccgaccagctcggggaccagctcaaggcccggacctcatggctccgagatatgaaggccctgattcgaaaccgcagctacgtcttctcctccctggccacgtcggctgtctccttcgccacgggggccctgggcatgtggatcccgctctacctgcaccgcgcccaagttgtgcagaagacagcagagacgtgcaacagcccgccctgtggggccaaggacagcctcatctttggggccatcacctgctttacgggatttctgggcgtggtcacgggggcaggagccacgcgctggtgccgcctgaagacccagcgggccgacccactggtgtgtgccgtgggcatgctgggctctgccatcttcatctgcctgatcttcgtggctgccaagagcagcatcgtaggagcctatatctgtatcttcgtcggggagacgctgctgttttctaactgggccatcactgcagacatcctcatgtacgtggtcatccccacgcggcgcgccactgccgtggccttgcagagcttcacctcccacctgctgggggacgccgggagcccctacctcattggctttatctcagacctgatccgccagagcactaaggactccccgctctgggagttcctgagcctgggctacgcgctcatgctctgccctttcgtcgtggtcctgggcggcatgttcttcctcgccactgcgctcttcttcgtcagcgaccgcgccagggctgagcagcaggtgaaccagctggcgatgccgcccgcatctgtgaaagtctga

SEQ ID NO: 237 - DNA, 1650 bp, synthetic construct
  misc_feature 1..1650: note = Homo sapiens
  source 1..1650: mol_type = other DNA
atgatgtgcctggaatgcgcctcggcggcggcgggcggcgcggaggaggaggaggcggacgcggagcggcggcgccggcgccggggggcgcagcgaggggctggcggtagcggttgctgcggggcgcggggcgcgggcggcgctggagtctcggccgcgggcgatgaggtgcagacgctgtcgggcagcgtaaggcgggccccgaccggaccccccggcacccccggcacccccggctgcgcagctactgcaaagggccccggcgctcagcagcccaaaccggccagcttgggccgcgggcggggggcagccgccgccatcctcagcttgggcaacgtgctcaactacctggacaggtacaccgtggcaggcgtccttctggacatccagcagcactttggggtcaaggaccgaggcgccggcctgctgcagtcagtgttcatctgtagcttcatggtggctgcccccatcttcggctacctgggcgaccgcttcaacaggaaggtgattctcagctgcggcattttcttctggtcggccgtcaccttctccagctccttcattccccagcagtacttctggctgctggtcctgtcccgggggctggtgggcatcggggaggccagctactccaccatcgcccccactatcattggcgacctcttcaccaagaacacgcgtacgctcatgctgtccgtcttctacttcgccatcccactgggcagtggcctgggctacattactggctccagcgtgaaggccgcagccggagactggcactgggcattgcgggtgtcccctgtcctgggcatgatcacaggaacactcatcctcattctggtcccagccactaaaaggggtcatgccgaccagctcggggaccagctcaaggcccggacctcatggctccgagatatgaaggccctgattcgaaaccgcagctacgtcttctcctccctggccacgtcggctgtctccttcgccacgggggccctgggcatgtggatcccgctctacctgcaccgcgcccaagttgtgcagaagacagcagagacgtgcaacagcccgccctgtggggccaaggacagcctcatctttggggccatcacctgctttacgggatttctgggcgtggtcacgggggcaggagccacgcgctggtgccgcctgaagacccagcgggccgacccactggtgtgtgccgtgggcatgctgggctctgccatcttcatctgcctgatcttcgtggctgccaagagcagcatcgtaggagcctatatctgtatcttcgtcggggagacgctgctgttttctaactgggccatcactgcagacatcctcatgtacgtggtcatccccacgcggcgcgccactgccgtggccttgcagagcttcacctcccacctgctgggggacgccgggagcccctacctcattggctttatctcagacctgatccgccagagcactaaggactccccgctctgggagttcctgagcctgggctacgcgctcatgctctgccctttcgtcgtggtcctgggcggcatgttcttcctcgccactgcgctcttcttcgtcagcgaccgcgccagggctgagcagcaggtgaaccagctggcgatgccgcccgcatctgtgaaagtctga

SEQ ID NO: 238 - DNA, 1650 bp, synthetic construct
  misc_feature 1..1650: note = Homo sapiens
  source 1..1650: mol_type = other DNA
atgatgtgcctggaatgcgcctcggcggcggcgggcggcgcggaggaggaggaggcggacgcggagcggcggcgccggcgccggggggcgcagcgaggggctggcggtagcggttgctgcggggcgcggggcgcgggcggcgctggagtctcggccgcgggcgatgaggtgcagacgctgtcgggcagcgtaaggcgggccccgaccggaccccccggcacccccggcacccccggctgcgcagctactgcaaagggccccggcgctcagcagcccaaaccggccagcttgggccgcgggcggggggcagccgccgccatcctcagcttgggcaacgtgctcaactacctggacaggtacaccgtggcaggcgtccttctggacatccagcagcactttggggtcaaggaccgaggcgccggcctgctgcagtcagtgttcatctgtagcttcatggtggctgcccccatcttcggctacctgggcgaccgcttcaacaggaaggtgattctcagctgcggcattttcttctggtcggccgtcaccttctccagctccttcattccccagcagtacttctggctgctggtcctgtcccgggggctggtgggcatcggggaggccagctactccaccatcgcccccactatcattggcgacctcttcaccaagaacacgcgtacgctcatgctgtccgtcttctacttcgccatcccactgggcagtggcctgggctacattactggctccagcgtgaagcaggcagccgccgactggcactgggcattgcgggtgtcccctgtcctgggcatgatcacaggaacactcatcctcattctggtcccagccactaaaaggggtcatgccgaccagctcggggaccagctcaaggcccggacctcatggctccgagatatgaaggccctgattcgaaaccgcagctacgtcttctcctccctggccacgtcggctgtctccttcgccacgggggccctgggcatgtggatcccgctctacctgcaccgcgcccaagttgtgcagaagacagcagagacgtgcaacagcccgccctgtggggccaaggacagcctcatctttggggccatcacctgctttacgggatttctgggcgtggtcacgggggcaggagccacgcgctggtgccgcctgaagacccagcgggccgacccactggtgtgtgccgtgggcatgctgggctctgccatcttcatctgcctgatcttcgtggctgccaagagcagcatcgtaggagcctatatctgtatcttcgtcggggagacgctgctgttttctaactgggccatcactgcagacatcctcatgtacgtggtcatccccacgcggcgcgccactgccgtggccttgcagagcttcacctcccacctgctgggggacgccgggagcccctacctcattggctttatctcagacctgatccgccagagcactaaggactccccgctctgggagttcctgagcctgggctacgcgctcatgctctgccctttcgtcgtggtcctgggcggcatgttcttcctcgccactgcgctcttcttcgtcagcgaccgcgccagggctgagcagcaggtgaaccagctggcgatgccgcccgcatctgtgaaagtctga

SEQ ID NO: 239 - DNA, 1650 bp, synthetic construct
  misc_feature 1..1650: note = Homo sapiens
  source 1..1650: mol_type = other DNA
atgatgtgcctggaatgcgcctcggcggcggcgggcggcgcggaggaggaggaggcggacgcggagcggcggcgccggcgccggggggcgcagcgaggggctggcggtagcggttgctgcggggcgcggggcgcgggcggcgctggagtctcggccgcgggcgatgaggtgcagacgctgtcgggcagcgtaaggcgggccccgaccggaccccccggcacccccggcacccccggctgcgcagctactgcaaagggccccggcgctcagcagcccaaaccggccagcttgggccgcgggcggggggcagccgccgccatcctcagcttgggcaacgtgctcaactacctggacaggtacaccgtggcaggcgtccttctggacatccagcagcactttggggtcaaggaccgaggcgccggcctgctgcagtcagtgttcatctgtagcttcatggtggctgcccccatcttcggctacctgggcgaccgcttcaacaggaaggtgattctcagctgcggcattttcttctggtcggccgtcaccttctccagctccttcattccccagcagtacttctggctgctggtcctgtcccgggggctggtgggcatcggggaggccagctactccaccatcgcccccactatcattggcgacctcttcaccaagaacacgcgtacgctcatgctgtccgtcttctacttcgccatcccactgggcagtggcctgggctacattactggctccagcgtgaagcaggcagccggagcctggcactgggcattgcgggtgtcccctgtcctgggcatgatcacaggaacactcatcctcattctggtcccagccactaaaaggggtcatgccgaccagctcggggaccagctcaaggcccggacctcatggctccgagatatgaaggccctgattcgaaaccgcagctacgtcttctcctccctggccacgtcggctgtctccttcgccacgggggccctgggcatgtggatcccgctctacctgcaccgcgcccaagttgtgcagaagacagcagagacgtgcaacagcccgccctgtggggccaaggacagcctcatctttggggccatcacctgctttacgggatttctgggcgtggtcacgggggcaggagccacgcgctggtgccgcctgaagacccagcgggccgacccactggtgtgtgccgtgggcatgctgggctctgccatcttcatctgcctgatcttcgtggctgccaagagcagcatcgtaggagcctatatctgtatcttcgtcggggagacgctgctgttttctaactgggccatcactgcagacatcctcatgtacgtggtcatccccacgcggcgcgccactgccgtggccttgcagagcttcacctcccacctgctgggggacgccgggagcccctacctcattggctttatctcagacctgatccgccagagcactaaggactccccgctctgggagttcctgagcctgggctacgcgctcatgctctgccctttcgtcgtggtcctgggcggcatgttcttcctcgccactgcgctcttcttcgtcagcgaccgcgccagggctgagcagcaggtgaaccagctggcgatgccgcccgcatctgtgaaagtctga

SEQ ID NO: 240 - DNA, 1650 bp, synthetic construct
  misc_feature 1..1650: note = Homo sapiens
  source 1..1650: mol_type = other DNA
atgatgtgcctggaatgcgcctcggcggcggcgggcggcgcggaggaggaggaggcggacgcggagcggcggcgccggcgccggggggcgcagcgaggggctggcggtagcggttgctgcggggcgcggggcgcgggcggcgctggagtctcggccgcgggcgatgaggtgcagacgctgtcgggcagcgtaaggcgggccccgaccggaccccccggcacccccggcacccccggctgcgcagctactgcaaagggccccggcgctcagcagcccaaaccggccagcttgggccgcgggcggggggcagccgccgccatcctcagcttgggcaacgtgctcaactacctggacaggtacaccgtggcaggcgtccttctggacatccagcagcactttggggtcaaggaccgaggcgccggcctgctgcagtcagtgttcatctgtagcttcatggtggctgcccccatcttcggctacctgggcgaccgcttcaacaggaaggtgattctcagctgcggcattttcttctggtcggccgtcaccttctccagctccttcattccccagcagtacttctggctgctggtcctgtcccgggggctggtgggcatcggggaggccagctactccaccatcgcccccactatcattggcgacctcttcaccaagaacacgcgtacgctcatgctgtccgtcttctacttcgccatcccactgggcagtggcctgggctacattactggctccagcgtgaagcaggcagccggagacgcccactgggcattgcgggtgtcccctgtcctgggcatgatcacaggaacactcatcctcattctggtcccagccactaaaaggggtcatgccgaccagctcggggaccagctcaaggcccggacctcatggctccgagatatgaaggccctgattcgaaaccgcagctacgtcttctcctccctggccacgtcggctgtctccttcgccacgggggccctgggcatgtggatcccgctctacctgcaccgcgcccaagttgtgcagaagacagcagagacgtgcaacagcccgccctgtggggccaaggacagcctcatctttggggccatcacctgctttacgggatttctgggcgtggtcacgggggcaggagccacgcgctggtgccgcctgaagacccagcgggccgacccactggtgtgtgccgtgggcatgctgggctctgccatcttcatctgcctgatcttcgtggctgccaagagcagcatcgtaggagcctatatctgtatcttcgtcggggagacgctgctgttttctaactgggccatcactgcagacatcctcatgtacgtggtcatccccacgcggcgcgccactgccgtggccttgcagagcttcacctcccacctgctgggggacgccgggagcccctacctcattggctttatctcagacctgatccgccagagcactaaggactccccgctctgggagttcctgagcctgggctacgcgctcatgctctgccctttcgtcgtggtcctgggcggcatgttcttcctcgccactgcgctcttcttcgtcagcgaccgcgccagggctgagcagcaggtgaaccagctggcgatgccgcccgcatctgtgaaagtctga

SEQ ID NO: 241 - DNA, 1650 bp, synthetic construct
  misc_feature 1..1650: note = Homo sapiens
  source 1..1650: mol_type = other DNA
atgatgtgcctggaatgcgcctcggcggcggcgggcggcgcggaggaggaggaggcggacgcggagcggcggcgccggcgccggggggcgcagcgaggggctggcggtagcggttgctgcggggcgcggggcgcgggcggcgctggagtctcggccgcgggcgatgaggtgcagacgctgtcgggcagcgtaaggcgggccccgaccggaccccccggcacccccggcacccccggctgcgcagctactgcaaagggccccggcgctcagcagcccaaaccggccagcttgggccgcgggcggggggcagccgccgccatcctcagcttgggcaacgtgctcaactacctggacaggtacaccgtggcaggcgtccttctggacatccagcagcactttggggtcaaggaccgaggcgccggcctgctgcagtcagtgttcatctgtagcttcatggtggctgcccccatcttcggctacctgggcgaccgcttcaacaggaaggtgattctcagctgcggcattttcttctggtcggccgtcaccttctccagctccttcattccccagcagtacttctggctgctggtcctgtcccgggggctggtgggcatcggggaggccagctactccaccatcgcccccactatcattggcgacctcttcaccaagaacacgcgtacgctcatgctgtccgtcttctacttcgccatcccactgggcagtggcctgggctacattactggctccagcgtgaagcaggcagccggagactgggcctgggcattgcgggtgtcccctgtcctgggcatgatcacaggaacactcatcctcattctggtcccagccactaaaaggggtcatgccgaccagctcggggaccagctcaaggcccggacctcatggctccgagatatgaaggccctgattcgaaaccgcagctacgtcttctcctccctggccacgtcggctgtctccttcgccacgggggccctgggcatgtggatcccgctctacctgcaccgcgcccaagttgtgcagaagacagcagagacgtgcaacagcccgccctgtggggccaaggacagcctcatctttggggccatcacctgctttacgggatttctgggcgtggtcacgggggcaggagccacgcgctggtgccgcctgaagacccagcgggccgacccactggtgtgtgccgtgggcatgctgggctctgccatcttcatctgcctgatcttcgtggctgccaagagcagcatcgtaggagcctatatctgtatcttcgtcggggagacgctgctgttttctaactgggccatcactgcagacatcctcatgtacgtggtcatccccacgcggcgcgccactgccgtggccttgcagagcttcacctcccacctgctgggggacgccgggagcccctacctcattggctttatctcagacctgatccgccagagcactaaggactccccgctctgggagttcctgagcctgggctacgcgctcatgctctgccctttcgtcgtggtcctgggcggcatgttcttcctcgccactgcgctcttcttcgtcagcgaccgcgccagggctgagcagcaggtgaaccagctggcgatgccgcccgcatctgtgaaagtctga

SEQ ID NO: 242 - DNA, 1650 bp, synthetic construct
  misc_feature 1..1650: note = Homo sapiens
  source 1..1650: mol_type = other DNA
atgatgtgcctggaatgcgcctcggcggcggcgggcggcgcggaggaggaggaggcggacgcggagcggcggcgccggcgccggggggcgcagcgaggggctggcggtagcggttgctgcggggcgcggggcgcgggcggcgctggagtctcggccgcgggcgatgaggtgcagacgctgtcgggcagcgtaaggcgggccccgaccggaccccccggcacccccggcacccccggctgcgcagctactgcaaagggccccggcgctcagcagcccaaaccggccagcttgggccgcgggcggggggcagccgccgccatcctcagcttgggcaacgtgctcaactacctggacaggtacaccgtggcaggcgtccttctggacatccagcagcactttggggtcaaggaccgaggcgccggcctgctgcagtcagtgttcatctgtagcttcatggtggctgcccccatcttcggctacctgggcgaccgcttcaacaggaaggtgattctcagctgcggcattttcttctggtcggccgtcaccttctccagctccttcattccccagcagtacttctggctgctggtcctgtcccgggggctggtgggcatcggggaggccagctactccaccatcgcccccactatcattggcgacctcttcaccaagaacacgcgtacgctcatgctgtccgtcttctacttcgccatcccactgggcagtggcctgggctacattactggctccagcgtgaagcagttcgccggagactggcactgggcattgcgggtgtcccctgtcctgggcatgatcacaggaacactcatcctcattctggtcccagccactaaaaggggtcatgccgaccagctcggggaccagctcaaggcccggacctcatggctccgagatatgaaggccctgattcgaaaccgcagctacgtcttctcctccctggccacgtcggctgtctccttcgccacgggggccctgggcatgtggatcccgctctacctgcaccgcgcccaagttgtgcagaagacagcagagacgtgcaacagcccgccctgtggggccaaggacagcctcatctttggggccatcacctgctttacgggatttctgggcgtggtcacgggggcaggagccacgcgctggtgccgcctgaagacccagcgggccgacccactggtgtgtgccgtgggcatgctgggctctgccatcttcatctgcctgatcttcgtggctgccaagagcagcatcgtaggagcctatatctgtatcttcgtcggggagacgctgctgttttctaactgggccatcactgcagacatcctcatgtacgtggtcatccccacgcggcgcgccactgccgtggccttgcagagcttcacctcccacctgctgggggacgccgggagcccctacctcattggctttatctcagacctgatccgccagagcactaaggactccccgctctgggagttcctgagcctgggctacgcgctcatgctctgccctttcgtcgtggtcctgggcggcatgttcttcctcgccactgcgctcttcttcgtcagcgaccgcgccagggctgagcagcaggtgaaccagctggcgatgccgcccgcatctgtgaaagtctga

SEQ ID NO: 243 - DNA, 1650 bp, synthetic construct
  misc_feature 1..1650: note = Homo sapiens
  source 1..1650: mol_type = other DNA
atgatgtgcctggaatgcgcctcggcggcggcgggcggcgcggaggaggaggaggcggacgcggagcggcggcgccggcgccggggggcgcagcgaggggctggcggtagcggttgctgcggggcgcggggcgcgggcggcgctggagtctcggccgcgggcgatgaggtgcagacgctgtcgggcagcgtaaggcgggccccgaccggaccccccggcacccccggcacccccggctgcgcagctactgcaaagggccccggcgctcagcagcccaaaccggccagcttgggccgcgggcggggggcagccgccgccatcctcagcttgggcaacgtgctcaactacctggacaggtacaccgtggcaggcgtccttctggacatccagcagcactttggggtcaaggaccgaggcgccggcctgctgcagtcagtgttcatctgtagcttcatggtggctgcccccatcttcggctacctgggcgaccgcttcaacaggaaggtgattctcagctgcggcattttcttctggtcggccgtcaccttctccagctccttcattccccagcagtacttctggctgctggtcctgtcccgggggctggtgggcatcggggaggccagctactccaccatcgcccccactatcattggcgacctcttcaccaagaacacgcgtacgctcatgctgtccgtcttctacttcgccatcccactgggcagtggcctgggctacattactggctccagcgtgaagcaggcattcggagactggcactgggcattgcgggtgtcccctgtcctgggcatgatcacaggaacactcatcctcattctggtcccagccactaaaaggggtcatgccgaccagctcggggaccagctcaaggcccggacctcatggctccgagatatgaaggccctgattcgaaaccgcagctacgtcttctcctccctggccacgtcggctgtctccttcgccacgggggccctgggcatgtggatcccgctctacctgcaccgcgcccaagttgtgcagaagacagcagagacgtgcaacagcccgccctgtggggccaaggacagcctcatctttggggccatcacctgctttacgggatttctgggcgtggtcacgggggcaggagccacgcgctggtgccgcctgaagacccagcgggccgacccactggtgtgtgccgtgggcatgctgggctctgccatcttcatctgcctgatcttcgtggctgccaagagcagcatcgtaggagcctatatctgtatcttcgtcggggagacgctgctgttttctaactgggccatcactgcagacatcctcatgtacgtggtcatccccacgcggcgcgccactgccgtggccttgcagagcttcacctcccacctgctgggggacgccgggagcccctacctcattggctttatctcagacctgatccgccagagcactaaggactccccgctctgggagttcctgagcctgggctacgcgctcatgctctgccctttcgtcgtggtcctgggcggcatgttcttcctcgccactgcgctcttcttcgtcagcgaccgcgccagggctgagcagcaggtgaaccagctggcgatgccgcccgcatctgtgaaagtctga

SEQ ID NO: 244 - DNA, 21 bp, synthetic construct
  misc_feature 1..21: note = primer
  source 1..21: mol_type = other DNA
gatagactgatgggggtgttg

SEQ ID NO: 245 - DNA, 21 bp, synthetic construct
  misc_feature 1..21: note = Primer
  source 1..21: mol_type = other DNA
gatagacagatgggggtgttg

SEQ ID NO: 246 - DNA, 21 bp, synthetic construct
  misc_feature 1..21: note = Primer
  source 1..21: mol_type = other DNA
gatagaccgatggggctgttg

SEQ ID NO: 247 - DNA, 21 bp, synthetic construct
  misc_feature 1..21: note = Primer
  source 1..21: mol_type = other DNA
gatagacagatggggctgttg

SEQ ID NO: 248 - DNA, 20 bp, synthetic construct
  misc_feature 1..20: note = Primer
  source 1..20: mol_type = other DNA
ccatggacatcagtctcagc

SEQ ID NO: 249 - DNA, 19 bp, synthetic construct
  misc_feature 1..19: note = Primer
  source 1..19: mol_type = other DNA
catggacatcaggctcagc

SEQ ID NO: 250 - DNA, 19 bp, synthetic construct
  misc_feature 1..19: note = Primer
  source 1..19: mol_type = other DNA
catggctgtcctggtgctg

SEQ ID NO: 251 - DNA, 19 bp, synthetic construct
  misc_feature 1..19: note = Primer
  source 1..19: mol_type = other DNA
aatggctgtcctggtgctg

SEQ ID NO: 252 - DNA, 19 bp, synthetic construct
  misc_feature 1..19: note = Primer
  source 1..19: mol_type = other DNA
catggctgtcctggtgcta

SEQ ID NO: 253 - DNA, 19 bp, synthetic construct
  misc_feature 1..19: note = Primer
  source 1..19: mol_type = other DNA
catggatgtcctggtgctg

SEQ ID NO: 254 - DNA, 19 bp, synthetic construct
  misc_feature 1..19: note = Primer
  source 1..19: mol_type = other DNA
catggctgtcctggcgctc

SEQ ID NO: 255 - DNA, 19 bp, synthetic construct
  misc_feature 1..19: note = Primer
  source 1..19: mol_type = other DNA
catggctatcctggtgctg

SEQ ID NO: 256 - DNA, 20 bp, synthetic construct
  misc_feature 1..20: note = Primer
  source 1..20: mol_type = other DNA
ccatgggatggagccagatc

SEQ ID NO: 257 - DNA, 20 bp, synthetic construct
  misc_feature 1..20: note = Primer
  source 1..20: mol_type = other DNA
ccatgggatggatctgtatc

SEQ ID NO: 258 - DNA, 20 bp, synthetic construct
  misc_feature 1..20: note = Primer
  source 1..20: mol_type = other DNA
ccatggacaggcttacttcc

SEQ ID NO: 259 - DNA, 20 bp, synthetic construct
  misc_feature 1..20: note = Primer
  source 1..20: mol_type = other DNA
ccatggacttcagcatcagc

SEQ ID NO: 260 - DNA, 20 bp, synthetic construct
  misc_feature 1..20: note = Primer
  source 1..20: mol_type = other DNA
ccatgtacttcagcatcagc

SEQ ID NO: 261 - DNA, 20 bp, synthetic construct
  misc_feature 1..20: note = Primer
  source 1..20: mol_type = other DNA
ccatggacttcaggctcagc

SEQ ID NO: 262 - DNA, 20 bp, synthetic construct
  misc_feature 1..20: note = Primer
  source 1..20: mol_type = other DNA
ccatggacttcaggctgaac

SEQ ID NO: 263 - DNA, 20 bp, synthetic construct
  misc_feature 1..20: note = Primer
  source 1..20: mol_type = other DNA
ccatggaatggagctgggtc

SEQ ID NO: 264 - DNA, 20 bp, synthetic construct
  misc_feature 1..20: note = Primer
  source 1..20: mol_type = other DNA
ccatggaatggaactgggtc

SEQ ID NO: 265 - DNA, 20 bp, synthetic construct
  misc_feature 1..20: note = Primer
  source 1..20: mol_type = other DNA
catgaaatgcagctggatca

SEQ ID NO: 266 - DNA, 20 bp, synthetic construct
  misc_feature 1..20: note = Primer
  source 1..20: mol_type = other DNA
catgaaaagcagctggatca

SEQ ID NO: 267 - DNA, 21 bp, synthetic construct
  misc_feature 1..21: note = Primer
  source 1..21: mol_type = other DNA
aacatggagttggaattgagc

SEQ ID NO: 268 - DNA, 22 bp, synthetic construct
  misc_feature 1..22: note = Primer
  source 1..22: mol_type = other DNA
catgaagttgagattgagctta

SEQ ID NO: 269 - DNA, 21 bp, synthetic construct
  misc_feature 1..21: note = Primer
  source 1..21: mol_type = other DNA
catggagttcagcatgatctg

SEQ ID NO: 270 - DNA, 20 bp, synthetic construct
  misc_feature 1..20: note = Primer
  source 1..20: mol_type = other DNA
ccatggaatggagctttgtc

SEQ ID NO: 271 - DNA, 21 bp, synthetic construct
  misc_feature 1..21: note = Primer
  source 1..21: mol_type = other DNA
agatgagaatgctggttcttc

SEQ ID NO: 272 - DNA, 20 bp, synthetic construct
  misc_feature 1..20: note = Primer
  source 1..20: mol_type = other DNA
ccatggattgtagctgggtc

SEQ ID NO: 273 - DNA, 19 bp, synthetic construct
  misc_feature 1..19: note = Primer
  source 1..19: mol_type = other DNA
catggacaccaggctcagc

SEQ ID NO: 274 - DNA, 19 bp, synthetic construct
  misc_feature 1..19: note = Primer
  source 1..19: mol_type = other DNA
catggctgccctggggctg

SEQ ID NO: 275 - DNA, 19 bp, synthetic construct
  misc_feature 1..19: note = Primer
  source 1..19: mol_type = other DNA
catggctttcctggggctg

SEQ ID NO: 276 - DNA, 19 bp, synthetic construct
  misc_feature 1..19: note = Primer
  source 1..19: mol_type = other DNA
catggctgtgctggtgttg

SEQ ID NO: 277 - DNA, 19 bp, synthetic construct
  misc_feature 1..19: note = Primer
  source 1..19: mol_type = other DNA
gatggcggtgcagatttcc

SEQ ID NO: 278 - DNA, 20 bp, synthetic construct
  misc_feature 1..20: note = Primer
  source 1..20: mol_type = other DNA
ccatggacaggctaacttcc

SEQ ID NO: 279 - DNA, 20 bp, synthetic construct
  misc_feature 1..20: note = Primer
  source 1..20: mol_type = other DNA
ccatggaatggggctgggtc

SEQ ID NO: 280 - DNA, 20 bp, synthetic construct
  misc_feature 1..20: note = Primer
  source 1..20: mol_type = other DNA
ccatgaagtcgtggctgaac

SEQ ID NO: 281 - DNA, 20 bp, synthetic construct
  misc_feature 1..20: note = Primer
  source 1..20: mol_type = other DNA
ccatgaagtcgtggctgaac

SEQ ID NO: 282 - DNA, 19 bp, synthetic construct
  misc_feature 1..19: note = Primer
  source 1..19: mol_type = other DNA
catgaaatgcagctgggtc

SEQ ID NO: 283 - DNA, 21 bp, synthetic construct
  misc_feature 1..21: note = Primer
  source 1..21: mol_type = other DNA
aacatggagttggaactgaga

SEQ ID NO: 284 - DNA, 22 bp, synthetic construct
  misc_feature 1..22: note = Primer
  source 1..22: mol_type = other DNA
caacatggaattggaactgaga

SEQ ID NO: 285 - DNA, 20 bp, synthetic construct
  misc_feature 1..20: note = Primer
  source 1..20: mol_type = other DNA
catgatggctccagttcaac

SEQ ID NO: 286 - DNA, 20 bp, synthetic construct
  misc_feature 1..20: note = Primer
  source 1..20: mol_type = other DNA
catgaactggatccgccagc

SEQ ID NO: 287 - DNA, 21 bp, synthetic construct
  misc_feature 1..21: note = Primer
  source 1..21: mol_type = other DNA
atcatggattggttgtggacc

SEQ ID NO: 288 - DNA, 20 bp, synthetic construct
  misc_feature 1..20: note = Primer
  source 1..20: mol_type = other DNA
gtgctgtctttgctgtcctg

SEQ ID NO: 289 - DNA, 20 bp, synthetic construct
  misc_feature 1..20: note = Primer
  source 1..20: mol_type = other DNA
catgatggctgcagttcaac

SEQ ID NO: 290 - DNA, 20 bp, synthetic construct
  misc_feature 1..20: note = Primer
  source 1..20: mol_type = other DNA
catgatggctgcacttcaac

SEQ ID NO: 291 - DNA, 20 bp, synthetic construct
  misc_feature 1..20: note = Primer
  source 1..20: mol_type = other DNA
catgatggcaccagttcaac

SEQ ID NO: 292 - DNA, 20 bp, synthetic construct
  misc_feature 1..20: note = Primer
  source 1..20: mol_type = other DNA
catgatggctccagttcaac

SEQ ID NO: 293 - DNA, 22 bp, synthetic construct
  misc_feature 1..22: note = Primer
  source 1..22: mol_type = other DNA
atggctccagttcaacttttag

SEQ ID NO: 294 - DNA, 20 bp, synthetic construct
  misc_feature 1..20: note = Primer
  source 1..20: mol_type = other DNA
catgatggctccagtccagc

SEQ ID NO: 295 - DNA, 20 bp, synthetic construct
  misc_feature 1..20: note = Primer
  source 1..20: mol_type = other DNA
caatgatgagtcctgcccag

SEQ ID NO: 296 - DNA, 23 bp, synthetic construct
  misc_feature 1..23: note = Primer
  source 1..23: mol_type = other DNA
caatgatgagtcctgcccagttc

SEQ ID NO: 297 - DNA, 22 bp, synthetic construct
  misc_feature 1..22: note = Primer
  source 1..22: mol_type = other DNA
caatgatgagtcctgtccagtc

SEQ ID NO: 298 - DNA, 22 bp, synthetic construct
  misc_feature 1..22: note = Primer
  source 1..22: mol_type = other DNA
caatgatgagtcctgtccagac

SEQ ID NO: 299 - DNA, 23 bp, synthetic construct
  misc_feature 1..23: note = Primer
  source 1..23: mol_type = other DNA
caatgatgattcctgcccagttc

SEQ ID NO: 300 - DNA, 21 bp, synthetic construct
  misc_feature 1..21: note = Primer
  source 1..21: mol_type = other DNA
aatgatgatcctgtttattcc

SEQ ID NO: 301 - DNA, 19 bp, synthetic construct
  misc_feature 1..19: note = Primer
  source 1..19: mol_type = other DNA
gatgagtcctgtccagtcc

SEQ ID NO: 302 - DNA, 20 bp, synthetic construct
  misc_feature 1..20: note = Primer
  source 1..20: mol_type = other DNA
acatgggtgtgcccactcag

SEQ ID NO: 303 - DNA, 20 bp, synthetic construct
  misc_feature 1..20: note = Primer
  source 1..20: mol_type = other DNA
acatgggtgtccccactcag

SEQ ID NO: 304 - DNA, 20 bp, synthetic construct
  misc_feature 1..20: note = Primer
  source 1..20: mol_type = other DNA
acatggctgtgcccactcag

SEQ ID NO: 305 - DNA, 21 bp, synthetic construct
  misc_feature 1..21: note = Primer
  source 1..21: mol_type = other DNA
aaatgaagtggcctgttaggc

SEQ ID NO: 306 - DNA, 21 bp, synthetic construct
  misc_feature 1..21: note = Primer
  source 1..21: mol_type = other DNA
aaatgaagtggcctgtgaggc

SEQ ID NO: 307 - DNA, 21 bp, synthetic construct
  misc_feature 1..21: note = Primer
  source 1..21: mol_type = other DNA
atgagggtggctgttcaattc

SEQ ID NO: 308 - DNA, 20 bp, synthetic construct
  misc_feature 1..20: note = Primer
  source 1..20: mol_type = other DNA
catgggtgtgcctactcatc

SEQ ID NO: 309 - DNA, 20 bp, synthetic construct
  misc_feature 1..20: note = Primer
  source 1..20: mol_type = other DNA
catgaacgtgcccactcaac

SEQ ID NO: 310 - DNA, 20 bp, synthetic construct
  misc_feature 1..20: note = Primer
  source 1..20: mol_type = other DNA
catgaatgtgcccactcaac

SEQ ID NO: 311 - DNA, 19 bp, synthetic construct
  misc_feature 1..19: note = Primer
  source 1..19: mol_type = other DNA
atggacatgagggcccatg

SEQ ID NO: 312 - DNA, 19 bp, synthetic construct
  misc_feature 1..19: note = Primer
  source 1..19: mol_type = other DNA
atggacatgagggtccatg

SEQ ID NO: 313 - DNA, 20 bp, synthetic construct
  misc_feature 1..20: note = Primer
  source 1..20: mol_type = other DNA
catggacatgagggcccata

SEQ ID NO: 314 - DNA, 20 bp, synthetic construct
  misc_feature 1..20: note = Primer
  source 1..20: mol_type = other DNA
catggacaagagggcccatg

SEQ ID NO: 315 - DNA, 21 bp, synthetic construct
  misc_feature 1..21: note = Primer
  source 1..21: mol_type = other DNA
atggaatcacaaactcaggcc

SEQ ID NO: 316 - DNA, 21 bp, synthetic construct
  misc_feature 1..21: note = Primer
  source 1..21: mol_type = other DNA
atggagtcatatactcgggtc

SEQ ID NO: 317 - DNA, 21 bp, synthetic construct
  misc_feature 1..21: note = Primer
  source 1..21: mol_type = other DNA
atggagtcacatactagggtc

SEQ ID NO: 318 - DNA, 21 bp, synthetic construct
  misc_feature 1..21: note = Primer
  source 1..21: mol_type = other DNA
atggaatcacatactcaggtc

SEQ ID NO: 319 - DNA, 20 bp, synthetic construct
  misc_feature 1..20: note = Primer
  source 1..20: mol_type = other DNA
gatggaatcacaaacgcagg

SEQ ID NO: 320 - DNA, 20 bp, synthetic construct
  misc_feature 1..20: note = Primer
  source 1..20: mol_type = other DNA
gatggaatcacagacccagg

SEQ ID NO: 321 - DNA, 21 bp, synthetic construct
  misc_feature 1..21: note = Primer
  source 1..21: mol_type = other DNA
atgaggtgctctttccagttc

SEQ ID NO: 322 - DNA, 22 bp, synthetic construct
  misc_feature 1..22: note = Primer
  source 1..22: mol_type = other DNA
atgaagtttcctgctcagtttc

SEQ ID NO: 323 - DNA, 24 bp, synthetic construct
  misc_feature 1..24: note = Primer
  source 1..24: mol_type = other DNA
atggattttctggtgcaaattttc

SEQ ID NO: 324 - DNA, 21 bp, synthetic construct
  misc_feature 1..21: note = Primer
  source 1..21: mol_type = other DNA
ctatggattgttgggtgcaga

SEQ ID NO: 325 - DNA, 21 bp, synthetic construct
  misc_feature 1..21: note = Primer
  source 1..21: mol_type = other DNA
caatggattttcgggtgcaga

SEQ ID NO: 326 - DNA, 21 bp, synthetic construct
  misc_feature 1..21: note = Primer
  source 1..21: mol_type = other DNA
caatggattttcaggtgcaga

SEQ ID NO: 327 - DNA, 21 bp, synthetic construct
  misc_feature 1..21: note = Primer
  source 1..21: mol_type = other DNA
catgaaaatgacgacacctgc

SEQ ID NO: 328 - DNA, 22 bp, synthetic construct
  misc_feature 1..22: note = Primer
  source 1..22: mol_type = other DNA
atgagggtccagattcagtttc

SEQ ID NO: 329 - DNA, 22 bp, synthetic construct
  misc_feature 1..22: note = Primer
  source 1..22: mol_type = other DNA
atgagggtccagattcagtttg

SEQ ID NO: 330 - DNA, 22 bp, synthetic construct
  misc_feature 1..22: note = Primer
  source 1..22: mol_type = other DNA
atgagggtccaggttcagtttc

SEQ ID NO: 331 - DNA, 21 bp, synthetic construct
  misc_feature 1..21: note = Primer
  source 1..21: mol_type = other DNA
atgagggtccctgttcaattc

SEQ ID NO: 332 - DNA, 21 bp, synthetic construct
  misc_feature 1..21: note = Primer
  source 1..21: mol_type = other DNA
atggagacagacagactcctg

SEQ ID NO: 333 - DNA, 21 bp, synthetic construct
  misc_feature 1..21: note = Primer
  source 1..21: mol_type = other DNA
atggagacagacacactcctg

SEQ ID NO: 334 - DNA, 19 bp, synthetic construct
  misc_feature 1..19: note = Primer
  source 1..19: mol_type = other DNA
catgctctccctagctcac

SEQ ID NO: 335 - DNA, 21 bp, synthetic construct
  misc_feature 1..21: note = Primer
  source 1..21: mol_type = other DNA
atggtgttcatacctcagttc

SEQ ID NO: 336 - DNA, 25 bp, synthetic construct
  misc_feature 1..25: note = Primer
  source 1..25: mol_type = other DNA
gataggtgyaccatytrccttccag

SEQ ID NO: 337 - DNA, 24 bp, synthetic construct
  misc_feature 1..24: note = Primer
  source 1..24: mol_type = other DNA
atggcctggayttcacttatactc

SEQ ID NO: 338 - DNA, 22 bp, synthetic construct
  misc_feature 1..22: note = Primer
  source 1..22: mol_type = other DNA
atggcctggactcctctcttct

SEQ ID NO: 339 - DNA, 25 bp, synthetic construct
  misc_feature 1..25: note = Primer
  source 1..25: mol_type = other DNA
atgacctgtacttcacttttgctta

SEQ ID NO: 340 - DNA, 25 bp, synthetic construct
  misc_feature 1..25: note = Primer
  source 1..25: mol_type = other DNA
atgacatggactctmctattccttg

SEQ ID NO: 341 - DNA, 23 bp, synthetic construct
  misc_feature 1..23: note = Primer
  source 1..23: mol_type = other DNA
atggccttggcctatcttctatc

SEQ ID NO: 342 - DNA, 22 bp, synthetic construct
  misc_feature 1..22: note = Primer
  source 1..22: mol_type = other DNA
atggccaggataccccttcttt

SEQ ID NO: 343 - DNA, 27 bp, synthetic construct
  misc_feature 1..27: note = Primer
  source 1..27: mol_type = other DNA
accatggactctactattccttgcctt

SEQ ID NO: 344 - DNA, 26 bp, synthetic construct
  misc_feature 1..26: note = Primer
  source 1..26: mol_type = other DNA
accatgacttgggctccactactcct

SEQ ID NO: 345 - protein, 459 aa, synthetic construct
  REGION 1..459: note = Mouse IgG1 chimera antibody: heavy chain
METDTLLLWVLLLWVPGSTGEVQLQQSGAGLVRPRTSVRLSCKISGDSITAYYVHFVKQRPGQGLEWIGRIDPEDDSTKYSEKFKNKATLTADVSSSTAYLILSSLTSDDSATYFCSTLTGLDYWGQGVMVTVSSAKTTPPSVYPLAPGSAAQTNSMVTLGCLVKGYFPEPVTVTWNSGSLSSGVHTFPAVLQSDLYTLSSSVTVPSSTWPSETVTCNVAHPASSTKVDKKIVPRDCGCKPCICTVPEVSSVFIFPPKPKDVLTITLTPKVTCVVVDISKDDPEVQFSWFVDDVEVHTAQTQPREEQFNSTFRSVSELPIMHQDWLNGKEFKCRVNSAAFPAPIEKTISKTKGRPKAPQVYTIPPPKEQMAKDKVSLTCMITDFFPEDITVEWQWNGQPAENYKNTQPIMDTDGSYFVYSKLNVQKSNWEAGNTFTCSVLHEGLHNHHTEKSLSHSPGK

SEQ ID NO: 346 - protein, 233 aa, synthetic construct
  REGION 1..233: note = Mouse IgG1 chimera antibody: light chain
METDTLLLWVLLLWVPGSTGDIQMTQSPPVLSASVGDRVTLSCKASQSVHNKLDWYQQKHGEAPKLLIYYTHNLQTGIPSRFSGSGSGSDYTLTISSLRAEDVATYYCFQYYSGWTFGGGTKLEMKRADAAPTVSIFPPSSEQLTSGGASVVCFLNNFYPKDINVKWKIDGSERQNGVLNSWTDQDSKDSTYSMSSTLTLTKDEYERHNSYTCEATHKTSTSPIVKSFNRNEC

SEQ ID NO: 347 - DNA, 1380 bp, synthetic construct
  misc_feature 1..1380: note = Expression vector of mouse IgG1 chimera antibody: heavy chain
  source 1..1380: mol_type = other DNA
atggaaaccgatacactgctgctgtgggtcctgctgctgtgggtgccaggatccacaggcgaagtccagctgcagcagtctggggctggacttgtgagacctaggacctctgtgaggttatcttgcaaaatttctggcgattccattacagcatattacgtgcactttgtgaaacaaaggcctggacagggtctggaatggataggaagaattgatcctgaggatgatagtactaaatattctgagaagttcaaaaacaaggcgacactcactgcagatgtatcctccagcacagcctacctgattctcagcagcctgacctctgacgactctgcaacctatttttgttccactctgactggccttgattactggggccagggagtcatggtcacggtctcctcagctaaaacgacacccccatctgtctatccactggcccctggatctgctgcccaaactaactccatggtgaccctgggatgcctggtcaagggctatttccctgagccagtgacagtgacctggaactctggatccctgtccagcggtgtgcacaccttcccagctgtcctgcagtctgacctctacactctgagcagctcagtgactgtcccctccagcacctggcccagcgagaccgtcacctgcaacgttgcccacccggccagcagcaccaaggtggacaagaaaattgtgcccagggattgtggttgtaagccttgcatatgtacagtcccagaagtatcatctgtcttcatcttccccccaaagcccaaggatgtgctcaccattactctgactcctaaggtcacgtgtgttgtggtagacatcagcaaggatgatcccgaggtccagttcagctggtttgtagatgatgtggaggtgcacacagctcagacgcaaccccgggaggagcagttcaacagcactttccgctcagtcagtgaacttcccatcatgcaccaggactggctcaatggcaaggagttcaaatgcagggtcaacagtgcagctttccctgcccccatcgagaaaaccatctccaaaaccaaaggcagaccgaaggctccgcaggtgtacaccattccacctcccaaggagcagatggccaaggataaagtcagtctgacctgcatgataacagacttcttccctgaagacattactgtggagtggcagtggaatgggcagccagcggagaactacaagaacactcagcccatcatggacacagatggctcttacttcgtctacagcaagctcaatgtgcagaagagcaactgggaggcaggaaatactttcacctgctctgtgttacatgagggcctgcacaaccaccatactgagaagagcctctcccactctcctggtaaatga

SEQ ID NO: 348 - DNA, 702 bp, synthetic construct
  misc_feature 1..702: note = Expression vector of mouse IgG1 chimera antibody: light chain
  source 1..702: mol_type = other DNA
atggaaaccgatactctgctgctgtgggtcctgctgctgtgggtccctggatccaccggagacatccagatgacccagtctcccccagtcctgtctgcatctgtgggagacagagtcactctcagctgcaaagcaagtcagagtgttcataacaagttagactggtatcagcaaaagcatggagaggctccgaaactcctgatttattatacacacaatttacaaacgggcatcccatcaaggttcagtggcagtggatccggttcagattacacactcaccatcagcagcctgcgggctgaagatgttgccacatattactgttttcaatattacagtgggtggacgttcggtggaggcaccaagctggaaatgaaacgggctgacgctgctcctacagtgtctatctttcccccctcgagtgagcagctgacctccggaggagctagcgtggtgtgcttcctgaacaacttctacccaaaggacatcaacgtgaagtggaagatcgatggctctgagaggcagaacggcgtgctgaattcctggacagaccaggattccaaggacagcacctattctatgagctctaccctgacactgaccaaggatgagtacgagagacataattcctatacctgtgaggcaacccataaaacttcaacaagcccaatcgtcaaatccttcaatcgtaatgagtgctga